European Patent Application EP 4 603 587 A1, published August 20, 2025. Title: Fusion protein of serum albumin and physiologically active protein. Applicant: JCR Pharmaceuticals Co., Ltd. The sequence listing filed with the application follows.

SEQUENCE LISTING (196 sequences)

SEQ ID NO: 1 - protein, 643 aa, Homo sapiens
YVLDDSDGLGREFDGIGAVSGGGATSRLLVNYPEPYRSQILDYLFKPNFGASLHILKVEIGGDGQTTDGTEPSHMHYALDENYFRGYEWWLMKEAKKRNPNITLIGLPWSFPGWLGKGFDWPYVNLQLTAYYVVTWIVGAKRYHDLDIDYIGIWNERSYNANYIKILRKMLNYQGLQRVKIIASDNLWESISASMLLDAELFKVVDVIGAHYPGTHSAKDAKLTGKKLWSSEDFSTLNSDMGAGCWGRILNQNYINGYMTSTIAWNLVASYYEQLPYGRCGLMTAQEPWSGHYVVESPVWVSAHTTQFTQPGWYYLKTVGHLEKGGSYVALTDGLGNLTIIIETMSHKHSKCIRPFLPYFNVSQQFATFVLKGSFSEIPELQVWYTKLGKTSERFLFKQLDSLWLLDSDGSFTLSLHEDELFTLTTLTTGRKGSYPLPPKSQPFPSTYKDDFNVDYPFFSEAPNFADQTGVFEYFTNIEDPGEHHFTLRQVLNQRPITWAADASNTISIIGDYNWTNLTIKCDVYIETPDTGGVFIAGRVNKGGILIRSARGIFFWIFANGSYRVTGDLAGWIIYALGRVEVTAKKWYTLTLTIKGHFTSGMLNDKSLWTDIPVNFPKNGWAAIGTHSFEFAQFDNFLVEATR

SEQ ID NO: 2 - DNA, 1929 bp, synthetic construct
  source 1..1929: mol_type = other DNA
tacgtgctggacgactctgacggactcggaagggagtttgacggcattggcgctgtgtccggaggcggcgctacatctcgtctgctggtgaattatcccgagccctaccggtcccagattttagactacctcttcaaacccaattttggagcctccctccacattttaaaggtggaaatcggcggcgacggacagacaaccgatggcaccgaacctagccatatgcactacgctttagacgagaactatttccggggctatgagtggtggctgatgaaggaggccaagaagaggaaccccaacattaccctcatcggactgccttggagctttcccggttggctgggcaaaggattcgactggccctacgtgaatttacagctgaccgcttactacgtggtgacttggattgtgggagccaagcggtaccacgatctcgacatcgattacattggcatctggaacgagcggagctacaacgctaactatatcaagattctgcggaaaatgctgaattaccaaggtttacagcgggtgaagatcatcgctagcgacaatttatgggaaagcatctccgctagcatgctgctggacgctgaactgttcaaagtcgtggatgtcatcggcgctcactatcccggcacccatagcgccaaggacgccaagctgaccggaaaaaagctgtggtccagcgaggatttcagcactttaaactccgatatgggagctggctgctggggccggattttaaaccagaactacatcaatggctacatgacaagcaccatcgcttggaatttagtggcctcctactacgagcagctgccctatggacggtgcggtttaatgacagcccaagagccttggagcggccattacgtggtggagagccccgtttgggtgagcgctcacaccacccagttcacccagcccggctggtactacctcaagaccgtcggacatctggagaagggcggctcctacgtggctttaactgatggtttaggcaatctgaccatcattatcgagaccatgtcccacaagcactccaagtgcatccggccctttctgccctacttcaacgtgtcccagcaattcgccacctttgtgctgaagggcagcttttccgagattcccgagctccaagtttggtacaccaagctgggaaaaaccagcgagaggtttttattcaagcaactggactctttatggctgctggacagcgatggctccttcacactgtctttacatgaggatgagctctttactttaaccactttaacaactggtcggaaaggctcctatcctttaccccccaagagccaacccttccccagcacctacaaggacgacttcaacgtggattaccccttcttctccgaggctcccaactttgctgaccagaccggcgtgttcgagtatttcaccaacatcgaggaccccggtgagcaccatttcaccctccggcaagttctgaaccaacggcctatcacttgggccgccgacgcttccaataccatctccattatcggcgactacaactggacaaatttaactatcaagtgcgacgtctacatcgagacccccgataccggaggcgtgtttatcgctggaagggtgaacaaaggcggcattttaatccggtccgctaggggcatctttttctggatcttcgctaacggcagctatcgggtgactggtgacctcgctggctggatcatttacgctctgggccgggtggaggtgacagccaagaagtggtacactttaactttaactattaagggacattttaccagcggcatgctgaacgacaaatctttatggaccgacatccccgtgaactttcccaagaatggctgggccgccatcggcacccattcctttgaattcgcccagttcgacaatttcctcgtggaagccacccgg

SEQ ID NO: 3 - protein, 585 aa, Homo sapiens [sequence omitted]

SEQ ID NO: 4 - DNA, 1755 bp, synthetic construct
  source 1..1755: mol_type = other DNA
gatgcacacaagagtgaggttgctcatcggtttaaagatttgggagaagaaaatttcaaagccttggtgttgattgcctttgctcagtatcttcagcagtgtccatttgaagatcatgtaaaattagtgaatgaagtaactgaatttgcaaaaacatgtgttgctgatgagtcagctgaaaattgtgacaaatcacttcataccctttttggagacaaattatgcacagttgcaactcttcgtgaaacctatggtgaaatggctgactgctgtgcaaaacaagaacctgagagaaatgaatgcttcttgcaacacaaagatgacaacccaaacctcccccgattggtgagaccagaggttgatgtgatgtgcactgcttttcatgacaatgaagagacatttttgaaaaaatacttatatgaaattgccagaagacatccttacttttatgccccggaactccttttctttgctaaaaggtataaagctgcttttacagaatgttgccaagctgctgataaagctgcctgcctgttgccaaagctcgatgaacttcgggatgaagggaaggcttcgtctgccaaacagagactcaagtgtgccagtctccaaaaatttggagaaagagctttcaaagcatgggcagtagctcgcctgagccagagatttcccaaagctgagtttgcagaagtttccaagttagtgacagatcttaccaaagtccacacggaatgctgccatggagatctgcttgaatgtgctgatgacagggcggaccttgccaagtatatctgtgaaaatcaagattcgatctccagtaaactgaaggaatgctgtgaaaaacctctgttggaaaaatcccactgcattgccgaagtggaaaatgatgagatgcctgctgacttgccttcattagctgctgattttgttgaaagtaaggatgtttgcaaaaactatgctgaggcaaaggatgtcttcctgggcatgtttttgtatgaatatgcaagaaggcatcctgattactctgtcgtgctgctgctgagacttgccaagacatatgaaaccactctagagaagtgctgtgccgctgcagatcctcatgaatgctatgccaaagtgttcgatgaatttaaacctcttgtggaagagcctcagaatttaatcaaacaaaattgtgagctttttgagcagcttggagagtacaaattccagaatgcgctattagttcgttacaccaagaaagtaccccaagtgtcaactccaactcttgtagaggtctcaagaaacctaggaaaagtgggcagcaaatgttgtaaacatcctgaagcaaaaagaatgccctgtgcagaagactatctatccgtggtcctgaaccagttatgtgtgttgcatgagaaaacgccagtaagtgacagagtcaccaaatgctgcacagaatccttggtgaacaggcgaccatgcttttcagctctggaagtcgatgaaacatacgttcccaaagagtttaatgctgaaacattcaccttccatgcagatatatgcacactttctgagaaggagagacaaatcaagaaacaaactgcacttgttgagctcgtgaaacacaagcccaaggcaacaaaagagcaactgaaagctgttatggatgatttcgcagcttttgtagagaagtgctgcaaggctgacgataaggagacctgctttgccgaggagggtaaaaaacttgttgctgcaagtcaagctgccttaggctta

SEQ ID NO: 5 - protein, 1230 aa, synthetic construct
DAHKSEVAHRFKDLGEENFKALVLIAFAQYLQQCPFEDHVKLVNEVTEFAKTCVADESAENCDKSLHTLFGDKLCTVATLRETYGEMADCCAKQEPERNECFLQHKDDNPNLPRLVRPEVDVMCTAFHDNEETFLKKYLYEIARRHPYFYAPELLFFAKRYKAAFTECCQAADKAACLLPKLDELRDEGKASSAKQRLKCASLQKFGERAFKAWAVARLSQRFPKAEFAEVSKLVTDLTKVHTECCHGDLLECADDRADLAKYICENQDSISSKLKECCEKPLLEKSHCIAEVENDEMPADLPSLAADFVESKDVCKNYAEAKDVFLGMFLYEYARRHPDYSVVLLLRLAKTYETTLEKCCAAADPHECYAKVFDEFKPLVEEPQNLIKQNCELFEQLGEYKFQNALLVRYTKKVPQVSTPTLVEVSRNLGKVGSKCCKHPEAKRMPCAEDYLSVVLNQLCVLHEKTPVSDRVTKCCTESLVNRRPCFSALEVDETYVPKEFNAETFTFHADICTLSEKERQIKKQTALVELVKHKPKATKEQLKAVMDDFAAFVEKCCKADDKETCFAEEGKKLVAASQAALGLGSYVLDDSDGLGREFDGIGAVSGGGATSRLLVNYPEPYRSQILDYLFKPNFGASLHILKVEIGGDGQTTDGTEPSHMHYALDENYFRGYEWWLMKEAKKRNPNITLIGLPWSFPGWLGKGFDWPYVNLQLTAYYVVTWIVGAKRYHDLDIDYIGIWNERSYNANYIKILRKMLNYQGLQRVKIIASDNLWESISASMLLDAELFKVVDVIGAHYPGTHSAKDAKLTGKKLWSSEDFSTLNSDMGAGCWGRILNQNYINGYMTSTIAWNLVASYYEQLPYGRCGLMTAQEPWSGHYVVESPVWVSAHTTQFTQPGWYYLKTVGHLEKGGSYVALTDGLGNLTIIIETMSHKHSKCIRPFLPYFNVSQQFATFVLKGSFSEIPELQVWYTKLGKTSERFLFKQLDSLWLLDSDGSFTLSLHEDELFTLTTLTTGRKGSYPLPPKSQPFPSTYKDDFNVDYPFFSEAPNFADQTGVFEYFTNIEDPGEHHFTLRQVLNQRPITWAADASNTISIIGDYNWTNLTIKCDVYIETPDTGGVFIAGRVNKGGILIRSARGIFFWIFANGSYRVTGDLAGWIIYALGRVEVTAKKWYTLTLTIKGHFTSGMLNDKSLWTDIPVNFPKNGWAAIGTHSFEFAQFDNFLVEATR

SEQ ID NO: 6 - DNA, 3690 bp, synthetic construct
  source 1..3690: mol_type = other DNA
gatgcacacaagagtgaggttgctcatcggtttaaagatttgggagaagaaaatttcaaagccttggtgttgattgcctttgctcagtatcttcagcagtgtccatttgaagatcatgtaaaattagtgaatgaagtaactgaatttgcaaaaacatgtgttgctgatgagtcagctgaaaattgtgacaaatcacttcataccctttttggagacaaattatgcacagttgcaactcttcgtgaaacctatggtgaaatggctgactgctgtgcaaaacaagaacctgagagaaatgaatgcttcttgcaacacaaagatgacaacccaaacctcccccgattggtgagaccagaggttgatgtgatgtgcactgcttttcatgacaatgaagagacatttttgaaaaaatacttatatgaaattgccagaagacatccttacttttatgccccggaactccttttctttgctaaaaggtataaagctgcttttacagaatgttgccaagctgctgataaagctgcctgcctgttgccaaagctcgatgaacttcgggatgaagggaaggcttcgtctgccaaacagagactcaagtgtgccagtctccaaaaatttggagaaagagctttcaaagcatgggcagtagctcgcctgagccagagatttcccaaagctgagtttgcagaagtttccaagttagtgacagatcttaccaaagtccacacggaatgctgccatggagatctgcttgaatgtgctgatgacagggcggaccttgccaagtatatctgtgaaaatcaagattcgatctccagtaaactgaaggaatgctgtgaaaaacctctgttggaaaaatcccactgcattgccgaagtggaaaatgatgagatgcctgctgacttgccttcattagctgctgattttgttgaaagtaaggatgtttgcaaaaactatgctgaggcaaaggatgtcttcctgggcatgtttttgtatgaatatgcaagaaggcatcctgattactctgtcgtgctgctgctgagacttgccaagacatatgaaaccactctagagaagtgctgtgccgctgcagatcctcatgaatgctatgccaaagtgttcgatgaatttaaacctcttgtggaagagcctcagaatttaatcaaacaaaattgtgagctttttgagcagcttggagagtacaaattccagaatgcgctattagttcgttacaccaagaaagtaccccaagtgtcaactccaactcttgtagaggtctcaagaaacctaggaaaagtgggcagcaaatgttgtaaacatcctgaagcaaaaagaatgccctgtgcagaagactatctatccgtggtcctgaaccagttatgtgtgttgcatgagaaaacgccagtaagtgacagagtcaccaaatgctgcacagaatccttggtgaacaggcgaccatgcttttcagctctggaagtcgatgaaacatacgttcccaaagagtttaatgctgaaacattcaccttccatgcagatatatgcacactttctgagaaggagagacaaatcaagaaacaaactgcacttgttgagctcgtgaaacacaagcccaaggcaacaaaagagcaactgaaagctgttatggatgatttcgcagcttttgtagagaagtgctgcaaggctgacgataaggagacctgctttgccgaggagggtaaaaaacttgttgctgcaagtcaagctgccttaggcttaggatcctacgtgctggacgactctgacggactcggaagggagtttgacggcattggcgctgtgtccggaggcggcgctacatctcgtctgctggtgaattatcccgagccctaccggtcccagattttagactacctcttcaaacccaattttggagcctccctccacattttaaaggtggaaatcggcggcgacggacagacaaccgatggcaccgaacctagccatatgcactacgctttagacgagaactatttccggggctatgagtggtggctgatgaaggaggccaagaagaggaaccccaacattaccctcatcggactgccttggagctttcccggttggctgggcaaaggattcgactggccctacgtgaatttacagctgaccgcttactacgtggtgacttggattgtgggagccaagcggtaccacgatctcgacatcgattacattggcatctggaacgagcggagctacaacgctaactatatcaagattctgcggaaaatgctgaattaccaaggtttacagcgggtgaagatcatcgctagcgacaatttatgggaaagcatctccgctagcatgctgctggacgctgaactgttcaaagtcgtggatgtcatcggcgctcactatcccggcacccatagcgccaaggacgccaagctgaccggaaaaaagctgtggtccagcgaggatttcagcactttaaactccgatatgggagctggctgctggggccggattttaaaccagaactacatcaatggctacatgacaagcaccatcgcttggaatttagtggcctcctactacgagcagctgccctatggacggtgcggtttaatgacagcccaagagccttggagcggccattacgtggtggagagccccgtttgggtgagcgctcacaccacccagttcacccagcccggctggtactacctcaagaccgtcggacatctggagaagggcggctcctacgtggctttaactgatggtttaggcaatctgaccatcattatcgagaccatgtcccacaagcactccaagtgcatccggccctttctgccctacttcaacgtgtcccagcaattcgccacctttgtgctgaagggcagcttttccgagattcccgagctccaagtttggtacaccaagctgggaaaaaccagcgagaggtttttattcaagcaactggactctttatggctgctggacagcgatggctccttcacactgtctttacatgaggatgagctctttactttaaccactttaacaactggtcggaaaggctcctatcctttaccccccaagagccaacccttccccagcacctacaaggacgacttcaacgtggattaccccttcttctccgaggctcccaactttgctgaccagaccggcgtgttcgagtatttcaccaacatcgaggaccccggtgagcaccatttcaccctccggcaagttctgaaccaacggcctatcacttgggccgccgacgcttccaataccatctccattatcggcgactacaactggacaaatttaactatcaagtgcgacgtctacatcgagacccccgataccggaggcgtgtttatcgctggaagggtgaacaaaggcggcattttaatccggtccgctaggggcatctttttctggatcttcgctaacggcagctatcgggtgactggtgacctcgctggctggatcatttacgctctgggccgggtggaggtgacagccaagaagtggtacactttaactttaactattaagggacattttaccagcggcatgctgaacgacaaatctttatggaccgacatccccgtgaactttcccaagaatggctgggccgccatcggcacccattcctttgaattcgcccagttcgacaatttcctcgtggaagccacccgg

SEQ ID NO: 7 - protein, 1230 aa, synthetic construct
YVLDDSDGLGREFDGIGAVSGGGATSRLLVNYPEPYRSQILDYLFKPNFGASLHILKVEIGGDGQTTDGTEPSHMHYALDENYFRGYEWWLMKEAKKRNPNITLIGLPWSFPGWLGKGFDWPYVNLQLTAYYVVTWIVGAKRYHDLDIDYIGIWNERSYNANYIKILRKMLNYQGLQRVKIIASDNLWESISASMLLDAELFKVVDVIGAHYPGTHSAKDAKLTGKKLWSSEDFSTLNSDMGAGCWGRILNQNYINGYMTSTIAWNLVASYYEQLPYGRCGLMTAQEPWSGHYVVESPVWVSAHTTQFTQPGWYYLKTVGHLEKGGSYVALTDGLGNLTIIIETMSHKHSKCIRPFLPYFNVSQQFATFVLKGSFSEIPELQVWYTKLGKTSERFLFKQLDSLWLLDSDGSFTLSLHEDELFTLTTLTTGRKGSYPLPPKSQPFPSTYKDDFNVDYPFFSEAPNFADQTGVFEYFTNIEDPGEHHFTLRQVLNQRPITWAADASNTISIIGDYNWTNLTIKCDVYIETPDTGGVFIAGRVNKGGILIRSARGIFFWIFANGSYRVTGDLAGWIIYALGRVEVTAKKWYTLTLTIKGHFTSGMLNDKSLWTDIPVNFPKNGWAAIGTHSFEFAQFDNFLVEATRGSDAHKSEVAHRFKDLGEENFKALVLIAFAQYLQQCPFEDHVKLVNEVTEFAKTCVADESAENCDKSLHTLFGDKLCTVATLRETYGEMADCCAKQEPERNECFLQHKDDNPNLPRLVRPEVDVMCTAFHDNEETFLKKYLYEIARRHPYFYAPELLFFAKRYKAAFTECCQAADKAACLLPKLDELRDEGKASSAKQRLKCASLQKFGERAFKAWAVARLSQRFPKAEFAEVSKLVTDLTKVHTECCHGDLLECADDRADLAKYICENQDSISSKLKECCEKPLLEKSHCIAEVENDEMPADLPSLAADFVESKDVCKNYAEAKDVFLGMFLYEYARRHPDYSVVLLLRLAKTYETTLEKCCAAADPHECYAKVFDEFKPLVEEPQNLIKQNCELFEQLGEYKFQNALLVRYTKKVPQVSTPTLVEVSRNLGKVGSKCCKHPEAKRMPCAEDYLSVVLNQLCVLHEKTPVSDRVTKCCTESLVNRRPCFSALEVDETYVPKEFNAETFTFHADICTLSEKERQIKKQTALVELVKHKPKATKEQLKAVMDDFAAFVEKCCKADDKETCFAEEGKKLVAASQAALGL

SEQ ID NO: 8 - DNA, 3690 bp, synthetic construct
  source 1..3690: mol_type = other DNA
tacgtgctggacgactctgacggactcggaagggagtttgacggcattggcgctgtgtccggaggcggcgctacatctcgtctgctggtgaattatcccgagccctaccggtcccagattttagactacctcttcaaacccaattttggagcctccctccacattttaaaggtggaaatcggcggcgacggacagacaaccgatggcaccgaacctagccatatgcactacgctttagacgagaactatttccggggctatgagtggtggctgatgaaggaggccaagaagaggaaccccaacattaccctcatcggactgccttggagctttcccggttggctgggcaaaggattcgactggccctacgtgaatttacagctgaccgcttactacgtggtgacttggattgtgggagccaagcggtaccacgatctcgacatcgattacattggcatctggaacgagcggagctacaacgctaactatatcaagattctgcggaaaatgctgaattaccaaggtttacagcgggtgaagatcatcgctagcgacaatttatgggaaagcatctccgctagcatgctgctggacgctgaactgttcaaagtcgtggatgtcatcggcgctcactatcccggcacccatagcgccaaggacgccaagctgaccggaaaaaagctgtggtccagcgaggatttcagcactttaaactccgatatgggagctggctgctggggccggattttaaaccagaactacatcaatggctacatgacaagcaccatcgcttggaatttagtggcctcctactacgagcagctgccctatggacggtgcggtttaatgacagcccaagagccttggagcggccattacgtggtggagagccccgtttgggtgagcgctcacaccacccagttcacccagcccggctggtactacctcaagaccgtcggacatctggagaagggcggctcctacgtggctttaactgatggtttaggcaatctgaccatcattatcgagaccatgtcccacaagcactccaagtgcatccggccctttctgccctacttcaacgtgtcccagcaattcgccacctttgtgctgaagggcagcttttccgagattcccgagctccaagtttggtacaccaagctgggaaaaaccagcgagaggtttttattcaagcaactggactctttatggctgctggacagcgatggctccttcacactgtctttacatgaggatgagctctttactttaaccactttaacaactggtcggaaaggctcctatcctttaccccccaagagccaacccttccccagcacctacaaggacgacttcaacgtggattaccccttcttctccgaggctcccaactttgctgaccagaccggcgtgttcgagtatttcaccaacatcgaggaccccggtgagcaccatttcaccctccggcaagttctgaaccaacggcctatcacttgggccgccgacgcttccaataccatctccattatcggcgactacaactggacaaatttaactatcaagtgcgacgtctacatcgagacccccgataccggaggcgtgtttatcgctggaagggtgaacaaaggcggcattttaatccggtccgctaggggcatctttttctggatcttcgctaacggcagctatcgggtgactggtgacctcgctggctggatcatttacgctctgggccgggtggaggtgacagccaagaagtggtacactttaactttaactattaagggacattttaccagcggcatgctgaacgacaaatctttatggaccgacatccccgtgaactttcccaagaatggctgggccgccatcggcacccattcctttgaattcgcccagttcgacaatttcctcgtggaagccacccggggatccgatgcacacaagagtgaggttgctcatcggtttaaagatttgggagaagaaaatttcaaagccttggtgttgattgcctttgctcagtatcttcagcagtgtccatttgaagatcatgtaaaattagtgaatgaagtaactgaatttgcaaaaacatgtgttgctgatgagtcagctgaaaattgtgacaaatcacttcataccctttttggagacaaattatgcacagttgcaactcttcgtgaaacctatggtgaaatggctgactgctgtgcaaaacaagaacctgagagaaatgaatgcttcttgcaacacaaagatgacaacccaaacctcccccgattggtgagaccagaggttgatgtgatgtgcactgcttttcatgacaatgaagagacatttttgaaaaaatacttatatgaaattgccagaagacatccttacttttatgccccggaactccttttctttgctaaaaggtataaagctgcttttacagaatgttgccaagctgctgataaagctgcctgcctgttgccaaagctcgatgaacttcgggatgaagggaaggcttcgtctgccaaacagagactcaagtgtgccagtctccaaaaatttggagaaagagctttcaaagcatgggcagtagctcgcctgagccagagatttcccaaagctgagtttgcagaagtttccaagttagtgacagatcttaccaaagtccacacggaatgctgccatggagatctgcttgaatgtgctgatgacagggcggaccttgccaagtatatctgtgaaaatcaagattcgatctccagtaaactgaaggaatgctgtgaaaaacctctgttggaaaaatcccactgcattgccgaagtggaaaatgatgagatgcctgctgacttgccttcattagctgctgattttgttgaaagtaaggatgtttgcaaaaactatgctgaggcaaaggatgtcttcctgggcatgtttttgtatgaatatgcaagaaggcatcctgattactctgtcgtgctgctgctgagacttgccaagacatatgaaaccactctagagaagtgctgtgccgctgcagatcctcatgaatgctatgccaaagtgttcgatgaatttaaacctcttgtggaagagcctcagaatttaatcaaacaaaattgtgagctttttgagcagcttggagagtacaaattccagaatgcgctattagttcgttacaccaagaaagtaccccaagtgtcaactccaactcttgtagaggtctcaagaaacctaggaaaagtgggcagcaaatgttgtaaacatcctgaagcaaaaagaatgccctgtgcagaagactatctatccgtggtcctgaaccagttatgtgtgttgcatgagaaaacgccagtaagtgacagagtcaccaaatgctgcacagaatccttggtgaacaggcgaccatgcttttcagctctggaagtcgatgaaacatacgttcccaaagagtttaatgctgaaacattcaccttccatgcagatatatgcacactttctgagaaggagagacaaatcaagaaacaaactgcacttgttgagctcgtgaaacacaagcccaaggcaacaaaagagcaactgaaagctgttatggatgatttcgcagcttttgtagagaagtgctgcaaggctgacgataaggagacctgctttgccgaggagggtaaaaaacttgttgctgcaagtcaagctgccttaggctta

SEQ ID NO: 9 - protein, 5 aa, synthetic construct
GGGGS

SEQ ID NO: 10 - protein, 6 aa, synthetic construct
GGGGGS

SEQ ID NO: 11 - protein, 5 aa, synthetic construct
SGGGG

SEQ ID NO: 12 - protein, 586 aa, Homo sapiens
RDAHKSEVAHRFKDLGEENFKALVLIAFAQYLQQCPFEDHVKLVNEVTEFAKTCVADESAENCDKSLHTLFGDKLCTVATLRETYGEMADCCAKQEPERNECFLQHKDDNPNLPRLVRPEVDVMCTAFHDNEETFLKKYLYEIARRHPYFYAPELLFFAKRYKAAFTECCQAADKAACLLPKLDELRDEGKASSAKQRLKCASLQKFGERAFKAWAVARLSQRFPKAEFAEVSKLVTDLTKVHTECCHGDLLECADDRADLAKYICENQDSISSKLKECCEKPLLEKSHCIAEVENDEMPADLPSLAADFVESKDVCKNYTEAKDVFLGMFLYEYARRHPDYSVVLLLRLAKTYETTLEKCCAAADPHECYAKVFDEFKPLVEEPQNLIKQNCELFEQLGEYKFQNALLVRYTKKVPQVSTPTLVEVSRNLGKVGSKCCKHPEAKRMPCAEDYLSVVLNQLCVLHEKTPVSDRVTKCCTESLVNRRPCFSALEVDETYVPKEFNAETFTFHADICTLSEKERQIKKQTALVELVKHKPKATKEQLKAVMDDFAAFVEKCCKADDKETCFAEEGKKLVAASQAALGL

SEQ ID NO: 13 - protein, 585 aa, synthetic construct
DAHKSEVAHRFKDLGEENFKALVLIAFAQYLQQCPFEDHVKLVNEVTEFAKTCVADESAENCDKSLHTLFGDKLCTVATLRETYGEMADCCAKQEPERNECFLQHKDDNPNLPRLVRPEVDVMCTAFHDNEETFLKKYLYEIARRHPYFYAPELLFFAKRYKAAFTECCQAADKAACLLPKLDELRDEGKASSAKQRLKCASLQKFGERAFKAWAVARLSQRFPKAEFAEVSKLVTDLTKVHTECCHGDLLECADDRADLAKYICENQDSISSKLKECCEKPLLEKSHCIAEVENDEMPADLPSLAADFVESKDVCKNYTEAKDVFLGMFLYEYARRHPDYSVVLLLRLAKTYETTLEKCCAAADPHECYAKVFDEFKPLVEEPQNLIKQNCELFEQLGEYKFQNALLVRYTKKVPQVSTPTLVEVSRNLGKVGSKCCKHPEAKRMPCAEDYLSVVLNQLCVLHEKTPVSDRVTKCCTESLVNRRPCFSALEVDETYVPKEFNAETFTFHADICTLSEKERQIKKQTALVELVKHKPKATKEQLKAVMDDFAAFVEKCCKADDKETCFAEEGKKLVAASQAALGL

SEQ ID NO: 14 - protein, 642 aa, Mus musculus
YVLDDSDGLGREFDGIGAVSGGGATSRLLVNYPEPYRSEILDYLFKPNFGASLHILKVEIGGDGQTTDGTEPSHMHYELDENYFRGYEWWLMKEAKKRNPDIILMGLPWSFPGWLGKGFSWPYVNLQLTAYYVVRWILGAKHYHDLDIDYIGIWNERPFDANYIKELRKMLDYQGLQRVRIIASDNLWEPISSSLLLDQELWKVVDVIGAHYPGTYTVWNAKMSGKKLWSSEDFSTINSNVGAGCWSRILNQNYINGNMTSTIAWNLVASYYEELPYGRSGLMTAQEPWSGHYVVASPIWVSAHTTQFTQPGWYYLKTVGHLEKGGSYVALTDGLGNLTIIIETMSHQHSMCIRPYLPYYNVSHQLATFTLKGSLREIQELQVWYTKLGTPQQRLHFKQLDTLWLLDGSGSFTLELEEDEIFTLTTLTTGRKGSYPPPPSSKPFPTNYKDDFNVEYPLFSEAPNFADQTGVFEYYMNNEDREHRFTLRQVLNQRPITWAADASSTISVIGDHHWTNMTVQCDVYIETPRSGGVFIAGRVNKGGILIRSATGVFFWIFANGSYRVTADLGGWITYASGHADVTAKRWYTLTLGIKGYFAFGMLNGTILWKNVRVKYPGHGWAAIGTHTFEFAQFDNFRVEAAR

SEQ ID NO: 15 - DNA, 1926 bp, synthetic construct
  source 1..1926: mol_type = other DNA
tacgttttagacgatagcgatggcctcggccgggaattcgatggaatcggcgctgtgagcggcggaggagctacatcccggctgctcgtgaactaccccgagccctaccggtccgagattttagactatttatttaagcccaactttggagcttctttacacattttaaaggtggaaattggcggcgatggacagaccaccgacggcaccgagcctagccacatgcactacgagctggacgagaactacttccggggatatgagtggtggctcatgaaggaggccaagaagaggaaccccgatatcattctcatgggtttaccttggtcctttcccggttggctcggcaaaggcttctcttggccttacgtcaatctgcagctgacagcctactacgtggtgaggtggattttaggagctaaacactaccacgatttagatatcgactacatcggcatctggaacgagcggcccttcgacgccaactacatcaaggagctgcggaagatgctcgactaccaaggtttacagagggtgcggatcatcgcttccgataatttatgggagcctatctccagctctttactgctcgatcaagaactgtggaaggtggtggacgtgatcggcgctcactaccccggcacctacaccgtgtggaacgccaagatgtccggcaaaaagctctggtcctccgaggatttttccaccatcaacagcaacgtgggcgctggatgctggtcccggattttaaaccagaattatatcaatggcaatatgacctccaccatcgcttggaatctggtggcttcctactatgaggagctgccctatggaaggtccggactgatgaccgcccaagaaccttggtccggccattacgtcgtggctagccctatctgggtgtccgcccacaccacccagttcacacagcccggatggtactatttaaagaccgtgggccatctggaaaaaggcggaagctatgtggctttaacagacggtttaggaaatttaaccatcatcatcgagaccatgagccaccagcattccatgtgtattcgtccctatctgccctactacaacgtgtcccaccagctggccacattcactttaaagggatctttaagggagatccaagaactgcaagtgtggtataccaagctcggaaccccccagcaacggctgcacttcaagcagctggatactttatggctgctggacggcagcggaagcttcactttagagctggaggaggatgaaatttttactttaaccacactgaccaccggacggaaaggctcctatcccccccccccttccagcaagcctttccccaccaactataaggacgacttcaatgtcgagtaccctttattttccgaagctcccaacttcgctgatcagaccggcgtcttcgagtactacatgaacaacgaggaccgggagcatcggttcacactgaggcaagttctgaaccaacggcccatcacttgggccgctgacgcttcctccaccatctccgtcatcggagaccaccactggacaaacatgaccgtgcagtgcgatgtctacatcgaaaccccccggagcggaggcgtgttcattgccggtcgtgtgaacaagggcggcattctgatccggtccgccactggtgtcttcttctggatctttgccaacggaagctatcgtgtcaccgccgatttaggaggatggatcacctacgccagcggccatgccgatgtgacagccaagaggtggtacacactcacactgggcatcaagggatacttcgccttcggaatgctgaacggcacaatcctctggaagaacgtgcgggtcaaataccccggccacggctgggctgctatcggcacacacacctttgagttcgcccagtttgacaattttcgggtggaggccgctagg

SEQ ID NO: 16 - protein, 584 aa, Mus musculus
EAHKSEIAHRYNDLGEQHFKGLVLIAFSQYLQKCSYDEHAKLVQEVTDFAKTCVADESAANCDKSLHTLFGDKLCAIPNLRENYGELADCCTKQEPERNECFLQHKDDNPSLPPFERPEAEAMCTSFKENPTTFMGHYLHEVARRHPYFYAPELLYYAEQYNEILTQCCAEADKESCLTPKLDGVKEKALVSSVRQRMKCSSMQKFGERAFKAWAVARLSQTFPNADFAEITKLATDLTKVNKECCHGDLLECADDRAELAKYMCENQATISSKLQTCCDKPLLKKAHCLSEVEHDTMPADLPAIAADFVEDQEVCKNYAEAKDVFLGTFLYEYSRRHPDYSVSLLLRLAKKYEATLEKCCAEANPPACYGTVLAEFQPLVEEPKNLVKTNCDLYEKLGEYGFQNAILVRYTQKAPQVSTPTLVEAARNLGRVGTKCCTLPEDQRLPCVEDYLSAILNRVCLLHEKTPVSEHVTKCCSGSLVERRPCFSALTVDETYVPKEFKAETFTFHSDICTLPEKEKQIKKQTALAELVKHKPKATAEQLKTVMDDFAQFLDTCCKAADKDTCFSTEGPNLVTRCKDALA

SEQ ID NO: 17 - DNA, 1752 bp, synthetic construct
  source 1..1752: mol_type = other DNA
gaggctcacaagagcgaaatcgctcatcgttacaacgatttaggcgagcagcacttcaagggtttagttttaatcgctttctcccagtacctccagaagtgctcctacgacgagcatgccaagctcgtgcaagaggtgaccgactttgctaagacttgtgtggccgatgagtccgccgctaactgcgataagtctttacacaccctctttggagacaaactgtgcgccatccctaatctgcgggagaactacggcgagctggccgattgctgcacaaagcaagaacccgaaaggaacgagtgtttcctccagcacaaagacgacaacccttctttacctccctttgagaggcccgaggccgaggctatgtgtacctccttcaaggaaaaccccacaacattcatgggacattatttacatgaggtcgctcggcggcacccttacttctacgcccccgagctgctgtattacgccgagcagtacaacgagattctgacccagtgttgtgccgaagctgataaagagagctgtttaacacccaagctggatggcgtgaaggaaaaggctttagtcagcagcgtgaggcagaggatgaaatgctcctccatgcaaaagttcggcgaacgggcctttaaggcttgggctgtggctcgtctgagccagacattccccaacgccgacttcgccgagattaccaaactcgccaccgatctgacaaaggtcaacaaggagtgctgccatggtgatttactggagtgcgccgacgatagggccgaactcgctaaatacatgtgcgagaaccaagctaccatctccagcaagctgcagacttgttgtgataaacccctcctcaagaaggctcactgtttatccgaggtcgagcacgacacaatgcccgctgatctgcccgctatcgccgctgattttgtggaagaccaagaagtctgtaagaattacgctgaggctaaggatgtgtttctcggcacctttttatacgaatatagccggaggcaccccgattatagcgtcagcctcttattacggctggctaagaagtatgaggccacactggaaaagtgctgtgccgaggctaaccctcccgcttgttacggaaccgtgctggctgaatttcagcctttagtcgaggagcccaagaatctggtgaagaccaactgtgatctgtacgaaaagctgggcgagtatggcttccaaaacgccattttagtgcggtatacacagaaggccccccaagtttccacccccacactggtcgaagctgcccggaatctgggacgggtgggcaccaagtgttgcactttacccgaggaccagaggctgccttgcgtggaggactacctcagcgctatcctcaatcgtgtctgtttactgcacgaaaagacacccgttagcgaacacgtgacaaagtgctgctccggctctttagtggaacggaggccttgctttagcgctttaacagtggacgaaacctacgtgcctaaggagtttaaggccgagaccttcacctttcactccgacatctgcactttacccgaaaaagagaagcagatcaaaaagcagaccgccctcgccgagctcgtcaaacataagcctaaggctaccgccgaacagctcaaaaccgtgatggacgacttcgcccaatttttagatacatgctgcaaggccgccgacaaggacacttgtttttccaccgagggccccaatttagtcactcgttgcaaggatgctttagct

SEQ ID NO: 18 - protein, 1228 aa, synthetic construct
EAHKSEIAHRYNDLGEQHFKGLVLIAFSQYLQKCSYDEHAKLVQEVTDFAKTCVADESAANCDKSLHTLFGDKLCAIPNLRENYGELADCCTKQEPERNECFLQHKDDNPSLPPFERPEAEAMCTSFKENPTTFMGHYLHEVARRHPYFYAPELLYYAEQYNEILTQCCAEADKESCLTPKLDGVKEKALVSSVRQRMKCSSMQKFGERAFKAWAVARLSQTFPNADFAEITKLATDLTKVNKECCHGDLLECADDRAELAKYMCENQATISSKLQTCCDKPLLKKAHCLSEVEHDTMPADLPAIAADFVEDQEVCKNYAEAKDVFLGTFLYEYSRRHPDYSVSLLLRLAKKYEATLEKCCAEANPPACYGTVLAEFQPLVEEPKNLVKTNCDLYEKLGEYGFQNAILVRYTQKAPQVSTPTLVEAARNLGRVGTKCCTLPEDQRLPCVEDYLSAILNRVCLLHEKTPVSEHVTKCCSGSLVERRPCFSALTVDETYVPKEFKAETFTFHSDICTLPEKEKQIKKQTALAELVKHKPKATAEQLKTVMDDFAQFLDTCCKAADKDTCFSTEGPNLVTRCKDALAGSYVLDDSDGLGREFDGIGAVSGGGATSRLLVNYPEPYRSEILDYLFKPNFGASLHILKVEIGGDGQTTDGTEPSHMHYELDENYFRGYEWWLMKEAKKRNPDIILMGLPWSFPGWLGKGFSWPYVNLQLTAYYVVRWILGAKHYHDLDIDYIGIWNERPFDANYIKELRKMLDYQGLQRVRIIASDNLWEPISSSLLLDQELWKVVDVIGAHYPGTYTVWNAKMSGKKLWSSEDFSTINSNVGAGCWSRILNQNYINGNMTSTIAWNLVASYYEELPYGRSGLMTAQEPWSGHYVVASPIWVSAHTTQFTQPGWYYLKTVGHLEKGGSYVALTDGLGNLTIIIETMSHQHSMCIRPYLPYYNVSHQLATFTLKGSLREIQELQVWYTKLGTPQQRLHFKQLDTLWLLDGSGSFTLELEEDEIFTLTTLTTGRKGSYPPPPSSKPFPTNYKDDFNVEYPLFSEAPNFADQTGVFEYYMNNEDREHRFTLRQVLNQRPITWAADASSTISVIGDHHWTNMTVQCDVYIETPRSGGVFIAGRVNKGGILIRSATGVFFWIFANGSYRVTADLGGWITYASGHADVTAKRWYTLTLGIKGYFAFGMLNGTILWKNVRVKYPGHGWAAIGTHTFEFAQFDNFRVEAAR

SEQ ID NO: 19 - DNA, 3682 bp, synthetic construct
  source 1..3682: mol_type = other DNA
gaggctcacaagagcgaaatcgctcatcgttacaacgatttaggcgagcagcacttcaagggtttagttttaatcgctttctcccagtacctccagaagtgctcctacgacgagcatgccaagctcgtgcaagaggtgaccgactttgctaagacttgtgtggccgatgagtccgccgctaactgcgataagtctttacacaccctctttggagacaaactgtgcgccatccctaatctgcgggagaactacggcgagctggccgattgctgcacaaagcaagaacccgaaaggaacgagtgtttcctccagcacaaagacgacaacccttctttacctccctttgagaggcccgaggccgaggctatgtgtacctccttcaaggaaaaccccacaacattcatgggacattatttacatgaggtcgctcggcggcacccttacttctacgcccccgagctgctgtattacgccgagcagtacaacgagattctgacccagtgttgtgccgaagctgataaagagagctgtttaacacccaagctggatggcgtgaaggaaaaggctttagtcagcagcgtgaggcagaggatgaaatgctcctccatgcaaaagttcggcgaacgggcctttaaggcttgggctgtggctcgtctgagccagacattccccaacgccgacttcgccgagattaccaaactcgccaccgatctgacaaaggtcaacaaggagtgctgccatggtgatttactggagtgcgccgacgatagggccgaactcgctaaatacatgtgcgagaaccaagctaccatctccagcaagctgcagacttgttgtgataaacccctcctcaagaaggctcactgtttatccgaggtcgagcacgacacaatgcccgctgatctgcccgctatcgccgctgattttgtggaagaccaagaagtctgtaagaattacgctgaggctaaggatgtgtttctcggcacctttttatacgaatatagccggaggcaccccgattatagcgtcagcctcttattacggctggctaagaagtatgaggccacactggaaaagtgctgtgccgaggctaaccctcccgcttgttacggaaccgtgctggctgaatttcagcctttagtcgaggagcccaagaatctggtgaagaccaactgtgatctgtacgaaaagctgggcgagtatggcttccaaaacgccattttagtgcggtatacacagaaggccccccaagtttccacccccacactggtcgaagctgcccggaatctgggacgggtgggcaccaagtgttgcactttacccgaggaccagaggctgccttgcgtggaggactacctcagcgctatcctcaatcgtgtctgtttactgcacgaaaagacacccgttagcgaacacgtgacaaagtgctgctccggctctttagtggaacggaggccttgctttagcgctttaacagtggacgaaacctacgtgcctaaggagtttaaggccgagaccttcacctttcactccgacatctgcactttacccgaaaaagagaagcagatcaaaaagcagaccgccctcgccgagctcgtcaaacataagcctaaggctaccgccgaacagctcaaaaccgtgatggacgacttcgcccaatttttagatacatgctgcaaggccgccgacaaggacacttgtttttccaccgagggccccaatttagtcactcgttgcaaggatgctttagctggatcctacgttttagacgatagcgatggcctcggccgggaattcgatggaatcggcgctgtgagcggcggaggagctacatcccggctgctcgtgaactaccccgagccctaccggtccgagattttagactatttatttaagcccaactttggagcttctttacacattttaaaggtggaaattggcggcgatggacagaccaccgacggcaccgagcctagccacatgcactacgagctggacgagaactacttccggggatatgagtggtggctcatgaaggaggccaagaagaggaaccccgatatcattctcatgggtttaccttggtcctttcccggttggctcggcaaaggcttctcttggccttacgtcaatctgcagctgacagcctactacgtggtgaggtggattttaggagctaaacactaccacgatttagatatcgactacatcggcatctggaacgagcggcccttcgacgccaactacatcaaggagctgcggaagatgctcgactaccaaggtttacagagggtgcggatcatcgcttccgataatttatgggagcctatctccagctctttactgctcgatcaagaactgtggaaggtggtggacgtgatcggcgctcactaccccggcacctacaccgtgtggaacgccaagatgtccggcaaaaagctctggtcctccgaggatttttccaccatcaacagcaacgtgggcgctggatgctggtcccggattttaaaccagaattatatcaatggcaatatgacctccaccatcgcttggaatctggtggcttcctactatgaggagctgccctatggaaggtccggactgatgaccgcccaagaaccttggtccggccattacgtcgtggctagccctatctgggtgtccgcccacaccacccagttcacacagcccggatggtactatttaaagaccgtgggccatctggaaaaaggcggaagctatgtggctttaacagacggtttaggaaatttaaccatcatcatcgagaccatgagccaccagcattccatgtgtattcgtccctatctgccctactacaacgtgtcccaccagctggccacattcactttaaagggatctttaagggagatccaagaactgcaagtgtggtataccaagctcggaaccccccagcaacggctgcacttcaagcagctggatactttatggctgctggacggcagcggaagcttcactttagagctggaggaggatgaaatttttactttaaccacactgaccaccggacggaaaggctcctatcccccccccccttccagcaagcctttccccaccaactataaggacgacttcaatgtcgagtaccctttattttccgaagctcccaacttcgctgatcagaccggcgtcttcgagtactacatgaacaacgaggaccgggagcatcggttcacactgaggcaagttctgaaccaacggcccatcacttgggccgctgacgcttcctccaccatctccgtcatcggagaccaccactggacaaacatgaccgtgcagtgcgatgtctacatcgaaaccccccggagcggaggcgtgttcattgccggtcgtgtgaacaagggcggcattctgatccggtccgccactggtgtcttcttctggatcttccaacggaagctatcgtgtcaccgccgatttaggaggatggatcacctacgccagcggccatgccgatgtgacagccaagaggtggtacacactcacactgggcatcaagggatacttcgccttcggaatgctgaacggcacaatcctctggaagaacgtgcgggtcaaataccccggccacggctgggctgctatcggcacacacacctttgagttcgcccagtttgacaattttcgggtggaggccgctagg

SEQ ID NO: 20 - protein, 1228 aa, synthetic construct
YVLDDSDGLGREFDGIGAVSGGGATSRLLVNYPEPYRSEILDYLFKPNFGASLHILKVEIGGDGQTTDGTEPSHMHYELDENYFRGYEWWLMKEAKKRNPDIILMGLPWSFPGWLGKGFSWPYVNLQLTAYYVVRWILGAKHYHDLDIDYIGIWNERPFDANYIKELRKMLDYQGLQRVRIIASDNLWEPISSSLLLDQELWKVVDVIGAHYPGTYTVWNAKMSGKKLWSSEDFSTINSNVGAGCWSRILNQNYINGNMTSTIAWNLVASYYEELPYGRSGLMTAQEPWSGHYVVASPIWVSAHTTQFTQPGWYYLKTVGHLEKGGSYVALTDGLGNLTIIIETMSHQHSMCIRPYLPYYNVSHQLATFTLKGSLREIQELQVWYTKLGTPQQRLHFKQLDTLWLLDGSGSFTLELEEDEIFTLTTLTTGRKGSYPPPPSSKPFPTNYKDDFNVEYPLFSEAPNFADQTGVFEYYMNNEDREHRFTLRQVLNQRPITWAADASSTISVIGDHHWTNMTVQCDVYIETPRSGGVFIAGRVNKGGILIRSATGVFFWIFANGSYRVTADLGGWITYASGHADVTAKRWYTLTLGIKGYFAFGMLNGTILWKNVRVKYPGHGWAAIGTHTFEFAQFDNFRVEAARGSEAHKSEIAHRYNDLGEQHFKGLVLIAFSQYLQKCSYDEHAKLVQEVTDFAKTCVADESAANCDKSLHTLFGDKLCAIPNLRENYGELADCCTKQEPERNECFLQHKDDNPSLPPFERPEAEAMCTSFKENPTTFMGHYLHEVARRHPYFYAPELLYYAEQYNEILTQCCAEADKESCLTPKLDGVKEKALVSSVRQRMKCSSMQKFGERAFKAWAVARLSQTFPNADFAEITKLATDLTKVNKECCHGDLLECADDRAELAKYMCENQATISSKLQTCCDKPLLKKAHCLSEVEHDTMPADLPAIAADFVEDQEVCKNYAEAKDVFLGTFLYEYSRRHPDYSVSLLLRLAKKYEATLEKCCAEANPPACYGTVLAEFQPLVEEPKNLVKTNCDLYEKLGEYGFQNAILVRYTQKAPQVSTPTLVEAARNLGRVGTKCCTLPEDQRLPCVEDYLSAILNRVCLLHEKTPVSEHVTKCCSGSLVERRPCFSALTVDETYVPKEFKAETFTFHSDICTLPEKEKQIKKQTALAELVKHKPKATAEQLKTVMDDFAQFLDTCCKAADKDTCFSTEGPNLVTRCKDALA

SEQ ID NO: 21 - DNA, 3684 bp, synthetic construct
  source 1..3684: mol_type = other DNA
tacgttttagacgatagcgatggcctcggccgggaattcgatggaatcggcgctgtgagcggcggaggagctacatcccggctgctcgtgaactaccccgagccctaccggtccgagattttagactatttatttaagcccaactttggagcttctttacacattttaaaggtggaaattggcggcgatggacagaccaccgacggcaccgagcctagccacatgcactacgagctggacgagaactacttccggggatatgagtggtggctcatgaaggaggccaagaagaggaaccccgatatcattctcatgggtttaccttggtcctttcccggttggctcggcaaaggcttctcttggccttacgtcaatctgcagctgacagcctactacgtggtgaggtggattttaggagctaaacactaccacgatttagatatcgactacatcggcatctggaacgagcggcccttcgacgccaactacatcaaggagctgcggaagatgctcgactaccaaggtttacagagggtgcggatcatcgcttccgataatttatgggagcctatctccagctctttactgctcgatcaagaactgtggaaggtggtggacgtgatcggcgctcactaccccggcacctacaccgtgtggaacgccaagatgtccggcaaaaagctctggtcctccgaggatttttccaccatcaacagcaacgtgggcgctggatgctggtcccggattttaaaccagaattatatcaatggcaatatgacctccaccatcgcttggaatctggtggcttcctactatgaggagctgccctatggaaggtccggactgatgaccgcccaagaaccttggtccggccattacgtcgtggctagccctatctgggtgtccgcccacaccacccagttcacacagcccggatggtactatttaaagaccgtgggccatctggaaaaaggcggaagctatgtggctttaacagacggtttaggaaatttaaccatcatcatcgagaccatgagccaccagcattccatgtgtattcgtccctatctgccctactacaacgtgtcccaccagctggccacattcactttaaagggatctttaagggagatccaagaactgcaagtgtggtataccaagctcggaaccccccagcaacggctgcacttcaagcagctggatactttatggctgctggacggcagcggaagcttcactttagagctggaggaggatgaaatttttactttaaccacactgaccaccggacggaaaggctcctatcccccccccccttccagcaagcctttccccaccaactataaggacgacttcaatgtcgagtaccctttattttccgaagctcccaacttcgctgatcagaccggcgtcttcgagtactacatgaacaacgaggaccgggagcatcggttcacactgaggcaagttctgaaccaacggcccatcacttgggccgctgacgcttcctccaccatctccgtcatcggagaccaccactggacaaacatgaccgtgcagtgcgatgtctacatcgaaaccccccggagcggaggcgtgttcattgccggtcgtgtgaacaagggcggcattctgatccggtccgccactggtgtcttcttctggatctttgccaacggaagctatcgtgtcaccgccgatttaggaggatggatcacctacgccagcggccatgccgatgtgacagccaagaggtggtacacactcacactgggcatcaagggatacttcgccttcggaatgctgaacggcacaatcctctggaagaacgtgcgggtcaaataccccggccacggctgggctgctatcggcacacacacctttgagttcgcccagtttgacaattttcgggtggaggccgctaggggatccgaggctcacaagagcgaaatcgctcatcgttacaacgatttaggcgagcagcacttcaagggtttagttttaatcgctttctcccagtacctccagaagtgctcctacgacgagcatgccaagctcgtgcaagaggtgaccgactttgctaagacttgtgtggccgatgagtccgccgctaactgcgataagtctttacacaccctctttggagacaaactgtgcgccatccctaatctgcgggagaactacggcgagctggccgattgctgcacaaagcaagaacccgaaaggaacgagtgtttcctccagcacaaagacgacaacccttctttacctccctttgagaggcccgaggccgaggctatgtgtacctccttcaaggaaaaccccacaacattcatgggacattatttacatgaggtcgctcggcggcacccttacttctacgcccccgagctgctgtattacgccgagcagtacaacgagattctgacccagtgttgtgccgaagctgataaagagagctgtttaacacccaagctggatggcgtgaaggaaaaggctttagtcagcagcgtgaggcagaggatgaaatgctcctccatgcaaaagttcggcgaacgggcctttaaggcttgggctgtggctcgtctgagccagacattccccaacgccgacttcgccgagattaccaaactcgccaccgatctgacaaaggtcaacaaggagtgctgccatggtgatttactggagtgcgccgacgatagggccgaactcgctaaatacatgtgcgagaaccaagctaccatctccagcaagctgcagacttgttgtgataaacccctcctcaagaaggctcactgtttatccgaggtcgagcacgacacaatgcccgctgatctgcccgctatcgccgctgattttgtggaagaccaagaagtctgtaagaattacgctgaggctaaggatgtgtttctcggcacctttttatacgaatatagccggaggcaccccgattatagcgtcagcctcttattacggctggctaagaagtatgaggccacactggaaaagtgctgtgccgaggctaaccctcccgcttgttacggaaccgtgctggctgaatttcagcctttagtcgaggagcccaagaatctggtgaagaccaactgtgatctgtacgaaaagctgggcgagtatggcttccaaaacgccattttagtgcggtatacacagaaggccccccaagtttccacccccacactggtcgaagctgcccggaatctgggacgggtgggcaccaagtgttgcactttacccgaggaccagaggctgccttgcgtggaggactacctcagcgctatcctcaatcgtgtctgtttactgcacgaaaagacacccgttagcgaacacgtgacaaagtgctgctccggctctttagtggaacggaggccttgctttagcgctttaacagtggacgaaacctacgtgcctaaggagtttaaggccgagaccttcacctttcactccgacatctgcactttacccgaaaaagagaagcagatcaaaaagcagaccgccctcgccgagctcgtcaaacataagcctaaggctaccgccgaacagctcaaaaccgtgatggacgacttcgcccaatttttagatacatgctgcaaggccgccgacaaggacacttgtttttccaccgagggccccaatttagtcactcgttgcaaggatgctttagct

SEQ ID NO: 22 - protein, 760 aa, Homo sapiens
MMDQARSAFSNLFGGEPLSYTRFSLARQVDGDNSHVEMKLAVDEEENADNNTKANVTKPKRCSGSICYGTIAVIVFFLIGFMIGYLGYCKGVEPKTECERLAGTESPVREEPGEDFPAARRLYWDDLKRKLSEKLDSTDFTGTIKLLNENSYVPREAGSQKDENLALYVENQFREFKLSKVWRDQHFVKIQVKDSAQNSVIIVDKNGRLVYLVENPGGYVAYSKAATVTGKLVHANFGTKKDFEDLYTPVNGSIVIVRAGKITFAEKVANAESLNAIGVLIYMDQTKFPIVNAELSFFGHAHLGTGDPYTPGFPSFNHTQFPPSRSSGLPNIPVQTISRAAAEKLFGNMEGDCPSDWKTDSTCRMVTSESKNVKLTVSNVLKEIKILNIFGVIKGFVEPDHYVVVGAQRDAWGPGAAKSGVGTALLLKLAQMFSDMVLKDGFQPSRSIIFASWSAGDFGSVGATEWLEGYLSSLHLKAFTYINLDKAVLGTSNFKVSASPLLYTLIEKTMQNVKHPVTGQFLYQDSNWASKVEKLTLDNAAFPFLAYSGIPAVSFCFCEDTDYPYLGTTMDTYKELIERIPELNKVARAAAEVAGQFVIKLTHDVELNLDYERYNSQLLSFVRDLNQYRADIKEMGLSLQWLYSARGDFFRATSRLTTDFGNAEKTDRFVMKKLNDRVMRVEYHFLSPYVSPKESPFRHVFWGSGSHTLPALLENLKLRKQNNGAFNETLFRNQLALATWTIQGAANALSGDVWDIDNEF

SEQ ID NO: 23 - protein, 219 aa, synthetic construct
DIVMTQTPLSLSVTPGQPASISCRSSQSLVHSNGNTYLHWYLQKPGQSPQLLIYKVSNRFSGVPDRFSGSGSGTDFTLKISRVEAEDVGVYYCSQSTHVPWTFGQGTKVEIKRTVAAPSVFIFPPSDEQLKSGTASVVCLLNNFYPREAKVQWKVDNALQSGNSQESVTEQDSKDSTYSLSSTLTLSKADYEKHKVYACEVTHQGLSSPVTKSFNRGEC

SEQ ID NO: 24 - protein, 160 aa, Homo sapiens
SPGQGTQSENSCTHFPGNLPNMLRDLRDAFSRVKTFFQMKDQLDNLLLKESLLEDFKGYLGCQALSEMIQFYLEEVMPQAENQDPDIKAHVNSLGENLKTLRLRLRRCHRFLPCENKSKAVEQVKNAFNKLQEKGIYKAMSEFDIFINYIEAYMTMKIRN

SEQ ID NO: 25 - protein, 226 aa, synthetic construct
EVQLVQSGAEVKKPGESLKISCKGSGYSFMNYWLGWVRQMPGKGLEWMGDIYPGGDYPTYSEKFKVQVTISADKSISTAYLQLSSLKASDTAMYYCARSGNYDEVAYWGQGTLVTVSSASTKGPSVFPLAPSSKSTSGGTAALGCLVKDYFPEPVTVSWNSGALTSGVHTFPAVLQSSGLYSLSSVVTVPSSSLGTQTYICNVNHKPSNTKVDKKVEPKSCDKTHT

SEQ ID NO: 26 - DNA, 28 bp, synthetic construct
  source 1..28: mol_type = other DNA
ctagcggcgcgcctcgcgaagcgctgca

SEQ ID NO: 27 - DNA, 28 bp, synthetic construct
  source 1..28: mol_type = other DNA
ggcctgcagcgcttcgcgaggcgcgccg

SEQ ID NO: 28 - protein, 1474 aa, synthetic construct
EVQLVQSGAEVKKPGESLKISCKGSGYSFMNYWLGWVRQMPGKGLEWMGDIYPGGDYPTYSEKFKVQVTISADKSISTAYLQLSSLKASDTAMYYCARSGNYDEVAYWGQGTLVTVSSASTKGPSVFPLAPSSKSTSGGTAALGCLVKDYFPEPVTVSWNSGALTSGVHTFPAVLQSSGLYSLSSVVTVPSSSLGTQTYICNVNHKPSNTKVDKKVEPKSCDKTHTGGGGSGGGGSGGGGSDAHKSEVAHRFKDLGEENFKALVLIAFAQYLQQCPFEDHVKLVNEVTEFAKTCVADESAENCDKSLHTLFGDKLCTVATLRETYGEMADCCAKQEPERNECFLQHKDDNPNLPRLVRPEVDVMCTAFHDNEETFLKKYLYEIARRHPYFYAPELLFFAKRYKAAFTECCQAADKAACLLPKLDELRDEGKASSAKQRLKCASLQKFGERAFKAWAVARLSQRFPKAEFAEVSKLVTDLTKVHTECCHGDLLECADDRADLAKYICENQDSISSKLKECCEKPLLEKSHCIAEVENDEMPADLPSLAADFVESKDVCKNYAEAKDVFLGMFLYEYARRHPDYSVVLLLRLAKTYETTLEKCCAAADPHECYAKVFDEFKPLVEEPQNLIKQNCELFEQLGEYKFQNALLVRYTKKVPQVSTPTLVEVSRNLGKVGSKCCKHPEAKRMPCAEDYLSVVLNQLCVLHEKTPVSDRVTKCCTESLVNRRPCFSALEVDETYVPKEFNAETFTFHADICTLSEKERQIKKQTALVELVKHKPKATKEQLKAVMDDFAAFVEKCCKADDKETCFAEEGKKLVAASQAALGLGGGGSYVLDDSDGLGREFDGIGAVSGGGATSRLLVNYPEPYRSQILDYLFKPNFGASLHILKVEIGGDGQTTDGTEPSHMHYALDENYFRGYEWWLMKEAKKRNPNITLIGLPWSFPGWLGKGFDWPYVNLQLTAYYVVTWIVGAKRYHDLDIDYIGIWNERSYNANYIKILRKMLNYQGLQRVKIIASDNLWESISASMLLDAELFKVVDVIGAHYPGTHSAKDAKLTGKKLWSSEDFSTLNSDMGAGCWGRILNQNYINGYMTSTIAWNLVASYYEQLPYGRCGLMTAQEPWSGHYVVESPVWVSAHTTQFTQPGWYYLKTVGHLEKGGSYVALTDGLGNLTIIIETMSHKHSKCIRPFLPYFNVSQQFATFVLKGSFSEIPELQVWYTKLGKTSERFLFKQLDSLWLLDSDGSFTLSLHEDELFTLTTLTTGRKGSYPLPPKSQPFPSTYKDDFNVDYPFFSEAPNFADQTGVFEYFTNIEDPGEHHFTLRQVLNQRPITWAADASNTISIIGDYNWTNLTIKCDVYIETPDTGGVFIAGRVNKGGILIRSARGIFFWIFANGSYRVTGDLAGWIIYALGRVEVTAKKWYTLTLTIKGHFTSGMLNDKSLWTDIPVNFPKNGWAAIGTHSFEFAQFDNFLVEATR

SEQ ID NO: 29 - DNA, 4413 bp, synthetic construct
  source 1..4413: mol_type = other DNA
gaggtgcaactagtgcagtctggagcagaggtgaaaaagcccggggagtctctgaagatttcctgtaagggttctggatacagctttatgaactactggctgggatgggtgcgccagatgcccgggaaaggcctggagtggatgggggacatctaccccggcggagactaccctacatacagcgagaagttcaaggtccaggtcaccatctcagccgacaagtccatcagcaccgcctacctgcagttgagcagcctgaaggcctcggacaccgccatgtattactgtgcgagatcaggcaattacgacgaagtggcctactggggccaaggaaccctggtcaccgtctcctcagctagcaccaagggcccatcggtcttccccctggcaccctcctccaagagcacctctgggggcacagcggccctgggctgcctggtcaaggactacttccccgaaccggtgacggtgtcgtggaactcaggcgccctgaccagcggcgtgcacaccttcccggctgtcctacagtcctcaggactctactccctcagcagcgtggtgaccgtgccctccagcagcttgggcacccagacctacatctgcaacgtgaatcacaagcccagcaacaccaaggtggacaagaaagttgagccgaagagctgtgataagacgcatacgggtggcggagggtctggaggtggcggatcaggcggaggtggatccgatgcacacaagagtgaggttgctcatcggtttaaagatttgggagaagaaaatttcaaagccttggtgttgattgcctttgctcagtatcttcagcagtgtccatttgaagatcatgtaaaattagtgaatgaagtaactgaatttgcaaaaacatgtgttgctgatgagtcagctgaaaattgtgacaaatcacttcataccctttttggagacaaattatgcacagttgcaactcttcgtgaaacctatggtgaaatggctgactgctgtgcaaaacaagaacctgagagaaatgaatgcttcttgcaacacaaagatgacaacccaaacctcccccgattggtgagaccagaggttgatgtgatgtgcactgcttttcatgacaatgaagagacatttttgaaaaaatacttatatgaaattgccagaagacatccttacttttatgccccggaactccttttctttgctaaaaggtataaagctgcttttacagaatgttgccaagctgctgataaagctgcctgcctgttgccaaagctcgatgaacttcgggatgaagggaaggcttcgtctgccaaacagagactcaagtgtgccagtctccaaaaatttggagaaagagctttcaaagcatgggcagtagctcgcctgagccagagatttcccaaagctgagtttgcagaagtttccaagttagtgacagatcttaccaaagtccacacggaatgctgccatggagatctgcttgaatgtgctgatgacagggcggaccttgccaagtatatctgtgaaaatcaagattcgatctccagtaaactgaaggaatgctgtgaaaaacctctgttggaaaaatcccactgcattgccgaagtggaaaatgatgagatgcctgctgacttgccttcattagctgctgattttgttgaaagtaaggatgtttgcaaaaactatgctgaggcaaaggatgtcttcctgggcatgtttttgtatgaatatgcaagaaggcatcctgattactctgtcgtgctgctgctgagacttgccaagacatatgaaaccactctagagaagtgctgtgccgctgcagatcctcatgaatgctatgccaaagtgttcgatgaatttaaacctcttgtggaagagcctcagaatttaatcaaacaaaattgtgagctttttgagcagcttggagagtacaaattccagaatgcgctattagttcgttacaccaagaaagtaccccaagtgtcaactccaactcttgtagaggtctcaagaaacctaggaaaagtgggcagcaaatgttgtaaacatcctgaagcaaaaagaatgccctgtgcagaagactatctatccgtggtcctgaaccagttatgtgtgttgcatgagaaaacgccagtaagtgacagagtcaccaaatgctgcacagaatccttggtgaacaggcgaccatgcttttcagctctggaagtcgatgaaacatacgttcccaaagagtttaatgctgaaacattcaccttccatgcagatatatgcacactttctgagaaggagagacaaatcaagaaacaaactgcacttgttgagctcgtgaaacacaagcccaaggcaacaaaagagcaactgaaagctgttatggatgatttcgcagcttttgtagagaagtgctgcaaggctgacgataaggagacctgctttgccgaggagggtaaaaaacttgttgctgcaagtcaagctgccttaggcttaggatcctacgtgctggacgactctgacggactcggaagggagtttgacggcattggcgctgtgtccggaggcggcgctacatctcgtctgctggtgaattatcccgagccctaccggtcccagattttagactacctcttcaaacccaattttggagcctccctccacattttaaaggtggaaatcggcggcgacggacagacaaccgatggcaccgaacctagccatatgcactacgctttagacgagaactatttccggggctatgagtggtggctgatgaaggaggccaagaagaggaaccccaacattaccctcatcggactgccttggagctttcccggttggctgggcaaaggattcgactggccctacgtgaatttacagctgaccgcttactacgtggtgacttggattgtgggagccaagcggtaccacgatctcgacatcgattacattggcatctggaacgagcggagctacaacgctaactatatcaagattctgcggaaaatgctgaattaccaaggtttacagcgggtgaagatcatcgctagcgacaatttatgggaaagcatctccgctagcatgctgctggacgctgaactgttcaaagtcgtggatgtcatcggcgctcactatcccggcacccatagcgccaaggacgccaagctgaccggaaaaaagctgtggtccagcgaggatttcagcactttaaactccgatatgggagctggctgctggggccggattttaaaccagaactacatcaatggctacatgacaagcaccatcgcttggaatttagtggcctcctactacgagcagctgccctatggacggtgcggtttaatgacagcccaagagccttggagcggccattacgtggtggagagccccgtttgggtgagcgctcacaccacccagttcacccagcccggctggtactacctcaagaccgtcggacatctggagaagggcggctcctacgtggctttaactgatggtttaggcaatctgaccatcattatcgagaccatgtcccacaagcactccaagtgcatccggccctttctgccctacttcaacgtgtcccagcaattcgccacctttgtgctgaagggcagcttttccgagattcccgagctccaagtttggtacaccaagctgggaaaaaccagcgagaggtttttattcaagcaactggactctttatggctgctggacagcgatggctccttcacactgtctttacatgaggatgagctctttactttaaccactttaacaactggtcggaaaggctcctatcctttaccccccaagagccaacccttccccagcacctacaaggacgacttcaacgtggattaccccttcttctccgaggctcccaactttgctgaccagaccggcgtgttcgagtatttcaccaacatcgaggaccccggtgagcaccatttcaccctccggcaagttctgaaccaacggcctatcacttgggccgccgacgcttccaataccatctccattatcggcgactacaactggacaaatttaactatcaagtgcgacgtctacatcgagacccccgataccggaggcgtgtttatcgctggaagggtgaacaaaggcggcattttaatccggtccgctaggggcatctttttctggatcttcgctaacggcagctatcgggtgactggtgacctcgctggctggatcatttacgctctgggccgggtggaggtgacagccaagaagtggtacactttaactttaactattaagggacattttaccagcggcatgctgaacgacaaatctttatggaccgacatccccgtgaactttcccaagaatggctgggccgccatcggcacccattcctttgaattcgcccagttcgacaatttcctcgtggaagccacccgg

SEQ ID NO: 30 - protein, 1474 aa, synthetic construct
DAHKSEVAHRFKDLGEENFKALVLIAFAQYLQQCPFEDHVKLVNEVTEFAKTCVADESAENCDKSLHTLFGDKLCTVATLRETYGEMADCCAKQEPERNECFLQHKDDNPNLPRLVRPEVDVMCTAFHDNEETFLKKYLYEIARRHPYFYAPELLFFAKRYKAAFTECCQAADKAACLLPKLDELRDEGKASSAKQRLKCASLQKFGERAFKAWAVARLSQRFPKAEFAEVSKLVTDLTKVHTECCHGDLLECADDRADLAKYICENQDSISSKLKECCEKPLLEKSHCIAEVENDEMPADLPSLAADFVESKDVCKNYAEAKDVFLGMFLYEYARRHPDYSVVLLLRLAKTYETTLEKCCAAADPHECYAKVFDEFKPLVEEPQNLIKQNCELFEQLGEYKFQNALLVRYTKKVPQVSTPTLVEVSRNLGKVGSKCCKHPEAKRMPCAEDYLSVVLNQLCVLHEKTPVSDRVTKCCTESLVNRRPCFSALEVDETYVPKEFNAETFTFHADICTLSEKERQIKKQTALVELVKHKPKATKEQLKAVMDDFAAFVEKCCKADDKETCFAEEGKKLVAASQAALGLGGGGSYVLDDSDGLGREFDGIGAVSGGGATSRLLVNYPEPYRSQILDYLFKPNFGASLHILKVEIGGDGQTTDGTEPSHMHYALDENYFRGYEWWLMKEAKKRNPNITLIGLPWSFPGWLGKGFDWPYVNLQLTAYYVVTWIVGAKRYHDLDIDYIGIWNERSYNANYIKILRKMLNYQGLQRVKIIASDNLWESISASMLLDAELFKVVDVIGAHYPGTHSAKDAKLTGKKLWSSEDFSTLNSDMGAGCWGRILNQNYINGYMTSTIAWNLVASYYEQLPYGRCGLMTAQEPWSGHYVVESPVWVSAHTTQFTQPGWYYLKTVGHLEKGGSYVALTDGLGNLTIIIETMSHKHSKCIRPFLPYFNVSQQFATFVLKGSFSEIPELQVWYTKLGKTSERFLFKQLDSLWLLDSDGSFTLSLHEDELFTLTTLTTGRKGSYPLPPKSQPFPSTYKDDFNVDYPFFSEAPNFADQTGVFEYFTNIEDPGEHHFTLRQVLNQRPITWAADASNTISIIGDYNWTNLTIKCDVYIETPDTGGVFIAGRVNKGGILIRSARGIFFWIFANGSYRVTGDLAGWIIYALGRVEVTAKKWYTLTLTIKGHFTSGMLNDKSLWTDIPVNFPKNGWAAIGTHSFEFAQFDNFLVEATRGGGGSGGGGSGGGGSEVQLVQSGAEVKKPGESLKISCKGSGYSFMNYWLGWVRQMPGKGLEWMGDIYPGGDYPTYSEKFKVQVTISADKSISTAYLQLSSLKASDTAMYYCARSGNYDEVAYWGQGTLVTVSSASTKGPSVFPLAPSSKSTSGGTAALGCLVKDYFPEPVTVSWNSGALTSGVHTFPAVLQSSGLYSLSSVVTVPSSSLGTQTYICNVNHKPSNTKVDKKVEPKSCDKTHT

SEQ ID NO: 31 - DNA, 4413 bp, synthetic construct
  source 1..4413: mol_type = other DNA
gatgcacacaagagtgaggttgctcatcggtttaaagatttgggagaagaaaatttcaaagccttggtgttgattgcctttgctcagtatcttcagcagtgtccatttgaagatcatgtaaaattagtgaatgaagtaactgaatttgcaaaaacatgtgttgctgatgagtcagctgaaaattgtgacaaatcacttcataccctttttggagacaaattatgcacagttgcaactcttcgtgaaacctatggtgaaatggctgactgctgtgcaaaacaagaacctgagagaaatgaatgcttcttgcaacacaaagatgacaacccaaacctcccccgattggtgagaccagaggttgatgtgatgtgcactgcttttcatgacaatgaagagacatttttgaaaaaatacttatatgaaattgccagaagacatccttacttttatgccccggaactccttttctttgctaaaaggtataaagctgcttttacagaatgttgccaagctgctgataaagctgcctgcctgttgccaaagctcgatgaacttcgggatgaagggaaggcttcgtctgccaaacagagactcaagtgtgccagtctccaaaaatttggagaaagagctttcaaagcatgggcagtagctcgcctgagccagagatttcccaaagctgagtttgcagaagtttccaagttagtgacagatcttaccaaagtccacacggaatgctgccatggagatctgcttgaatgtgctgatgacagggcggaccttgccaagtatatctgtgaaaatcaagattcgatctccagtaaactgaaggaatgctgtgaaaaacctctgttggaaaaatcccactgcattgccgaagtggaaaatgatgagatgcctgctgacttgccttcattagctgctgattttgttgaaagtaaggatgtttgcaaaaactatgctgaggcaaaggatgtcttcctgggcatgtttttgtatgaatatgcaagaaggcatcctgattactctgtcgtgctgctgctgagacttgccaagacatatgaaaccactctagagaagtgctgtgccgctgcagatcctcatgaatgctatgccaaagtgttcgatgaatttaaacctcttgtggaagagcctcagaatttaatcaaacaaaattgtgagctttttgagcagcttggagagtacaaattccagaatgcgctattagttcgttacaccaagaaagtaccccaagtgtcaactccaactcttgtagaggtctcaagaaacctaggaaaagtgggcagcaaatgttgtaaacatcctgaagcaaaaagaatgccctgtgcagaagactatctatccgtggtcctgaaccagttatgtgtgttgcatgagaaaacgccagtaagtgacagagtcaccaaatgctgcacagaatccttggtgaacaggcgaccatgcttttcagctctggaagtcgatgaaacatacgttcccaaagagtttaatgctgaaacattcaccttccatgcagatatatgcacactttctgagaaggagagacaaatcaagaaacaaactgcacttgttgagctcgtgaaacacaagcccaaggcaacaaaagagcaactgaaagctgttatggatgatttcgcagcttttgtagagaagtgctgcaaggctgacgataaggagacctgctttgccgaggagggtaaaaaacttgttgctgcaagtcaagctgccttaggcttaggatcctacgtgctggacgactctgacggactcggaagggagtttgacggcattggcgctgtgtccggaggcggcgctacatctcgtctgctggtgaattatcccgagccctaccggtcccagattttagactacctcttcaaacccaattttggagcctccctccacattttaaaggtggaaatcggcggcgacggacagacaaccgatggcaccgaacctagccatatgcactacgctttagacgagaactatttccggggctatgagtggtggctgatgaaggaggccaagaagaggaaccccaacattaccctcatcggactgccttggagctttcccggttggctgggcaaaggattcgactggccctacgtgaatttacagctgaccgcttactacgtggtgacttggattgtgggagccaagcggtaccacgatctcgacatcgattacattggcatctggaacgagcggagctacaacgctaactatatcaagattctgcggaaaatgctgaattaccaaggtttacagcgggtgaagatcatcgctagcgacaatttatgggaaagcatctccgctagcatgctgctggacgctgaactgttcaaagtcgtggatgtcatcggcgctcactatcccggcacccatagcgccaaggacgccaagctgaccggaaaaaagctgtggtccagcgaggatttcagcactttaaactccgatatgggagctggctgctggggccggattttaaaccagaactacatcaatggctacatgacaagcaccatcgcttggaatttagtggcctcctactacgagcagctgccctatggacggtgcggtttaatgacagcccaagagccttggagcggccattacgtggtggagagccccgtttgggtgagcgctcacaccacccagttcacccagcccggctggtactacctcaagaccgtcggacatctggagaagggcggctcctacgtggctttaactgatggtttaggcaatctgaccatcattatcgagaccatgtcccacaagcactccaagtgcatccggccctttctgccctacttcaacgtgtcccagcaattcgccacctttgtgctgaagggcagcttttccgagattcccgagctccaagtttggtacaccaagctgggaaaaaccagcgagaggtttttattcaagcaactggactctttatggctgctggacagcgatggctccttcacactgtctttacatgaggatgagctctttactttaaccactttaacaactggtcggaaaggctcctatcctttaccccccaagagccaacccttccccagcacctacaaggacgacttcaacgtggattaccccttcttctccgaggctcccaactttgctgaccagaccggcgtgttcgagtatttcaccaacatcgaggaccccggtgagcaccatttcaccctccggcaagttctgaaccaacggcctatcacttgggccgccgacgcttccaataccatctccattatcggcgactacaactggacaaatttaactatcaagtgcgacgtctacatcgagacccccgataccggaggcgtgtttatcgctggaagggtgaacaaaggcggcattttaatccggtccgctaggggcatctttttctggatcttcgctaacggcagctatcgggtgactggtgacctcgctggctggatcatttacgctctgggccgggtggaggtgacagccaagaagtggtacactttaactttaactattaagggacattttaccagcggcatgctgaacgacaaatctttatggaccgacatccccgtgaactttcccaagaatggctgggccgccatcggcacccattcctttgaattcgcccagttcgacaatttcctcgtggaagccacccggggtggcggaggttcaggcggcggtgggtcgggaggtggtggaagcgaggtgcaactagtgcagtctggagcagaggtgaaaaagcccggggagtctctgaagatttcctgtaagggttctggatacagctttatgaactactggctgggatgggtgcgccagatgcccgggaaaggcctggagtggatgggggacatctaccccggcggagactaccctacatacagcgagaagttcaaggtccaggtcaccatctcagccgacaagtccatcagcaccgcctacctgcagttgagcagcctgaaggcctcggacaccgccatgtattactgtgcgagatcaggcaattacgacgaagtggcctactggggccaaggaaccctggtcaccgtctcctcagctagcaccaagggcccatcggtcttccccctggcaccctcctccaagagcacctctgggggcacagcggccctgggctgcctggtcaaggactacttccccgaaccggtgacggtgtcgtggaactcaggcgccctgaccagcggcgtgcacaccttcccggctgtcctacagtcctcaggactctactccctcagcagcgtggtgaccgtgccctccagcagcttgggcacccagacctacatctgcaacgtgaatcacaagcccagcaacaccaaggtggacaagaaagttgagccgaagagctgtgataagacgcatacg

SEQ ID NO: 32 - protein, 1474 aa, synthetic construct
EVQLVQSGAEVKKPGESLKISCKGSGYSFMNYWLGWVRQMPGKGLEWMGDIYPGGDYPTYSEKFKVQVTISADKSISTAYLQLSSLKASDTAMYYCARSGNYDEVAYWGQGTLVTVSSASTKGPSVFPLAPSSKSTSGGTAALGCLVKDYFPEPVTVSWNSGALTSGVHTFPAVLQSSGLYSLSSVVTVPSSSLGTQTYICNVNHKPSNTKVDKKVEPKSCDKTHTGGGGSGGGGSGGGGSYVLDDSDGLGREFDGIGAVSGGGATSRLLVNYPEPYRSQILDYLFKPNFGASLHILKVEIGGDGQTTDGTEPSHMHYALDENYFRGYEWWLMKEAKKRNPNITLIGLPWSFPGWLGKGFDWPYVNLQLTAYYVVTWIVGAKRYHDLDIDYIGIWNERSYNANYIKILRKMLNYQGLQRVKIIASDNLWESISASMLLDAELFKVVDVIGAHYPGTHSAKDAKLTGKKLWSSEDFSTLNSDMGAGCWGRILNQNYINGYMTSTIAWNLVASYYEQLPYGRCGLMTAQEPWSGHYVVESPVWVSAHTTQFTQPGWYYLKTVGHLEKGGSYVALTDGLGNLTIIIETMSHKHSKCIRPFLPYFNVSQQFATFVLKGSFSEIPELQVWYTKLGKTSERFLFKQLDSLWLLDSDGSFTLSLHEDELFTLTTLTTGRKGSYPLPPKSQPFPSTYKDDFNVDYPFFSEAPNFADQTGVFEYFTNIEDPGEHHFTLRQVLNQRPITWAADASNTISIIGDYNWTNLTIKCDVYIETPDTGGVFIAGRVNKGGILIRSARGIFFWIFANGSYRVTGDLAGWIIYALGRVEVTAKKWYTLTLTIKGHFTSGMLNDKSLWTDIPVNFPKNGWAAIGTHSFEFAQFDNFLVEATRGGGGSDAHKSEVAHRFKDLGEENFKALVLIAFAQYLQQCPFEDHVKLVNEVTEFAKTCVADESAENCDKSLHTLFGDKLCTVATLRETYGEMADCCAKQEPERNECFLQHKDDNPNLPRLVRPEVDVMCTAFHDNEETFLKKYLYEIARRHPYFYAPELLFFAKRYKAAFTECCQAADKAACLLPKLDELRDEGKASSAKQRLKCASLQKFGERAFKAWAVARLSQRFPKAEFAEVSKLVTDLTKVHTECCHGDLLECADDRADLAKYICENQDSISSKLKECCEKPLLEKSHCIAEVENDEMPADLPSLAADFVESKDVCKNYAEAKDVFLGMFLYEYARRHPDYSVVLLLRLAKTYETTLEKCCAAADPHECYAKVFDEFKPLVEEPQNLIKQNCELFEQLGEYKFQNALLVRYTKKVPQVSTPTLVEVSRNLGKVGSKCCKHPEAKRMPCAEDYLSVVLNQLCVLHEKTPVSDRVTKCCTESLVNRRPCFSALEVDETYVPKEFNAETFTFHADICTLSEKERQIKKQTALVELVKHKPKATKEQLKAVMDDFAAFVEKCCKADDKETCFAEEGKKLVAASQAALGL

SEQ ID NO: 33 - DNA, 4413 bp, synthetic construct
  source 1..4413: mol_type = other DNA
gaggtgcaactagtgcagtctggagcagaggtgaaaaagcccggggagtctctgaagatttcctgtaagggttctggatacagctttatgaactactggctgggatgggtgcgccagatgcccgggaaaggcctggagtggatgggggacatctaccccggcggagactaccctacatacagcgagaagttcaaggtccaggtcaccatctcagccgacaagtccatcagcaccgcctacctgcagttgagcagcctgaaggcctcggacaccgccatgtattactgtgcgagatcaggcaattacgacgaagtggcctactggggccaaggaaccctggtcaccgtctcctcagctagcaccaagggcccatcggtcttccccctggcaccctcctccaagagcacctctgggggcacagcggccctgggctgcctggtcaaggactacttccccgaaccggtgacggtgtcgtggaactcaggcgccctgaccagcggcgtgcacaccttcccggctgtcctacagtcctcaggactctactccctcagcagcgtggtgaccgtgccctccagcagcttgggcacccagacctacatctgcaacgtgaatcacaagcccagcaacaccaaggtggacaagaaagttgagccgaagagctgtgataagacgcatacgggtggcggagggtctggaggtggcggatcaggcggaggtggatcctacgtgctggacgactctgacggactcggaagggagtttgacggcattggcgctgtgtccggaggcggcgctacatctcgtctgctggtgaattatcccgagccctaccggtcccagattttagactacctcttcaaacccaattttggagcctccctccacattttaaaggtggaaatcggcggcgacggacagacaaccgatggcaccgaacctagccatatgcactacgctttagacgagaactatttccggggctatgagtggtggctgatgaaggaggccaagaagaggaaccccaacattaccctcatcggactgccttggagctttcccggttggctgggcaaaggattcgactggccctacgtgaatttacagctgaccgcttactacgtggtgacttggattgtgggagccaagcggtaccacgatctcgacatcgattacattggcatctggaacgagcggagctacaacgctaactatatcaagattctgcggaaaatgctgaattaccaaggtttacagcgggtgaagatcatcgctagcgacaatttatgggaaagcatctccgctagcatgctgctggacgctgaactgttcaaagtcgtggatgtcatcggcgctcactatcccggcacccatagcgccaaggacgccaagctgaccggaaaaaagctgtggtccagcgaggatttcagcactttaaactccgatatgggagctggctgctggggccggattttaaaccagaactacatcaatggctacatgacaagcaccatcgcttggaatttagtggcctcctactacgagcagctgccctatggacggtgcggtttaatgacagcccaagagccttggagcggccattacgtggtggagagccccgtttgggtgagcgctcacaccacccagttcacccagcccggctggtactacctcaagaccgtcggacatctggagaagggcggctcctacgtggctttaactgatggtttaggcaatctgaccatcattatcgagaccatgtcccacaagcactccaagtgcatccggccctttctgccctacttcaacgtgtcccagcaattcgccacctttgtgctgaagggcagcttttccgagattcccgagctccaagtttggtacaccaagctgggaaaaaccagcgagaggtttttattcaagcaactggactctttatggctgctggacagcgatggctccttcacactgtctttacatgaggatgagctctttactttaaccactttaacaactggtcggaaaggctcctatcctttaccccccaagagccaacccttccccagcacctacaaggacgacttcaacgtggattaccccttcttctccgaggctcccaactttgctgaccagaccggcgtgttcgagtatttcaccaacatcgaggaccccggtgagcaccatttcaccctccggcaagttctgaaccaacggcctatcacttgggccgccgacgcttccaataccatctccattatcggcgactacaactggacaaatttaactatcaagtgcgacgtctacatcgagacccccgataccggaggcgtgtttatcgctggaagggtgaacaaaggcggcattttaatccggtccgctaggggcatctttttctggatcttcgctaacggcagctatcgggtgactggtgacctcgctggctggatcatttacgctctgggccgggtggaggtgacagccaagaagtggtacactttaactttaactattaagggacattttaccagcggcatgctgaacgacaaatctttatggaccgacatccccgtgaactttcccaagaatggctgggccgccatcggcacccattcctttgaattcgcccagttcgacaatttcctcgtggaagccacccggggatccgatgcacacaagagtgaggttgctcatcggtttaaagatttgggagaagaaaatttcaaagccttggtgttgattgcctttgctcagtatcttcagcagtgtccatttgaagatcatgtaaaattagtgaatgaagtaactgaatttgcaaaaacatgtgttgctgatgagtcagctgaaaattgtgacaaatcacttcataccctttttggagacaaattatgcacagttgcaactcttcgtgaaacctatggtgaaatggctgactgctgtgcaaaacaagaacctgagagaaatgaatgcttcttgcaacacaaagatgacaacccaaacctcccccgattggtgagaccagaggttgatgtgatgtgcactgcttttcatgacaatgaagagacatttttgaaaaaatacttatatgaaattgccagaagacatccttacttttatgccccggaactccttttctttgctaaaaggtataaagctgcttttacagaatgttgccaagctgctgataaagctgcctgcctgttgccaaagctcgatgaacttcgggatgaagggaaggcttcgtctgccaaacagagactcaagtgtgccagtctccaaaaatttggagaaagagctttcaaagcatgggcagtagctcgcctgagccagagatttcccaaagctgagtttgcagaagtttccaagttagtgacagatcttaccaaagtccacacggaatgctgccatggagatctgcttgaatgtgctgatgacagggcggaccttgccaagtatatctgtgaaaatcaagattcgatctccagtaaactgaaggaatgctgtgaaaaacctctgttggaaaaatcccactgcattgccgaagtggaaaatgatgagatgcctgctgacttgccttcattagctgctgattttgttgaaagtaaggatgtttgcaaaaactatgctgaggcaaaggatgtcttcctgggcatgtttttgtatgaatatgcaagaaggcatcctgattactctgtcgtgctgctgctgagacttgccaagacatatgaaaccactctagagaagtgctgtgccgctgcagatcctcatgaatgctatgccaaagtgttcgatgaatttaaacctcttgtggaagagcctcagaatttaatcaaacaaaattgtgagctttttgagcagcttggagagtacaaattccagaatgcgctattagttcgttacaccaagaaagtaccccaagtgtcaactccaactcttgtagaggtctcaagaaacctaggaaaagtgggcagcaaatgttgtaaacatcctgaagcaaaaagaatgccctgtgcagaagactatctatccgtggtcctgaaccagttatgtgtgttgcatgagaaaacgccagtaagtgacagagtcaccaaatgctgcacagaatccttggtgaacaggcgaccatgcttttcagctctggaagtcgatgaaacatacgttcccaaagagtttaatgctgaaacattcaccttccatgcagatatatgcacactttctgagaaggagagacaaatcaagaaacaaactgcacttgttgagctcgtgaaacacaagcccaaggcaacaaaagagcaactgaaagctgttatggatgatttcgcagcttttgtagagaagtgctgcaaggctgacgataaggagacctgctttgccgaggagggtaaaaaacttgttgctgcaagtcaagctgccttaggctta

SEQ ID NO: 34 - protein, 1474 aa, synthetic construct
YVLDDSDGLGREFDGIGAVSGGGATSRLLVNYPEPYRSQILDYLFKPNFGASLHILKVEIGGDGQTTDGTEPSHMHYALDENYFRGYEWWLMKEAKKRNPNITLIGLPWSFPGWLGKGFDWPYVNLQLTAYYVVTWIVGAKRYHDLDIDYIGIWNERSYNANYIKILRKMLNYQGLQRVKIIASDNLWESISASMLLDAELFKVVDVIGAHYPGTHSAKDAKLTGKKLWSSEDFSTLNSDMGAGCWGRILNQNYINGYMTSTIAWNLVASYYEQLPYGRCGLMTAQEPWSGHYVVESPVWVSAHTTQFTQPGWYYLKTVGHLEKGGSYVALTDGLGNLTIIIETMSHKHSKCIRPFLPYFNVSQQFATFVLKGSFSEIPELQVWYTKLGKTSERFLFKQLDSLWLLDSDGSFTLSLHEDELFTLTTLTTGRKGSYPLPPKSQPFPSTYKDDFNVDYPFFSEAPNFADQTGVFEYFTNIEDPGEHHFTLRQVLNQRPITWAADASNTISIIGDYNWTNLTIKCDVYIETPDTGGVFIAGRVNKGGILIRSARGIFFWIFANGSYRVTGDLAGWIIYALGRVEVTAKKWYTLTLTIKGHFTSGMLNDKSLWTDIPVNFPKNGWAAIGTHSFEFAQFDNFLVEATRGGGGSDAHKSEVAHRFKDLGEENFKALVLIAFAQYLQQCPFEDHVKLVNEVTEFAKTCVADESAENCDKSLHTLFGDKLCTVATLRETYGEMADCCAKQEPERNECFLQHKDDNPNLPRLVRPEVDVMCTAFHDNEETFLKKYLYEIARRHPYFYAPELLFFAKRYKAAFTECCQAADKAACLLPKLDELRDEGKASSAKQRLKCASLQKFGERAFKAWAVARLSQRFPKAEFAEVSKLVTDLTKVHTECCHGDLLECADDRADLAKYICENQDSISSKLKECCEKPLLEKSHCIAEVENDEMPADLPSLAADFVESKDVCKNYAEAKDVFLGMFLYEYARRHPDYSVVLLLRLAKTYETTLEKCCAAADPHECYAKVFDEFKPLVEEPQNLIKQNCELFEQLGEYKFQNALLVRYTKKVPQVSTPTLVEVSRNLGKVGSKCCKHPEAKRMPCAEDYLSVVLNQLCVLHEKTPVSDRVTKCCTESLVNRRPCFSALEVDETYVPKEFNAETFTFHADICTLSEKERQIKKQTALVELVKHKPKATKEQLKAVMDDFAAFVEKCCKADDKETCFAEEGKKLVAASQAALGLGGGGSGGGGSGGGGSEVQLVQSGAEVKKPGESLKISCKGSGYSFMNYWLGWVRQMPGKGLEWMGDIYPGGDYPTYSEKFKVQVTISADKSISTAYLQLSSLKASDTAMYYCARSGNYDEVAYWGQGTLVTVSSASTKGPSVFPLAPSSKSTSGGTAALGCLVKDYFPEPVTVSWNSGALTSGVHTFPAVLQSSGLYSLSSVVTVPSSSLGTQTYICNVNHKPSNTKVDKKVEPKSCDKTHT

SEQ ID NO: 35 - DNA, 4413 bp, synthetic construct
  source 1..4413: mol_type = other DNA
tacgtgctggacgactctgacggactcggaagggagtttgacggcattggcgctgtgtccggaggcggcgctacatctcgtctgctggtgaattatcccgagccctaccggtcccagattttagactacctcttcaaacccaattttggagcctccctccacattttaaaggtggaaatcggcggcgacggacagacaaccgatggcaccgaacctagccatatgcactacgctttagacgagaactatttccggggctatgagtggtggctgatgaaggaggccaagaagaggaaccccaacattaccctcatcggactgccttggagctttcccggttggctgggcaaaggattcgactggccctacgtgaatttacagctgaccgcttactacgtggtgacttggattgtgggagccaagcggtaccacgatctcgacatcgattacattggcatctggaacgagcggagctacaacgctaactatatcaagattctgcggaaaatgctgaattaccaaggtttacagcgggtgaagatcatcgctagcgacaatttatgggaaagcatctccgctagcatgctgctggacgctgaactgttcaaagtcgtggatgtcatcggcgctcactatcccggcacccatagcgccaaggacgccaagctgaccggaaaaaagctgtggtccagcgaggatttcagcactttaaactccgatatgggagctggctgctggggccggattttaaaccagaactacatcaatggctacatgacaagcaccatcgcttggaatttagtggcctcctactacgagcagctgccctatggacggtgcggtttaatgacagcccaagagccttggagcggccattacgtggtggagagccccgtttgggtgagcgctcacaccacccagttcacccagcccggctggtactacctcaagaccgtcggacatctggagaagggcggctcctacgtggctttaactgatggtttaggcaatctgaccatcattatcgagaccatgtcccacaagcactccaagtgcatccggccctttctgccctacttcaacgtgtcccagcaattcgccacctttgtgctgaagggcagcttttccgagattcccgagctccaagtttggtacaccaagctgggaaaaaccagcgagaggtttttattcaagcaactggactctttatggctgctggacagcgatggctccttcacactgtctttacatgaggatgagctctttactttaaccactttaacaactggtcggaaaggctcctatcctttaccccccaagagccaacccttccccagcacctacaaggacgacttcaacgtggattaccccttcttctccgaggctcccaactttgctgaccagaccggcgtgttcgagtatttcaccaacatcgaggaccccggtgagcaccatttcaccctccggcaagttctgaaccaacggcctatcacttgggccgccgacgcttccaataccatctccattatcggcgactacaactggacaaatttaactatcaagtgcgacgtctacatcgagacccccgataccggaggcgtgtttatcgctggaagggtgaacaaaggcggcattttaatccggtccgctaggggcatctttttctggatcttcgctaacggcagctatcgggtgactggtgacctcgctggctggatcatttacgctctgggccgggtggaggtgacagccaagaagtggtacactttaactttaactattaagggacattttaccagcggcatgctgaacgacaaatctttatggaccgacatccccgtgaactttcccaagaatggctgggccgccatcggcacccattcctttgaattcgcccagttcgacaatttcctcgtggaagccacccggggatccgatgcacacaagagtgaggttgctcatcggtttaaagatttgggagaagaaaatttcaaagccttggtgttgattgcctttgctcagtatcttcagcagtgtccatttgaagatcatgtaaaattagtgaatgaagtaactgaatttgcaaaaacatgtgttgctgatgagtcagctgaaaattgtgacaaatcacttcataccctttttggagacaaattatgcacagttgcaactcttcgtgaaacctatggtgaaatggctgactgctgtgcaaaacaagaacctgagagaaatgaatgcttcttgcaacacaaagatgacaacccaaacctcccccgattggtgagaccagaggttgatgtgatgtgcactgcttttcatgacaatgaagagacatttttgaaaaaatacttatatgaaattgccagaagacatccttacttttatgccccggaactccttttctttgctaaaaggtataaagctgcttttacagaatgttgccaagctgctgataaagctgcctgcctgttgccaaagctcgatgaacttcgggatgaagggaaggcttcgtctgccaaacagagactcaagtgtgccagtctccaaaaatttggagaaagagctttcaaagcatgggcagtagctcgcctgagccagagatttcccaaagctgagtttgcagaagtttccaagttagtgacagatcttaccaaagtccacacggaatgctgccatggagatctgcttgaatgtgctgatgacagggcggaccttgccaagtatatctgtgaaaatcaagattcgatctccagtaaactgaaggaatgctgtgaaaaacctctgttggaaaaatcccactgcattgccgaagtggaaaatgatgagatgcctgctgacttgccttcattagctgctgattttgttgaaagtaaggatgtttgcaaaaactatgctgaggcaaaggatgtcttcctgggcatgtttttgtatgaatatgcaagaaggcatcctgattactctgtcgtgctgctgctgagacttgccaagacatatgaaaccactctagagaagtgctgtgccgctgcagatcctcatgaatgctatgccaaagtgttcgatgaatttaaacctcttgtggaagagcctcagaatttaatcaaacaaaattgtgagctttttgagcagcttggagagtacaaattccagaatgcgctattagttcgttacaccaagaaagtaccccaagtgtcaactccaactcttgtagaggtctcaagaaacctaggaaaagtgggcagcaaatgttgtaaacatcctgaagcaaaaagaatgccctgtgcagaagactatctatccgtggtcctgaaccagttatgtgtgttgcatgagaaaacgccagtaagtgacagagtcaccaaatgctgcacagaatccttggtgaacaggcgaccatgcttttcagctctggaagtcgatgaaacatacgttcccaaagagtttaatgctgaaacattcaccttccatgcagatatatgcacactttctgagaaggagagacaaatcaagaaacaaactgcacttgttgagctcgtgaaacacaagcccaaggcaacaaaagagcaactgaaagctgttatggatgatttcgcagcttttgtagagaagtgctgcaaggctgacgataaggagacctgctttgccgaggagggtaaaaaacttgttgctgcaagtcaagctgccttaggcttaggtggcggaggttcaggcggcggtgggtcgggaggtggtggaagcgaggtgcaactagtgcagtctggagcagaggtgaaaaagcccggggagtctctgaagatttcctgtaagggttctggatacagctttatgaactactggctgggatgggtgcgccagatgcccgggaaaggcctggagtggatgggggacatctaccccggcggagactaccctacatacagcgagaagttcaaggtccaggtcaccatctcagccgacaagtccatcagcaccgcctacctgcagttgagcagcctgaaggcctcggacaccgccatgtattactgtgcgagatcaggcaattacgacgaagtggcctactggggccaaggaaccctggtcaccgtctcctcagctagcaccaagggcccatcggtcttccccctggcaccctcctccaagagcacctctgggggcacagcggccctgggctgcctggtcaaggactacttccccgaaccggtgacggtgtcgtggaactcaggcgccctgaccagcggcgtgcacaccttcccggctgtcctacagtcctcaggactctactccctcagcagcgtggtgaccgtgccctccagcagcttgggcacccagacctacatctgcaacgtgaatcacaagcccagcaacaccaaggtggacaagaaagttgagccgaagagctgtgataagacgcatacg

SEQ ID NO: 36 - DNA, 657 bp, synthetic construct
  source 1..657: mol_type = other DNA
gacatcgtgatgacccagactcccctgagcctgagcgtgacacctggccagcctgccagcatcagctgcagaagctctcagagcctggtgcacagcaacggcaacacctacctgcactggtatctgcagaagcccggccagagccctcagctgctgatctacaaggtgtccaacagattcagcggcgtgcccgacagattctccggcagcggctctggcaccgacttcaccctgaagatttccagagtggaagccgaggacgtgggcgtgtactactgcagccagagcacccacgtgccctggacattcggccagggcaccaaggtggaaatcaagagaaccgtggccgctcccagcgtgttcatcttcccacctagcgacgagcagctgaagtccggcacagcctctgtcgtgtgcctgctgaacaacttctacccccgcgaggccaaggtgcagtggaaggtggacaacgccctgcagagcggcaacagccaggaaagcgtgaccgagcaggactccaaggacagcacctacagcctgagcagcaccctgaccctgagcaaggccgactacgagaagcacaaggtgtacgcctgcgaagtgacccaccagggcctgtctagccccgtgaccaagagcttcaacagaggcgagtgc

SEQ ID NO: 37 - protein, 497 aa, Homo sapiens
ARPCIPKSFGYSSVVCVCNATYCDSFDPPTFPALGTFSRYESTRSGRRMELSMGPIQANHTGTGLLLTLQPEQKFQKVKGFGGAMTDAAALNILALSPPAQNLLLKSYFSEEGIGYNIIRVPMASCDFSIRTYTYADTPDDFQLHNFSLPEEDTKLKIPLIHRALQLAQRPVSLLASPWTSPTWLKTNGAVNGKGSLKGQPGDIYHQTWARYFVKFLDAYAEHKLQFWAVTAENEPSAGLLSGYPFQCLGFTPEHQRDFIARDLGPTLANSTHHNVRLLMLDDQRLLLPHWAKVVLTDPEAAKYVHGIAVHWYLDFLAPAKATLGETHRLFPNTMLFASEACVGSKFWEQSVRLGSWDRGMQYSHSIITNLLYHVVGWTDWNLALNPEGGPNWVRNFVDSPIIVDITKDTFYKQPMFYHLGHFSKFIPEGSQRVGLVASQKNDLDAVALMHPDGSAVVVVLNRSSKDVPLTIKDPAVGFLETISPGYSIHTYLWRRQ

SEQ ID NO: 38 - DNA, 1491 bp, synthetic construct
  source 1..1491: mol_type = other DNA
gctaggccatgcatcccaaaatcctttggctactcctccgtggtctgtgtctgcaacgctacttactgcgatagcttcgacccaccaacattcccagccctcggcacattctctaggtacgaaagcactaggagcggcagaagaatggaactgagcatgggcccaatccaagccaaccacactggcactggactgctcctcactctgcaaccagagcagaagttccagaaggtgaagggattcggcggcgctatgactgatgccgccgctctgaacattctcgctctcagccctccagcccagaatctgctgctgaagagctacttcagcgaagagggcatcggctacaatattattagggtgcctatggctagctgcgacttcagcattaggacttacacatacgccgacacaccagacgactttcagctgcataacttctctctgccagaggaggacactaagctcaagatcccactcatccatagggctctccaactggcccagaggccagtgtctctgctcgcctccccatggacttccccaacttggctgaagacaaacggcgctgtcaatggcaaaggctctctgaagggccagcccggcgacatctaccaccagacatgggctaggtatttcgtcaagtttctggatgcctacgccgaacacaaactgcagttttgggccgtgactgctgaaaacgaaccatccgctggactgctgtccggctacccattccagtgcctcggcttcactccagagcaccagagggatttcatcgctagggatctgggacctactctggccaatagcactcaccacaacgtgagactgctgatgctggatgaccaaaggctgctgctcccacactgggctaaggtcgtgctgacagatccagaagctgctaagtacgtgcacggaattgccgtgcactggtacctcgactttctggctccagccaaagccacactgggcgagactcataggctctttccaaacactatgctcttcgcctccgaggcttgtgtgggatccaagttttgggagcagtccgtgaggctgggcagctgggataggggcatgcagtacagccactccatcatcacaaatctgctgtaccacgtggtgggctggactgactggaatctggctctgaatccagaaggcggccctaactgggtgaggaactttgtggacagccctattattgtggatattactaaggatactttttacaagcagcctatgttttatcatctgggccacttctccaagtttatcccagaaggcagccaaagggtcggcctcgtcgctagccagaaaaacgacctcgatgctgtcgctctcatgcatccagatggctccgctgtcgtcgtcgtcctcaataggagcagcaaggacgtgcctctcacaatcaaggatccagccgtgggcttcctcgagactattagccccggctacagcatccacacatatctctggagaaggcaa

SEQ ID NO: 39 - protein, 1087 aa, synthetic construct
DAHKSEVAHRFKDLGEENFKALVLIAFAQYLQQCPFEDHVKLVNEVTEFAKTCVADESAENCDKSLHTLFGDKLCTVATLRETYGEMADCCAKQEPERNECFLQHKDDNPNLPRLVRPEVDVMCTAFHDNEETFLKKYLYEIARRHPYFYAPELLFFAKRYKAAFTECCQAADKAACLLPKLDELRDEGKASSAKQRLKCASLQKFGERAFKAWAVARLSQRFPKAEFAEVSKLVTDLTKVHTECCHGDLLECADDRADLAKYICENQDSISSKLKECCEKPLLEKSHCIAEVENDEMPADLPSLAADFVESKDVCKNYAEAKDVFLGMFLYEYARRHPDYSVVLLLRLAKTYETTLEKCCAAADPHECYAKVFDEFKPLVEEPQNLIKQNCELFEQLGEYKFQNALLVRYTKKVPQVSTPTLVEVSRNLGKVGSKCCKHPEAKRMPCAEDYLSVVLNQLCVLHEKTPVSDRVTKCCTESLVNRRPCFSALEVDETYVPKEFNAETFTFHADICTLSEKERQIKKQTALVELVKHKPKATKEQLKAVMDDFAAFVEKCCKADDKETCFAEEGKKLVAASQAALGLGGGGSARPCIPKSFGYSSVVCVCNATYCDSFDPPTFPALGTFSRYESTRSGRRMELSMGPIQANHTGTGLLLTLQPEQKFQKVKGFGGAMTDAAALNILALSPPAQNLLLKSYFSEEGIGYNIIRVPMASCDFSIRTYTYADTPDDFQLHNFSLPEEDTKLKIPLIHRALQLAQRPVSLLASPWTSPTWLKTNGAVNGKGSLKGQPGDIYHQTWARYFVKFLDAYAEHKLQFWAVTAENEPSAGLLSGYPFQCLGFTPEHQRDFIARDLGPTLANSTHHNVRLLMLDDQRLLLPHWAKVVLTDPEAAKYVHGIAVHWYLDFLAPAKATLGETHRLFPNTMLFASEACVGSKFWEQSVRLGSWDRGMQYSHSIITNLLYHVVGWTDWNLALNPEGGPNWVRNFVDSPIIVDITKDTFYKQPMFYHLGHFSKFIPEGSQRVGLVASQKNDLDAVALMHPDGSAVVVVLNRSSKDVPLTIKDPAVGFLETISPGYSIHTYLWRRQ

SEQ ID NO: 40 - DNA, 3261 bp, synthetic construct
  source 1..3261: mol_type = other DNA
gacgctcataagagcgaagtggcccataggttcaaggacctcggagaggaaaacttcaaagctctggtgctgatcgctttcgctcagtatctgcaacagtgccctttcgaggaccatgtgaaactggtgaacgaggtgactgaattcgctaagacttgcgtcgccgacgaaagcgctgagaattgcgacaagtctctgcatacactgttcggcgacaagctgtgtacagtcgctacactgagggagacttatggagagatggctgactgctgtgccaaacaagagccagagaggaacgagtgctttctgcaacacaaggacgataaccctaatctgccaagactcgtgaggccagaggtcgacgtcatgtgcacagctttccacgacaacgaagaaacatttctgaagaaatatctgtatgagatcgccagaaggcacccatacttctacgctccagagctgctgttctttgccaagaggtacaaagccgctttcactgagtgctgtcaagccgctgataaagccgcttgtctcctccctaaactggacgagctgagggacgagggaaaagcttcctccgccaagcagagactgaaatgcgcctctctgcagaagtttggcgaaagggccttcaaggcttgggctgtggccagactcagccagagattcccaaaggccgaatttgccgaagtgtccaagctggtgactgatctgactaaggtgcacactgaatgctgccatggagatctgctggaatgcgctgacgatagggctgacctcgctaagtacatctgcgagaaccaagattccatcagcagcaaactgaaggaatgctgtgagaaacctctgctcgagaagagccactgtatcgctgaggtcgaaaatgacgagatgccagccgatctcccatctctggccgctgacttcgtcgagtccaaggatgtgtgcaaaaactacgccgaggccaaggacgtgtttctgggcatgtttctgtacgagtacgctaggagacatccagattattccgtggtgctgctgctgaggctggccaaaacatacgagactactctggaaaagtgctgcgccgctgccgatccacacgaatgctacgccaaggtgttcgacgagttcaagccactcgtggaggagcctcagaatctgattaagcagaactgcgaactgttcgaacagctcggcgagtacaagttccagaatgctctgctcgtgaggtacactaagaaggtcccacaagtgtccactcctactctcgtcgaggtgtctaggaatctcggaaaggtcggatccaagtgctgtaagcacccagaggctaagagaatgccatgtgccgaggactatctgagcgtggtgctgaatcagctctgtgtgctgcacgagaaaactccagtgagcgatagggtgactaagtgttgtacagagtctctggtgaatagaaggccttgctttagcgctctggaggtggatgaaacatacgtcccaaaggaattcaatgccgagactttcactttccacgccgatatctgcacactctccgagaaagagaggcagatcaagaaacagacagctctggtggaactcgtcaagcacaagccaaaggccactaaagagcagctgaaggccgtgatggatgacttcgccgcctttgtggagaaatgctgcaaagccgatgataaggaaacatgcttcgccgaggagggaaagaagctcgtcgctgccagccaagctgctctgggactgggaggcggaggcagcgctagaccatgtatcccaaagagcttcggctacagctccgtcgtctgcgtctgtaatgctacttattgcgacagcttcgaccctccaacttttccagctctgggcacattctctaggtacgagtccacaaggtccggaaggaggatggaactgagcatgggcccaattcaagccaaccatactggcactggactgctgctgactctccagccagagcagaagttccagaaggtcaaaggattcggcggagccatgacagatgctgctgctctgaatattctggctctcagccctccagcccaaaatctgctgctgaaaagctatttctccgaggagggcattggctacaacatcattagggtgcctatggccagctgtgactttagcattaggacttacacttacgccgacacaccagacgacttccagctccacaatttctctctgccagaagaagacactaagctgaagattcctctcattcacagagctctgcagctggctcagagaccagtgtctctgctcgcctccccatggacatccccaacttggctgaaaacaaacggcgccgtgaacggaaaaggctccctcaaaggccaacccggcgatatctaccaccagacttgggctaggtacttcgtcaagtttctggacgcttatgccgagcataagctgcaattctgggccgtgactgccgagaacgagccatccgctggactgctgagcggatatccattccagtgtctcggcttcacaccagagcaccaaagggactttatcgctagggatctgggaccaactctggctaacagcacacaccacaacgtgaggctcctcatgctggacgatcagaggctgctgctgccacactgggctaaggtggtgctgacagacccagaggctgccaaatacgtccatggaatcgccgtgcattggtatctggattttctggccccagccaaggctacactcggagagacacataggctcttccctaacactatgctcttcgcttccgaagcttgtgtcggctccaagttttgggagcagtccgtcagactgggaagctgggataggggaatgcagtacagccactccatcatcactaatctgctgtatcatgtcgtgggctggactgactggaacctcgctctgaacccagagggcggccctaactgggtgaggaacttcgtcgacagcccaatcattgtggatattactaaggatacattttataaacagcctatgttctaccatctcggccacttctccaagttcatcccagagggatcccagagggtgggcctcgtggcttcccagaagaatgatctggatgctgtcgctctgatgcacccagatggatccgccgtggtggtggtgctgaataggagcagcaaggatgtccctctcacaatcaaagatccagccgtgggctttctcgagacaatcagccccggctatagcatccacacatatctgtggagaagacag

SEQ ID NO: 41 - protein, 1087 aa, synthetic construct
ARPCIPKSFGYSSVVCVCNATYCDSFDPPTFPALGTFSRYESTRSGRRMELSMGPIQANHTGTGLLLTLQPEQKFQKVKGFGGAMTDAAALNILALSPPAQNLLLKSYFSEEGIGYNIIRVPMASCDFSIRTYTYADTPDDFQLHNFSLPEEDTKLKIPLIHRALQLAQRPVSLLASPWTSPTWLKTNGAVNGKGSLKGQPGDIYHQTWARYFVKFLDAYAEHKLQFWAVTAENEPSAGLLSGYPFQCLGFTPEHQRDFIARDLGPTLANSTHHNVRLLMLDDQRLLLPHWAKVVLTDPEAAKYVHGIAVHWYLDFLAPAKATLGETHRLFPNTMLFASEACVGSKFWEQSVRLGSWDRGMQYSHSIITNLLYHVVGWTDWNLALNPEGGPNWVRNFVDSPIIVDITKDTFYKQPMFYHLGHFSKFIPEGSQRVGLVASQKNDLDAVALMHPDGSAVVVVLNRSSKDVPLTIKDPAVGFLETISPGYSIHTYLWRRQGGGGSDAHKSEVAHRFKDLGEENFKALVLIAFAQYLQQCPFEDHVKLVNEVTEFAKTCVADESAENCDKSLHTLFGDKLCTVATLRETYGEMADCCAKQEPERNECFLQHKDDNPNLPRLVRPEVDVMCTAFHDNEETFLKKYLYEIARRHPYFYAPELLFFAKRYKAAFTECCQAADKAACLLPKLDELRDEGKASSAKQRLKCASLQKFGERAFKAWAVARLSQRFPKAEFAEVSKLVTDLTKVHTECCHGDLLECADDRADLAKYICENQDSISSKLKECCEKPLLEKSHCIAEVENDEMPADLPSLAADFVESKDVCKNYAEAKDVFLGMFLYEYARRHPDYSVVLLLRLAKTYETTLEKCCAAADPHECYAKVFDEFKPLVEEPQNLIKQNCELFEQLGEYKFQNALLVRYTKKVPQVSTPTLVEVSRNLGKVGSKCCKHPEAKRMPCAEDYLSVVLNQLCVLHEKTPVSDRVTKCCTESLVNRRPCFSALEVDETYVPKEFNAETFTFHADICTLSEKERQIKKQTALVELVKHKPKATKEQLKAVMDDFAAFVEKCCKADDKETCFAEEGKKLVAASQAALGL

SEQ ID NO: 42 - DNA, 3276 bp, synthetic construct
  source 1..3276: mol_type = other DNA
gctaggccatgcatcccaaaatcctttggctactcctccgtggtctgtgtctgcaacgctacttactgcgatagcttcgacccaccaacattcccagccctcggcacattctctaggtacgaaagcactaggagcggcagaagaatggaactgagcatgggcccaatccaagccaaccacactggcactggactgctcctcactctgcaaccagagcagaagttccagaaggtgaagggattcggcggcgctatgactgatgccgccgctctgaacattctcgctctcagccctccagcccagaatctgctgctgaagagctacttcagcgaagagggcatcggctacaatattattagggtgcctatggctagctgcgacttcagcattaggacttacacatacgccgacacaccagacgactttcagctgcataacttctctctgccagaggaggacactaagctcaagatcccactcatccatagggctctccaactggcccagaggccagtgtctctgctcgcctccccatggacttccccaacttggctgaagacaaacggcgctgtcaatggcaaaggctctctgaagggccagcccggcgacatctaccaccagacatgggctaggtatttcgtcaagtttctggatgcctacgccgaacacaaactgcagttttgggccgtgactgctgaaaacgaaccatccgctggactgctgtccggctacccattccagtgcctcggcttcactccagagcaccagagggatttcatcgctagggatctgggacctactctggccaatagcactcaccacaacgtgagactgctgatgctggatgaccaaaggctgctgctcccacactgggctaaggtcgtgctgacagatccagaagctgctaagtacgtgcacggaattgccgtgcactggtacctcgactttctggctccagccaaagccacactgggcgagactcataggctctttccaaacactatgctcttcgcctccgaggcttgtgtgggatccaagttttgggagcagtccgtgaggctgggcagctgggataggggcatgcagtacagccactccatcatcacaaatctgctgtaccacgtggtgggctggactgactggaatctggctctgaatccagaaggcggccctaactgggtgaggaactttgtggacagccctattattgtggatattactaaggatactttttacaagcagcctatgttttatcatctgggccacttctccaagtttatcccagaaggcagccaaagggtcggcctcgtcgctagccagaaaaacgacctcgatgctgtcgctctcatgcatccagatggctccgctgtcgtcgtcgtcctcaataggagcagcaaggacgtgcctctcacaatcaaggatccagccgtgggcttcctcgagactattagccccggctacagcatccacacatatctctggagaaggcaaggcggcggaggctccgatgctcataaatccgaggtcgctcataggttcaaggatctcggcgaggagaacttcaaggctctcgtgctgatcgcctttgcccagtacctccaacagtgtcctttcgaggaccatgtgaagctggtcaacgaagtgacagagttcgccaaaacttgcgtggccgacgagagcgccgagaactgcgataagtctctgcatacactgttcggcgacaagctctgcactgtcgccacactgagggagacatacggagaaatggccgactgttgtgctaagcaagagccagagaggaacgagtgctttctgcaacacaaggatgacaaccctaacctcccaaggctggtgaggccagaagtcgacgtgatgtgcacagctttccacgataacgaggagacttttctgaagaagtacctctacgagattgctaggagacacccttatttctacgccccagaactgctgttcttcgccaagaggtacaaggccgccttcactgagtgttgccaagccgctgacaaggctgcttgcctcctcccaaagctcgatgagctgagggacgagggaaaggctagctccgccaagcaaaggctgaagtgcgcctctctgcagaagtttggcgagagagccttcaaggcttgggctgtggccagactcagccagaggtttccaaaggccgagttcgctgaggtcagcaagctggtgacagatctgacaaaagtccacactgagtgctgccacggagatctgctggagtgtgctgatgacagagccgatctggccaagtacatctgtgagaaccaagactccatcagcagcaaactgaaggagtgctgtgagaagccactgctggaaaagagccactgcatcgccgaggtcgagaacgatgagatgccagctgatctgccatctctggccgctgacttcgtggagagcaaggacgtctgtaagaactacgctgaagccaaggatgtctttctgggcatgttcctctatgagtacgctaggaggcacccagattacagcgtcgtgctgctgctgagactcgccaagacttacgagactactctcgagaagtgctgcgccgccgccgatcctcatgagtgctacgctaaggtgtttgatgagtttaaacctctcgtcgaggagccacagaacctcatcaaacaaaattgtgagctcttcgagcagctgggcgagtacaagttccaaaacgctctgctggtgaggtacacaaagaaagtgccacaagtgtccacacctactctcgtggaggtgtctaggaatctgggcaaggtcggctccaagtgttgcaaacacccagaggccaaaaggatgccttgcgctgaggactatctgtccgtggtgctgaaccagctgtgcgtcctccacgaaaagacaccagtgagcgatagggtcactaagtgttgcacagagtccctcgtcaataggaggccatgtttttccgctctggaggtggacgaaacttacgtgcctaaggaattcaacgccgaaacattcacattccatgccgacatttgtacactgagcgagaaggagaggcagatcaagaagcagacagctctggtggagctcgtcaagcacaagccaaaagccactaaggagcagctgaaggctgtcatggatgacttcgctgccttcgtcgagaaatgctgtaaggccgacgacaaggagacatgtttcgccgaggagggcaaaaagctcgtcgccgccagccaagccgctctcggactgggcggcggaggctcc

SEQ ID NO: 43 - protein, 496 aa, Mus musculus
AQPCIPKSFGYSSVVCVCNASYCDSLDPVTLPALGTFSRYESTRRGRRMELSVGAIQANRTGTGLLLTLQPEKKFQKVKGFGGAMTDATALNILALSPPTQKLLLRSYFSTNGIEYNIIRVPMASCDFSIRVYTYADTPNDFQLSNFSLPEEDTKLKIPLIHQALKMSSRPISLFASPWTSPTWLKTNGRVNGKGSLKGQPGDIFHQTWANYFVKFLDAYAKYGLRFWAVTAENEPTAGLFTGYPFQCLGFTPEHQRDFISRDLGPALANSSHDVKLLMLDDQRLLLPRWAEVVLSDPEAAKYVHGIAVHWYMDFLAPAKATLGETHRLFPNTMLFASEACVGSKFWEQSVRLGSWDRGMQYSHSIITNLLYHVTGWTDWNLALNPEGGPNWVRNFVDSPIIVDIPKDAFYKQPMFYHLGHFSKFIPEGSQRVALVASESTDLETVALLRPDGSAVVVVLNRSSEDVPLTISDPDLGFLETVSPGYSIHTYLWRRQ

SEQ ID NO: 44 - DNA, 1488 bp, synthetic construct
  source 1..1488: mol_type = other DNA
gcccagccttgcatccctaagtcctttggctactccagcgtcgtgtgcgtctgcaatgctagctactgtgactctctggacccagtgacactgccagctctgggaactttctctaggtacgagagcactaggagaggcagaaggatggaactgagcgtgggagccatccaagccaataggactggcactggactgctgctgacactgcagccagagaagaagtttcaaaaagtcaaaggcttcggcggcgctatgacagacgctactgctctgaacattctggctctgagcccacctactcagaagctgctgctgaggagctacttcagcactaacggaatcgaatacaacattattagggtgcctatggccagctgtgacttctccattagggtctacacatacgccgacactcctaacgacttccagctgagcaacttctctctgccagaggaagacacaaagctgaagatccctctcatccaccaagccctcaagatgagctctaggcctatctctctgttcgcttccccttggacttcccctacatggctgaagacaaacggaagggtgaacggcaaaggctctctgaagggccaacccggcgacatcttccaccagacttgggccaactatttcgtcaagtttctggacgcctatgccaagtatggactgaggttttgggctgtgactgccgagaatgagcctactgccggactgttcactggatacccattccagtgcctcggattcacaccagagcaccagagggactttatctctagggatctgggaccagccctcgccaatagctcccatgacgtcaagctgctcatgctcgacgaccagaggctgctgctgcctagatgggccgaggtcgtgctgagcgacccagaagccgctaagtatgtgcatggcatcgccgtgcactggtacatggattttctggctccagccaaggctactctgggagagactcataggctgttcccaaacactatgctcttcgccagcgaggcttgtgtgggctccaagttttgggagcaaagcgtcagactgggcagctgggacagaggcatgcagtattcccactccatcatcacaaatctgctgtaccacgtgactggctggactgattggaacctcgctctgaatccagagggcggccctaattgggtgagaaacttcgtcgactccccaatcatcgtcgacatccctaaggacgctttctacaaacagccaatgttctaccacctcggccacttctccaagttcattccagagggctcccagagagtcgccctcgtggctagcgagtccactgatctggaaacagtcgctctgctgaggccagatggcagcgctgtggtggtcgtgctgaatagatcctccgaggatgtccctctgacaatctccgatcccgatctgggctttctggagacagtgagccccggctactccatccacacatatctgtggaggaggcag

SEQ ID NO: 45 - protein, 1085 aa, synthetic construct
EAHKSEIAHRYNDLGEQHFKGLVLIAFSQYLQKCSYDEHAKLVQEVTDFAKTCVADESAANCDKSLHTLFGDKLCAIPNLRENYGELADCCTKQEPERNECFLQHKDDNPSLPPFERPEAEAMCTSFKENPTTFMGHYLHEVARRHPYFYAPELLYYAEQYNEILTQCCAEADKESCLTPKLDGVKEKALVSSVRQRMKCSSMQKFGERAFKAWAVARLSQTFPNADFAEITKLATDLTKVNKECCHGDLLECADDRAELAKYMCENQATISSKLQTCCDKPLLKKAHCLSEVEHDTMPADLPAIAADFVEDQEVCKNYAEAKDVFLGTFLYEYSRRHPDYSVSLLLRLAKKYEATLEKCCAEANPPACYGTVLAEFQPLVEEPKNLVKTNCDLYEKLGEYGFQNAILVRYTQKAPQVSTPTLVEAARNLGRVGTKCCTLPEDQRLPCVEDYLSAILNRVCLLHEKTPVSEHVTKCCSGSLVERRPCFSALTVDETYVPKEFKAETFTFHSDICTLPEKEKQIKKQTALAELVKHKPKATAEQLKTVMDDFAQFLDTCCKAADKDTCFSTEGPNLVTRCKDALAGGGGSAQPCIPKSFGYSSVVCVCNASYCDSLDPVTLPALGTFSRYESTRRGRRMELSVGAIQANRTGTGLLLTLQPEKKFQKVKGFGGAMTDATALNILALSPPTQKLLLRSYFSTNGIEYNIIRVPMASCDFSIRVYTYADTPNDFQLSNFSLPEEDTKLKIPLIHQALKMSSRPISLFASPWTSPTWLKTNGRVNGKGSLKGQPGDIFHQTWANYFVKFLDAYAKYGLRFWAVTAENEPTAGLFTGYPFQCLGFTPEHQRDFISRDLGPALANSSHDVKLLMLDDQRLLLPRWAEVVLSDPEAAKYVHGIAVHWYMDFLAPAKATLGETHRLFPNTMLFASEACVGSKFWEQSVRLGSWDRGMQYSHSIITNLLYHVTGWTDWNLALNPEGGPNWVRNFVDSPIIVDIPKDAFYKQPMFYHLGHFSKFIPEGSQRVALVASESTDLETVALLRPDGSAVVVVLNRSSEDVPLTISDPDLGFLETVSPGYSIHTYLWRRQ

SEQ ID NO: 46 - DNA, 3255 bp, synthetic construct
  source 1..3255: mol_type = other DNA
gaggctcacaagagcgaaatcgctcatcgttacaacgatttaggcgagcagcacttcaagggtttagttttaatcgctttctcccagtacctccagaagtgctcctacgacgagcatgccaagctcgtgcaagaggtgaccgactttgctaagacttgtgtggccgatgagtccgccgctaactgcgataagtctttacacaccctctttggagacaaactgtgcgccatccctaatctgcgggagaactacggcgagctggccgattgctgcacaaagcaagaacccgaaaggaacgagtgtttcctccagcacaaagacgacaacccttctttacctccctttgagaggcccgaggccgaggctatgtgtacctccttcaaggaaaaccccacaacattcatgggacattatttacatgaggtcgctcggcggcacccttacttctacgcccccgagctgctgtattacgccgagcagtacaacgagattctgacccagtgttgtgccgaagctgataaagagagctgtttaacacccaagctggatggcgtgaaggaaaaggctttagtcagcagcgtgaggcagaggatgaaatgctcctccatgcaaaagttcggcgaacgggcctttaaggcttgggctgtggctcgtctgagccagacattccccaacgccgacttcgccgagattaccaaactcgccaccgatctgacaaaggtcaacaaggagtgctgccatggtgatttactggagtgcgccgacgatagggccgaactcgctaaatacatgtgcgagaaccaagctaccatctccagcaagctgcagacttgttgtgataaacccctcctcaagaaggctcactgtttatccgaggtcgagcacgacacaatgcccgctgatctgcccgctatcgccgctgattttgtggaagaccaagaagtctgtaagaattacgctgaggctaaggatgtgtttctcggcacctttttatacgaatatagccggaggcaccccgattatagcgtcagcctcttattacggctggctaagaagtatgaggccacactggaaaagtgctgtgccgaggctaaccctcccgcttgttacggaaccgtgctggctgaatttcagcctttagtcgaggagcccaagaatctggtgaagaccaactgtgatctgtacgaaaagctgggcgagtatggcttccaaaacgccattttagtgcggtatacacagaaggccccccaagtttccacccccacactggtcgaagctgcccggaatctgggacgggtgggcaccaagtgttgcactttacccgaggaccagaggctgccttgcgtggaggactacctcagcgctatcctcaatcgtgtctgtttactgcacgaaaagacacccgttagcgaacacgtgacaaagtgctgctccggctctttagtggaacggaggccttgctttagcgctttaacagtggacgaaacctacgtgcctaaggagtttaaggccgagaccttcacctttcactccgacatctgcactttacccgaaaaagagaagcagatcaaaaagcagaccgccctcgccgagctcgtcaaacataagcctaaggctaccgccgaacagctcaaaaccgtgatggacgacttcgcccaatttttagatacatgctgcaaggccgccgacaaggacacttgtttttccaccgagggccccaatttagtcactcgttgcaaggatgctttagctggcggcggaggctccgcccagccttgcatccctaagtcctttggctactccagcgtcgtgtgcgtctgcaatgctagctactgtgactctctggacccagtgacactgccagctctgggaactttctctaggtacgagagcactaggagaggcagaaggatggaactgagcgtgggagccatccaagccaataggactggcactggactgctgctgacactgcagccagagaagaagtttcaaaaagtcaaaggcttcggcggcgctatgacagacgctactgctctgaacattctggctctgagcccacctactcagaagctgctgctgaggagctacttcagcactaacggaatcgaatacaacattattagggtgcctatggccagctgtgacttctccattagggtctacacatacgccgacactcctaacgacttccagctgagcaacttctctctgccagaggaagacacaaagctgaagatccctctcatccaccaagccctcaagatgagctctaggcctatctctctgttcgcttccccttggacttcccctacatggctgaagacaaacggaagggtgaacggcaaaggctctctgaagggccaacccggcgacatcttccaccagacttgggccaactatttcgtcaagtttctggacgcctatgccaagtatggactgaggttttgggctgtgactgccgagaatgagcctactgccggactgttcactggatacccattccagtgcctcggattcacaccagagcaccagagggactttatctctagggatctgggaccagccctcgccaatagctcccatgacgtcaagctgctcatgctcgacgaccagaggctgctgctgcctagatgggccgaggtcgtgctgagcgacccagaagccgctaagtatgtgcatggcatcgccgtgcactggtacatggattttctggctccagccaaggctactctgggagagactcataggctgttcccaaacactatgctcttcgccagcgaggcttgtgtgggctccaagttttgggagcaaagcgtcagactgggcagctgggacagaggcatgcagtattcccactccatcatcacaaatctgctgtaccacgtgactggctggactgattggaacctcgctctgaatccagagggcggccctaattgggtgagaaacttcgtcgactccccaatcatcgtcgacatccctaaggacgctttctacaaacagccaatgttctaccacctcggccacttctccaagttcattccagagggctcccagagagtcgccctcgtggctagcgagtccactgatctggaaacagtcgctctgctgaggccagatggcagcgctgtggtggtcgtgctgaatagatcctccgaggatgtccctctgacaatctccgatcccgatctgggctttctggagacagtgagccccggctactccatccacacatatctgtggaggaggcag

SEQ ID NO: 47 - protein, 1085 aa, synthetic construct
AQPCIPKSFGYSSVVCVCNASYCDSLDPVTLPALGTFSRYESTRRGRRMELSVGAIQANRTGTGLLLTLQPEKKFQKVKGFGGAMTDATALNILALSPPTQKLLLRSYFSTNGIEYNIIRVPMASCDFSIRVYTYADTPNDFQLSNFSLPEEDTKLKIPLIHQALKMSSRPISLFASPWTSPTWLKTNGRVNGKGSLKGQPGDIFHQTWANYFVKFLDAYAKYGLRFWAVTAENEPTAGLFTGYPFQCLGFTPEHQRDFISRDLGPALANSSHDVKLLMLDDQRLLLPRWAEVVLSDPEAAKYVHGIAVHWYMDFLAPAKATLGETHRLFPNTMLFASEACVGSKFWEQSVRLGSWDRGMQYSHSIITNLLYHVTGWTDWNLALNPEGGPNWVRNFVDSPIIVDIPKDAFYKQPMFYHLGHFSKFIPEGSQRVALVASESTDLETVALLRPDGSAVVVVLNRSSEDVPLTISDPDLGFLETVSPGYSIHTYLWRRQGGGGSEAHKSEIAHRYNDLGEQHFKGLVLIAFSQYLQKCSYDEHAKLVQEVTDFAKTCVADESAANCDKSLHTLFGDKLCAIPNLRENYGELADCCTKQEPERNECFLQHKDDNPSLPPFERPEAEAMCTSFKENPTTFMGHYLHEVARRHPYFYAPELLYYAEQYNEILTQCCAEADKESCLTPKLDGVKEKALVSSVRQRMKCSSMQKFGERAFKAWAVARLSQTFPNADFAEITKLATDLTKVNKECCHGDLLECADDRAELAKYMCENQATISSKLQTCCDKPLLKKAHCLSEVEHDTMPADLPAIAADFVEDQEVCKNYAEAKDVFLGTFLYEYSRRHPDYSVSLLLRLAKKYEATLEKCCAEANPPACYGTVLAEFQPLVEEPKNLVKTNCDLYEKLGEYGFQNAILVRYTQKAPQVSTPTLVEAARNLGRVGTKCCTLPEDQRLPCVEDYLSAILNRVCLLHEKTPVSEHVTKCCSGSLVERRPCFSALTVDETYVPKEFKAETFTFHSDICTLPEKEKQIKKQTALAELVKHKPKATAEQLKTVMDDFAQFLDTCCKAADKDTCFSTEGPNLVTRCKDALA

SEQ ID NO: 48 - DNA, 3255 bp, synthetic construct
  source 1..3255: mol_type = other DNA
gcccagccttgcatccctaagtcctttggctactccagcgtcgtgtgcgtctgcaatgctagctactgtgactctctggacccagtgacactgccagctctgggaactttctctaggtacgagagcactaggagaggcagaaggatggaactgagcgtgggagccatccaagccaataggactggcactggactgctgctgacactgcagccagagaagaagtttcaaaaagtcaaaggcttcggcggcgctatgacagacgctactgctctgaacattctggctctgagcccacctactcagaagctgctgctgaggagctacttcagcactaacggaatcgaatacaacattattagggtgcctatggccagctgtgacttctccattagggtctacacatacgccgacactcctaacgacttccagctgagcaacttctctctgccagaggaagacacaaagctgaagatccctctcatccaccaagccctcaagatgagctctaggcctatctctctgttcgcttccccttggacttcccctacatggctgaagacaaacggaagggtgaacggcaaaggctctctgaagggccaacccggcgacatcttccaccagacttgggccaactatttcgtcaagtttctggacgcctatgccaagtatggactgaggttttgggctgtgactgccgagaatgagcctactgccggactgttcactggatacccattccagtgcctcggattcacaccagagcaccagagggactttatctctagggatctgggaccagccctcgccaatagctcccatgacgtcaagctgctcatgctcgacgaccagaggctgctgctgcctagatgggccgaggtcgtgctgagcgacccagaagccgctaagtatgtgcatggcatcgccgtgcactggtacatggattttctggctccagccaaggctactctgggagagactcataggctgttcccaaacactatgctcttcgccagcgaggcttgtgtgggctccaagttttgggagcaaagcgtcagactgggcagctgggacagaggcatgcagtattcccactccatcatcacaaatctgctgtaccacgtgactggctggactgattggaacctcgctctgaatccagagggcggccctaattgggtgagaaacttcgtcgactccccaatcatcgtcgacatccctaaggacgctttctacaaacagccaatgttctaccacctcggccacttctccaagttcattccagagggctcccagagagtcgccctcgtggctagcgagtccactgatctggaaacagtcgctctgctgaggccagatggcagcgctgtggtggtcgtgctgaatagatcctccgaggatgtccctctgacaatctccgatcccgatctgggctttctggagacagtgagccccggctactccatccacacatatctgtggaggaggcagggcggcggaggctccgaggctcacaagagcgaaatcgctcatcgttacaacgatttaggcgagcagcacttcaagggtttagttttaatcgctttctcccagtacctccagaagtgctcctacgacgagcatgccaagctcgtgcaagaggtgaccgactttgctaagacttgtgtggccgatgagtccgccgctaactgcgataagtctttacacaccctctttggagacaaactgtgcgccatccctaatctgcgggagaactacggcgagctggccgattgctgcacaaagcaagaacccgaaaggaacgagtgtttcctccagcacaaagacgacaacccttctttacctccctttgagaggcccgaggccgaggctatgtgtacctccttcaaggaaaaccccacaacattcatgggacattatttacatgaggtcgctcggcggcacccttacttctacgcccccgagctgctgtattacgccgagcagtacaacgagattctgacccagtgttgtgccgaagctgataaagagagctgtttaacacccaagctggatggcgtgaaggaaaaggctttagtcagcagcgtgaggcagaggatgaaatgctcctccatgcaaaagttcggcgaacgggcctttaaggcttgggctgtggctcgtctgagccagacattccccaacgccgacttcgccgagattaccaaactcgccaccgatctgacaaaggtcaacaaggagtgctgccatggtgatttactggagtgcgccgacgatagggccgaactcgctaaatacatgtgcgagaaccaagctaccatctccagcaagctgcagacttgttgtgataaacccctcctcaagaaggctcactgtttatccgaggtcgagcacgacacaatgcccgctgatctgcccgctatcgccgctgattttgtggaagaccaagaagtctgtaagaattacgctgaggctaaggatgtgtttctcggcacctttttatacgaatatagccggaggcaccccgattatagcgtcagcctcttattacggctggctaagaagtatgaggccacactggaaaagtgctgtgccgaggctaaccctcccgcttgttacggaaccgtgctggctgaatttcagcctttagtcgaggagcccaagaatctggtgaagaccaactgtgatctgtacgaaaagctgggcgagtatggcttccaaaacgccattttagtgcggtatacacagaaggccccccaagtttccacccccacactggtcgaagctgcccggaatctgggacgggtgggcaccaagtgttgcactttacccgaggaccagaggctgccttgcgtggaggactacctcagcgctatcctcaatcgtgtctgtttactgcacgaaaagacacccgttagcgaacacgtgacaaagtgctgctccggctctttagtggaacggaggccttgctttagcgctttaacagtggacgaaacctacgtgcctaaggagtttaaggccgagaccttcacctttcactccgacatctgcactttacccgaaaaagagaagcagatcaaaaagcagaccgccctcgccgagctcgtcaaacataagcctaaggctaccgccgaacagctcaaaaccgtgatggacgacttcgcccaatttttagatacatgctgcaaggccgccgacaaggacacttgtttttccaccgagggccccaatttagtcactcgttgcaaggatgctttagct

SEQ ID NO: 49 - DNA, 534 bp, synthetic construct
  source 1..534: mol_type = other DNA
atgcacagcagcgctctgctgtgttgtctggtgctgctgactggcgtcagagccagccccggccaaggcactcagagcgagaacagctgtactcatttccccggcaacctccctaatatgctgagggatctgagggacgccttctctagggtcaagacattcttccagatgaaggaccaactggacaatctgctgctgaaggaatctctgctggaggactttaagggctatctgggctgccaagccctctccgagatgatccagttttatctggaggaggtcatgcctcaagccgagaaccaagatccagacatcaaggctcacgtcaattctctgggcgaaaatctgaagacactgaggctgaggctcagaaggtgccatagatttctgccatgcgagaacaaaagcaaggctgtggagcaagtgaagaacgccttcaacaagctgcaagagaagggcatctataaggctatgagcgagtttgacatcttcatcaactatatcgaggcttacatgactatgaagattaggaac

SEQ ID NO: 50 - protein, 745 aa, synthetic construct
DAHKSEVAHRFKDLGEENFKALVLIAFAQYLQQCPFEDHVKLVNEVTEFAKTCVADESAENCDKSLHTLFGDKLCTVATLRETYGEMADCCAKQEPERNECFLQHKDDNPNLPRLVRPEVDVMCTAFHDNEETFLKKYLYEIARRHPYFYAPELLFFAKRYKAAFTECCQAADKAACLLPKLDELRDEGKASSAKQRLKCASLQKFGERAFKAWAVARLSQRFPKAEFAEVSKLVTDLTKVHTECCHGDLLECADDRADLAKYICENQDSISSKLKECCEKPLLEKSHCIAEVENDEMPADLPSLAADFVESKDVCKNYAEAKDVFLGMFLYEYARRHPDYSVVLLLRLAKTYETTLEKCCAAADPHECYAKVFDEFKPLVEEPQNLIKQNCELFEQLGEYKFQNALLVRYTKKVPQVSTPTLVEVSRNLGKVGSKCCKHPEAKRMPCAEDYLSVVLNQLCVLHEKTPVSDRVTKCCTESLVNRRPCFSALEVDETYVPKEFNAETFTFHADICTLSEKERQIKKQTALVELVKHKPKATKEQLKAVMDDFAAFVEKCCKADDKETCFAEEGKKLVAASQAALGLSPGQGTQSENSCTHFPGNLPNMLRDLRDAFSRVKTFFQMKDQLDNLLLKESLLEDFKGYLGCQALSEMIQFYLEEVMPQAENQDPDIKAHVNSLGENLKTLRLRLRRCHRFLPCENKSKAVEQVKNAFNKLQEKGIYKAMSEFDIFINYIEAYMTMKIRN

SEQ ID NO: 51 - DNA, 2235 bp, synthetic construct
  source 1..2235: mol_type = other DNA
gatgcacacaagagtgaggttgctcatcggtttaaagatttgggagaagaaaatttcaaagccttggtgttgattgcctttgctcagtatcttcagcagtgtccatttgaagatcatgtaaaattagtgaatgaagtaactgaatttgcaaaaacatgtgttgctgatgagtcagctgaaaattgtgacaaatcacttcataccctttttggagacaaattatgcacagttgcaactcttcgtgaaacctatggtgaaatggctgactgctgtgcaaaacaagaacctgagagaaatgaatgcttcttgcaacacaaagatgacaacccaaacctcccccgattggtgagaccagaggttgatgtgatgtgcactgcttttcatgacaatgaagagacatttttgaaaaaatacttatatgaaattgccagaagacatccttacttttatgccccggaactccttttctttgctaaaaggtataaagctgcttttacagaatgttgccaagctgctgataaagctgcctgcctgttgccaaagctcgatgaacttcgggatgaagggaaggcttcgtctgccaaacagagactcaagtgtgccagtctccaaaaatttggagaaagagctttcaaagcatgggcagtagctcgcctgagccagagatttcccaaagctgagtttgcagaagtttccaagttagtgacagatcttaccaaagtccacacggaatgctgccatggagatctgcttgaatgtgctgatgacagggcggaccttgccaagtatatctgtgaaaatcaagattcgatctccagtaaactgaaggaatgctgtgaaaaacctctgttggaaaaatcccactgcattgccgaagtggaaaatgatgagatgcctgctgacttgccttcattagctgctgattttgttgaaagtaaggatgtttgcaaaaactatgctgaggcaaaggatgtcttcctgggcatgtttttgtatgaatatgcaagaaggcatcctgattactctgtcgtgctgctgctgagacttgccaagacatatgaaaccactctagagaagtgctgtgccgctgcagatcctcatgaatgctatgccaaagtgttcgatgaatttaaacctcttgtggaagagcctcagaatttaatcaaacaaaattgtgagctttttgagcagcttggagagtacaaattccagaatgcgctattagttcgttacaccaagaaagtaccccaagtgtcaactccaactcttgtagaggtctcaagaaacctaggaaaagtgggcagcaaatgttgtaaacatcctgaagcaaaaagaatgccctgtgcagaagactatctatccgtggtcctgaaccagttatgtgtgttgcatgagaaaacgccagtaagtgacagagtcaccaaatgctgcacagaatccttggtgaacaggcgaccatgcttttcagctctggaagtcgatgaaacatacgttcccaaagagtttaatgctgaaacattcaccttccatgcagatatatgcacactttctgagaaggagagacaaatcaagaaacaaactgcacttgttgagctcgtgaaacacaagcccaaggcaacaaaagagcaactgaaagctgttatggatgatttcgcagcttttgtagagaagtgctgcaaggctgacgataaggagacctgctttgccgaggagggtaaaaaacttgttgctgcaagtcaagctgccttaggcttaagccccggccaaggcactcagagcgagaacagctgtactcatttccccggcaacctccctaatatgctgagggatctgagggacgccttctctagggtcaagacattcttccagatgaaggaccaactggacaatctgctgctgaaggaatctctgctggaggactttaagggctatctgggctgccaagccctctccgagatgatccagttttatctggaggaggtcatgcctcaagccgagaaccaagatccagacatcaaggctcacgtcaattctctgggcgaaaatctgaagacactgaggctgaggctcagaaggtgccatagatttctgccatgcgagaacaaaagcaaggctgtggagcaagtgaagaacgccttcaacaagctgcaagagaagggcatctataaggctatgagcgagtttgacatcttcatcaactatatcgaggcttacatgactatgaagattaggaac

SEQ ID NO: 52 - protein, 745 aa, synthetic construct
SPGQGTQSENSCTHFPGNLPNMLRDLRDAFSRVKTFFQMKDQLDNLLLKESLLEDFKGYLGCQALSEMIQFYLEEVMPQAENQDPDIKAHVNSLGENLKTLRLRLRRCHRFLPCENKSKAVEQVKNAFNKLQEKGIYKAMSEFDIFINYIEAYMTMKIRNDAHKSEVAHRFKDLGEENFKALVLIAFAQYLQQCPFEDHVKLVNEVTEFAKTCVADESAENCDKSLHTLFGDKLCTVATLRETYGEMADCCAKQEPERNECFLQHKDDNPNLPRLVRPEVDVMCTAFHDNEETFLKKYLYEIARRHPYFYAPELLFFAKRYKAAFTECCQAADKAACLLPKLDELRDEGKASSAKQRLKCASLQKFGERAFKAWAVARLSQRFPKAEFAEVSKLVTDLTKVHTECCHGDLLECADDRADLAKYICENQDSISSKLKECCEKPLLEKSHCIAEVENDEMPADLPSLAADFVESKDVCKNYAEAKDVFLGMFLYEYARRHPDYSVVLLLRLAKTYETTLEKCCAAADPHECYAKVFDEFKPLVEEPQNLIKQNCELFEQLGEYKFQNALLVRYTKKVPQVSTPTLVEVSRNLGKVGSKCCKHPEAKRMPCAEDYLSVVLNQLCVLHEKTPVSDRVTKCCTESLVNRRPCFSALEVDETYVPKEFNAETFTFHADICTLSEKERQIKKQTALVELVKHKPKATKEQLKAVMDDFAAFVEKCCKADDKETCFAEEGKKLVAASQAALGL

SEQ ID NO: 53 - DNA, 2289 bp, synthetic construct
  source 1..2289: mol_type = other DNA
atgcacagcagcgctctgctgtgttgtctggtgctgctgactggcgtcagagccagccccggccaaggcactcagagcgagaacagctgtactcatttccccggcaacctccctaatatgctgagggatctgagggacgccttctctagggtcaagacattcttccagatgaaggaccaactggacaatctgctgctgaaggaatctctgctggaggactttaagggctatctgggctgccaagccctctccgagatgatccagttttatctggaggaggtcatgcctcaagccgagaaccaagatccagacatcaaggctcacgtcaattctctgggcgaaaatctgaagacactgaggctgaggctcagaaggtgccatagatttctgccatgcgagaacaaaagcaaggctgtggagcaagtgaagaacgccttcaacaagctgcaagagaagggcatctataaggctatgagcgagtttgacatcttcatcaactatatcgaggcttacatgactatgaagattaggaacgacgcccacaagagtgaggttgctcatcggtttaaagatttgggagaagaaaatttcaaagccttggtgttgattgcctttgctcagtatcttcagcagtgtccatttgaagatcatgtaaaattagtgaatgaagtaactgaatttgcaaaaacatgtgttgctgatgagtcagctgaaaattgtgacaaatcacttcataccctttttggagacaaattatgcacagttgcaactcttcgtgaaacctatggtgaaatggctgactgctgtgcaaaacaagaacctgagagaaatgaatgcttcttgcaacacaaagatgacaacccaaacctcccccgattggtgagaccagaggttgatgtgatgtgcactgcttttcatgacaatgaagagacatttttgaaaaaatacttatatgaaattgccagaagacatccttacttttatgccccggaactccttttctttgctaaaaggtataaagctgcttttacagaatgttgccaagctgctgataaagctgcctgcctgttgccaaagctcgatgaacttcgggatgaagggaaggcttcgtctgccaaacagagactcaagtgtgccagtctccaaaaatttggagaaagagctttcaaagcatgggcagtagctcgcctgagccagagatttcccaaagctgagtttgcagaagtttccaagttagtgacagatcttaccaaagtccacacggaatgctgccatggagatctgcttgaatgtgctgatgacagggcggaccttgccaagtatatctgtgaaaatcaagattcgatctccagtaaactgaaggaatgctgtgaaaaacctctgttggaaaaatcccactgcattgccgaagtggaaaatgatgagatgcctgctgacttgccttcattagctgctgattttgttgaaagtaaggatgtttgcaaaaactatgctgaggcaaaggatgtcttcctgggcatgtttttgtatgaatatgcaagaaggcatcctgattactctgtcgtgctgctgctgagacttgccaagacatatgaaaccactctagagaagtgctgtgccgctgcagatcctcatgaatgctatgccaaagtgttcgatgaatttaaacctcttgtggaagagcctcagaatttaatcaaacaaaattgtgagctttttgagcagcttggagagtacaaattccagaatgcgctattagttcgttacaccaagaaagtaccccaagtgtcaactccaactcttgtagaggtctcaagaaacctaggaaaagtgggcagcaaatgttgtaaacatcctgaagcaaaaagaatgccctgtgcagaagactatctatccgtggtcctgaaccagttatgtgtgttgcatgagaaaacgccagtaagtgacagagtcaccaaatgctgcacagaatccttggtgaacaggcgaccatgcttttcagctctggaagtcgatgaaacatacgttcccaaagagtttaatgctgaaacattcaccttccatgcagatatatgcacactttctgagaaggagagacaaatcaagaaacaaactgcacttgttgagctcgtgaaacacaagcccaaggcaacaaaagagcaactgaaagctgttatggatgatttcgcagcttttgtagagaagtgctgcaaggctgacgataaggagacctgctttgccgaggagggtaaaaaacttgttgctgcaagtcaagctgccttaggctta

SEQ ID NO: 54 - protein, 750 aa, synthetic construct
DAHKSEVAHRFKDLGEENFKALVLIAFAQYLQQCPFEDHVKLVNEVTEFAKTCVADESAENCDKSLHTLFGDKLCTVATLRETYGEMADCCAKQEPERNECFLQHKDDNPNLPRLVRPEVDVMCTAFHDNEETFLKKYLYEIARRHPYFYAPELLFFAKRYKAAFTECCQAADKAACLLPKLDELRDEGKASSAKQRLKCASLQKFGERAFKAWAVARLSQRFPKAEFAEVSKLVTDLTKVHTECCHGDLLECADDRADLAKYICENQDSISSKLKECCEKPLLEKSHCIAEVENDEMPADLPSLAADFVESKDVCKNYAEAKDVFLGMFLYEYARRHPDYSVVLLLRLAKTYETTLEKCCAAADPHECYAKVFDEFKPLVEEPQNLIKQNCELFEQLGEYKFQNALLVRYTKKVPQVSTPTLVEVSRNLGKVGSKCCKHPEAKRMPCAEDYLSVVLNQLCVLHEKTPVSDRVTKCCTESLVNRRPCFSALEVDETYVPKEFNAETFTFHADICTLSEKERQIKKQTALVELVKHKPKATKEQLKAVMDDFAAFVEKCCKADDKETCFAEEGKKLVAASQAALGLGGGGSSPGQGTQSENSCTHFPGNLPNMLRDLRDAFSRVKTFFQMKDQLDNLLLKESLLEDFKGYLGCQALSEMIQFYLEEVMPQAENQDPDIKAHVNSLGENLKTLRLRLRRCHRFLPCENKSKAVEQVKNAFNKLQEKGIYKAMSEFDIFINYIEAYMTMKIRN

SEQ ID NO: 55 - protein, 750 aa, synthetic construct
SPGQGTQSENSCTHFPGNLPNMLRDLRDAFSRVKTFFQMKDQLDNLLLKESLLEDFKGYLGCQALSEMIQFYLEEVMPQAENQDPDIKAHVNSLGENLKTLRLRLRRCHRFLPCENKSKAVEQVKNAFNKLQEKGIYKAMSEFDIFINYIEAYMTMKIRNGGGGSDAHKSEVAHRFKDLGEENFKALVLIAFAQYLQQCPFEDHVKLVNEVTEFAKTCVADESAENCDKSLHTLFGDKLCTVATLRETYGEMADCCAKQEPERNECFLQHKDDNPNLPRLVRPEVDVMCTAFHDNEETFLKKYLYEIARRHPYFYAPELLFFAKRYKAAFTECCQAADKAACLLPKLDELRDEGKASSAKQRLKCASLQKFGERAFKAWAVARLSQRFPKAEFAEVSKLVTDLTKVHTECCHGDLLECADDRADLAKYICENQDSISSKLKECCEKPLLEKSHCIAEVENDEMPADLPSLAADFVESKDVCKNYAEAKDVFLGMFLYEYARRHPDYSVVLLLRLAKTYETTLEKCCAAADPHECYAKVFDEFKPLVEEPQNLIKQNCELFEQLGEYKFQNALLVRYTKKVPQVSTPTLVEVSRNLGKVGSKCCKHPEAKRMPCAEDYLSVVLNQLCVLHEKTPVSDRVTKCCTESLVNRRPCFSALEVDETYVPKEFNAETFTFHADICTLSEKERQIKKQTALVELVKHKPKATKEQLKAVMDDFAAFVEKCCKADDKETCFAEEGKKLVAASQAALGL

SEQ ID NO: 56 - protein, 745 aa, synthetic construct
DAHKSEVAHRFKDLGEENFKALVLIAFAQYLQQCPFEDHVKLVNEVTEFAKTCVADESAENCDKSLHTLFGDKLCTVATLRETYGEMADCCAKQEPERNECFLQHKDDNPNLPRLVRPEVDVMCTAFHDNEETFLKKYLYEIARRHPYFYAPELLFFAKRYKAAFTECCQAADKAACLLPKLDELRDEGKASSAKQRLKCASLQKFGERAFKAWAVARLSQRFPKAEFAEVSKLVTDLTKVHTECCHGDLLECADDRADLAKYICENQDSISSKLKECCEKPLLEKSHCIAEVENDEMPADLPSLAADFVESKDVCKNYTEAKDVFLGMFLYEYARRHPDYSVVLLLRLAKTYETTLEKCCAAADPHECYAKVFDEFKPLVEEPQNLIKQNCELFEQLGEYKFQNALLVRYTKKVPQVSTPTLVEVSRNLGKVGSKCCKHPEAKRMPCAEDYLSVVLNQLCVLHEKTPVSDRVTKCCTESLVNRRPCFSALEVDETYVPKEFNAETFTFHADICTLSEKERQIKKQTALVELVKHKPKATKEQLKAVMDDFAAFVEKCCKADDKETCFAEEGKKLVAASQAALGLSPGQGTQSENSCTHFPGNLPNMLRDLRDAFSRVKTFFQMKDQLDNLLLKESLLEDFKGYLGCQALSEMIQFYLEEVMPQAENQDPDIKAHVNSLGENLKTLRLRLRRCHRFLPCENKSKAVEQVKNAFNKLQEKGIYKAMSEFDIFINYIEAYMTMKIRN

SEQ ID NO: 57 - protein, 745 aa, synthetic construct
SPGQGTQSENSCTHFPGNLPNMLRDLRDAFSRVKTFFQMKDQLDNLLLKESLLEDFKGYLGCQALSEMIQFYLEEVMPQAENQDPDIKAHVNSLGENLKTLRLRLRRCHRFLPCENKSKAVEQVKNAFNKLQEKGIYKAMSEFDIFINYIEAYMTMKIRNDAHKSEVAHRFKDLGEENFKALVLIAFAQYLQQCPFEDHVKLVNEVTEFAKTCVADESAENCDKSLHTLFGDKLCTVATLRETYGEMADCCAKQEPERNECFLQHKDDNPNLPRLVRPEVDVMCTAFHDNEETFLKKYLYEIARRHPYFYAPELLFFAKRYKAAFTECCQAADKAACLLPKLDELRDEGKASSAKQRLKCASLQKFGERAFKAWAVARLSQRFPKAEFAEVSKLVTDLTKVHTECCHGDLLECADDRADLAKYICENQDSISSKLKECCEKPLLEKSHCIAEVENDEMPADLPSLAADFVESKDVCKNYTEAKDVFLGMFLYEYARRHPDYSVVLLLRLAKTYETTLEKCCAAADPHECYAKVFDEFKPLVEEPQNLIKQNCELFEQLGEYKFQNALLVRYTKKVPQVSTPTLVEVSRNLGKVGSKCCKHPEAKRMPCAEDYLSVVLNQLCVLHEKTPVSDRVTKCCTESLVNRRPCFSALEVDETYVPKEFNAETFTFHADICTLSEKERQIKKQTALVELVKHKPKATKEQLKAVMDDFAAFVEKCCKADDKETCFAEEGKKLVAASQAALGL

SEQ ID NO: 58 - protein, 750 aa, synthetic construct
DAHKSEVAHRFKDLGEENFKALVLIAFAQYLQQCPFEDHVKLVNEVTEFAKTCVADESAENCDKSLHTLFGDKLCTVATLRETYGEMADCCAKQEPERNECFLQHKDDNPNLPRLVRPEVDVMCTAFHDNEETFLKKYLYEIARRHPYFYAPELLFFAKRYKAAFTECCQAADKAACLLPKLDELRDEGKASSAKQRLKCASLQKFGERAFKAWAVARLSQRFPKAEFAEVSKLVTDLTKVHTECCHGDLLECADDRADLAKYICENQDSISSKLKECCEKPLLEKSHCIAEVENDEMPADLPSLAADFVESKDVCKNYTEAKDVFLGMFLYEYARRHPDYSVVLLLRLAKTYETTLEKCCAAADPHECYAKVFDEFKPLVEEPQNLIKQNCELFEQLGEYKFQNALLVRYTKKVPQVSTPTLVEVSRNLGKVGSKCCKHPEAKRMPCAEDYLSVVLNQLCVLHEKTPVSDRVTKCCTESLVNRRPCFSALEVDETYVPKEFNAETFTFHADICTLSEKERQIKKQTALVELVKHKPKATKEQLKAVMDDFAAFVEKCCKADDKETCFAEEGKKLVAASQAALGLGGGGSSPGQGTQSENSCTHFPGNLPNMLRDLRDAFSRVKTFFQMKDQLDNLLLKESLLEDFKGYLGCQALSEMIQFYLEEVMPQAENQDPDIKAHVNSLGENLKTLRLRLRRCHRFLPCENKSKAVEQVKNAFNKLQEKGIYKAMSEFDIFINYIEAYMTMKIRN

SEQ ID NO: 59 - protein, 750 aa, synthetic construct
SPGQGTQSENSCTHFPGNLPNMLRDLRDAFSRVKTFFQMKDQLDNLLLKESLLEDFKGYLGCQALSEMIQFYLEEVMPQAENQDPDIKAHVNSLGENLKTLRLRLRRCHRFLPCENKSKAVEQVKNAFNKLQEKGIYKAMSEFDIFINYIEAYMTMKIRNGGGGSDAHKSEVAHRFKDLGEENFKALVLIAFAQYLQQCPFEDHVKLVNEVTEFAKTCVADESAENCDKSLHTLFGDKLCTVATLRETYGEMADCCAKQEPERNECFLQHKDDNPNLPRLVRPEVDVMCTAFHDNEETFLKKYLYEIARRHPYFYAPELLFFAKRYKAAFTECCQAADKAACLLPKLDELRDEGKASSAKQRLKCASLQKFGERAFKAWAVARLSQRFPKAEFAEVSKLVTDLTKVHTECCHGDLLECADDRADLAKYICENQDSISSKLKECCEKPLLEKSHCIAEVENDEMPADLPSLAADFVESKDVCKNYTEAKDVFLGMFLYEYARRHPDYSVVLLLRLAKTYETTLEKCCAAADPHECYAKVFDEFKPLVEEPQNLIKQNCELFEQLGEYKFQNALLVRYTKKVPQVSTPTLVEVSRNLGKVGSKCCKHPEAKRMPCAEDYLSVVLNQLCVLHEKTPVSDRVTKCCTESLVNRRPCFSALEVDETYVPKEFNAETFTFHADICTLSEKERQIKKQTALVELVKHKPKATKEQLKAVMDDFAAFVEKCCKADDKETCFAEEGKKLVAASQAALGL

SEQ ID NO: 60 - protein, 119 aa, Homo sapiens
HSDPARRGELSVCDSISEWVTAADKKTAVDMSGGTVTVLEKVPVSKGQLKQYFYETKCNPMGYTKEGCRGIDKRHWNSQCRTTQSYVRALTMDSKKRIGWRFIRIDTSCVCTLTIKRGR

SEQ ID NO: 61 - DNA, 741 bp, synthetic construct
  source 1..741: mol_type = other DNA
atgacaattctgttcctcacaatggtgatcagctacttcggctgcatgaaggccgcccctatgaaggaggctaacatcagaggacaaggcggactcgcctatcccggcgtgaggactcacggcactctggaaagcgtgaatggccctaaggccggaagcagaggactcacatctctggctgacacattcgagcacgtgatcgaagagctgctggatgaggatcagaaggtgaggcctaacgaggagaacaacaaggacgccgatctgtacacatctagggtcatgctgtccagccaagtgccactggagcctcctctcctctttctgctggaggagtacaagaactatctggacgccgccaacatgtccatgagagtgagaaggcacagcgacccagccagaagaggcgagctgagcgtctgcgatagcatctccgaatgggtgactgctgccgataagaagacagccgtcgatatgagcggcggcacagtgacagtgctggaaaaagtcccagtcagcaagggccagctgaagcagtacttctacgagactaagtgcaaccctatgggctacacaaaggaaggctgtaggggcatcgacaaaaggcactggaactcccagtgtaggactactcagagctatgtgagggccctcactatggacagcaagaagaggatcggctggaggtttattaggattgacacaagctgcgtgtgcacactgacaatcaagaggggcaga

SEQ ID NO: 62 - protein, 120 aa, Homo sapiens
SSSHPIFHRGEFSVCDSVSVWVGDKTTATDIKGKEVMVLGEVNINNSVFKQYFFETKCRDPNPVDSGCRGIDSKHWNSYCTTTHTFVKALTMDGKQAAWRFIRIDTACVCVLSRKAVRRA

SEQ ID NO: 63 - DNA, 723 bp, synthetic construct
  source 1..723: mol_type = other DNA
atgagcatgctgttctacacactgatcactgcctttctgatcggcatccaagccgagcctcatagcgagagcaatgtgccagccggccacacaatcccacaagcccactggactaagctgcaacatagcctcgacacagctctgaggagagctaggtccgctccagccgctgctatcgctgctagagtggccggccagacaagaaacatcactgtggaccctaggctcttcaagaagagaaggctgaggtccccaagagtgctcttcagcacacagcctccaagggaggccgctgatacacaagatttggacttcgaggtgggaggcgctgcccctttcaataggactcataggtccaagaggagcagctcccacccaattttccacagaggcgagttcagcgtgtgcgattccgtgtccgtctgggtgggcgacaaaactactgccactgacatcaagggcaaagaggtgatggtgctcggcgaggtgaacattaacaacagcgtgttcaagcagtatttcttcgagacaaagtgtagggacccaaacccagtggatagcggctgtaggggcatcgactccaagcactggaacagctactgcacaactactcacactttcgtcaaggctctgacaatggatggcaagcaagccgcttggaggttcatcagaatcgacacagcttgtgtgtgcgtgctgtctaggaaggccgtgaggagggct

SEQ ID NO: 64 - protein, 119 aa, Homo sapiens [sequence omitted]

SEQ ID NO: 65 - DNA, 771 bp, synthetic construct
  source 1..771: mol_type = other DNA
atgtccattctgttctacgtcatctttctggcctatctgaggggcatccaaggcaataacatggaccagaggtctctgccagaggactctctgaactctctgatcatcaagctgatccaagccgatattctgaagaacaagctgagcaaacagatggtggacgtcaaggagaactaccagagcacactcccaaaggctgaggcccctagggaaccagaaagaggcggcccagccaaaagcgccttccagccagtgattgctatggacactgagctcctcagacagcagagaaggtacaactccccaagggtgctgctgagcgacagcactcctctggagcctccaccactgtacctcatggaggattacgtgggcagcccagtggtggccaataggacttctaggaggaagaggtacgctgaacacaagagccataggggagagtacagcgtctgcgattccgagagcctctgggtgactgacaagtcctccgctatcgatattaggggccaccaagtgacagtgctcggcgaaatcaagactggcaactccccagtgaagcagtacttctacgagacaaggtgcaaggaggctaggccagtgaagaacggctgtaggggaattgacgacaagcactggaacagccagtgcaagactagccagacatatgtgagggccctcactagcgagaacaacaagctcgtgggctggagatggattaggatcgacacaagctgtgtctgcgctctgtctaggaagatcggaaggact

SEQ ID NO: 66 - protein, 130 aa, Homo sapiens
GVSETAPASRRGELAVCDAVSGWVTDRRTAVDLRGREVEVLGEVPAAGGSPLRQYFFETRCKADNAEEGGPGAGGGGCRGVDRRHWVSECKAKQSYVRALTADAQGRVGWRWIRIDTACVCTLLSRTGRA

SEQ ID NO: 67 - DNA, 630 bp, synthetic construct
  source 1..630: mol_type = other DNA
atgctgccactgccaagctgttctctgcctattctgctgctgtttctgctcccaagcgtgcctatcgagtcccagcctccaccttccacactgcctccatttctggccccagagtgggatctgctgagcccaagggtggtgctcagcagaggcgctccagccggacctccactgctgtttctgctggaagctggcgcctttagagaaagcgccggagctccagccaataggtctaggaggggcgtgtccgagactgctccagccagcagaagaggcgaactggctgtgtgcgatgccgtgagcggctgggtcacagataggaggactgccgtggatctgagaggaagggaggtggaggtgctgggagaagtgccagctgccggaggcagccctctgaggcagtacttcttcgagacaaggtgcaaggccgacaatgccgaagaaggaggccccggcgctggaggcggaggatgtagaggcgtggataggagacattgggtgagcgagtgtaaggccaagcagagctatgtgagagctctgactgctgatgctcaaggcagagtgggatggaggtggatcagaatcgacactgcttgtgtctgcacactgctgtctaggactggcagagct

SEQ ID NO: 68 - protein, 706 aa, synthetic construct
DAHKSEVAHRFKDLGEENFKALVLIAFAQYLQQCPFEDHVKLVNEVTEFAKTCVADESAENCDKSLHTLFGDKLCTVATLRETYGEMADCCAKQEPERNECFLQHKDDNPNLPRLVRPEVDVMCTAFHDNEETFLKKYLYEIARRHPYFYAPELLFFAKRYKAAFTECCQAADKAACLLPKLDELRDEGKASSAKQGLKCASLQKFGERAFKAWAVARLSQRFPKAEFAEVSKLVTDLTKVHTECCHGDLLECADDRADLAKYICENQDSISSKLKECCEKPLLEKSHCIAEVENDEMPADLPSLAADFVGSKDVCKNYAEAKDVFLGMFLYEYARRHPDYSVVLLLRLAKTYETTLEKCCAAADPHECYAKVFDEFKPLVEEPQNLIKQNCELFEQLGEYKFQNALLVRYTKKVPQVSTPTLVEVSRNLGKVGSKCCKHPEAKRMPCAEDCLSVFLNQLCVLHEKTPVSDRVTKCCTESLVNGRPCFSALEVDETYVPKEFNAETFTFHADICTLSEKERQIKKQTALVELVKHKPKATKEQLKAVMDDFAAFVEKCCKADDKETCFAEEGKKLVAASQAALGLGSHSDPARRGELSVCDSISEWVTAADKKTAVDMSGGTVTVLEKVPVSKGQLKQYFYETKCNPMGYTKEGCRGIDKRHWNSQCRTTQSYVRALTMDSKKRIGWRFIRIDTSCVCTLTIKRGR

SEQ ID NO: 69 - DNA, 2190 bp, synthetic construct
  source 1..2190: mol_type = other DNA
atgaagtgggtgactttcatctctctgctgttcctcttcagcagcgcctacagcagaggcgtgttcagaagggatgcccacaagagcgaggtcgcccatagattcaaggatctgggcgaggagaacttcaaggctctcgtgctcatcgctttcgcccagtatctgcagcagtgccctttcgaagaccatgtgaagctggtgaacgaggtgacagagttcgccaagacatgtgtggccgatgagagcgccgagaactgcgacaagtctctgcacacactgttcggagataagctgtgcacagtcgctactctgagggagacttacggcgaaatggccgactgttgtgccaagcaagagccagagaggaatgagtgcttcctccagcacaaggacgacaaccctaatctgcctagactcgtgaggccagaagtggatgtgatgtgcacagctttccacgacaacgaggagactttcctcaagaagtacctctacgagatcgctaggagacacccttacttctatgccccagagctgctcttcttcgccaagaggtataaagccgctttcacagagtgctgtcaagccgccgacaaagctgcttgtctgctgcctaagctggatgagctgagggatgagggcaaggcctctagcgccaaacaaggcctcaaatgcgcttccctccagaagttcggagagagggcctttaaggcttgggccgtcgctaggctcagccaaagattcccaaaggccgagttcgctgaggtgagcaagctggtcacagacctcactaaggtgcacactgagtgctgtcacggagatctgctcgaatgtgccgacgacagagctgacctcgccaaatacatctgcgagaatcaagattccatcagctccaagctcaaggagtgctgtgagaagccactgctcgagaagagccattgcatcgccgaggtcgagaacgatgagatgccagccgatctgccttctctggctgccgatttcgtgggctccaaagacgtctgcaagaactacgccgaggctaaggacgtctttctgggcatgtttctgtacgagtatgctaggagacatccagattactccgtggtgctgctgctgagactggccaagacttacgagacaacactggaaaagtgctgcgccgctgctgacccacacgagtgctacgccaaggtgtttgacgagttcaagcctctcgtcgaggagccacagaatctgattaagcagaactgtgaactcttcgagcagctgggcgagtacaagttccaaaatgctctgctggtgaggtacactaagaaggtgcctcaagtgtccactcctacactggtggaggtgagcagaaatctcggcaaggtcggcagcaaatgttgcaagcacccagaggccaagagaatgccttgtgctgaggactgtctgagcgtgtttctgaaccagctctgtgtgctgcacgagaagacaccagtcagcgacagagtgactaagtgctgcacagagtctctggtgaacggaaggccatgtttctccgctctggaggtcgacgagacttacgtgcctaaggagttcaacgccgagactttcacattccacgccgacatctgcactctctccgaaaaggaaaggcagatcaagaagcagacagctctggtggagctggtcaagcacaagccaaaggccacaaaggaacagctcaaggctgtcatggacgacttcgccgccttcgtcgagaagtgttgcaaagccgacgacaaggagacatgcttcgccgaggagggcaaaaaactggtcgctgccagccaagccgctctcggcctcggatctcacagcgacccagccagaagaggcgagctgagcgtctgcgatagcatctccgaatgggtgactgctgccgataagaagacagccgtcgatatgagcggcggcacagtgacagtgctggaaaaagtcccagtcagcaagggccagctgaagcagtacttctacgagactaagtgcaaccctatgggctacacaaaggaaggctgtaggggcatcgacaaaaggcactggaactcccagtgtaggactactcagagctatgtgagggccctcactatggacagcaagaagaggatcggctggaggtttattaggattgacacaagctgcgtgtgcacactgacaatcaagaggggcaga

SEQ ID NO: 70 - protein, 707 aa, synthetic construct
DAHKSEVAHRFKDLGEENFKALVLIAFAQYLQQCPFEDHVKLVNEVTEFAKTCVADESAENCDKSLHTLFGDKLCTVATLRETYGEMADCCAKQEPERNECFLQHKDDNPNLPRLVRPEVDVMCTAFHDNEETFLKKYLYEIARRHPYFYAPELLFFAKRYKAAFTECCQAADKAACLLPKLDELRDEGKASSAKQGLKCASLQKFGERAFKAWAVARLSQRFPKAEFAEVSKLVTDLTKVHTECCHGDLLECADDRADLAKYICENQDSISSKLKECCEKPLLEKSHCIAEVENDEMPADLPSLAADFVGSKDVCKNYAEAKDVFLGMFLYEYARRHPDYSVVLLLRLAKTYETTLEKCCAAADPHECYAKVFDEFKPLVEEPQNLIKQNCELFEQLGEYKFQNALLVRYTKKVPQVSTPTLVEVSRNLGKVGSKCCKHPEAKRMPCAEDCLSVFLNQLCVLHEKTPVSDRVTKCCTESLVNGRPCFSALEVDETYVPKEFNAETFTFHADICTLSEKERQIKKQTALVELVKHKPKATKEQLKAVMDDFAAFVEKCCKADDKETCFAEEGKKLVAASQAALGLGSSSSHPIFHRGEFSVCDSVSVWVGDKTTATDIKGKEVMVLGEVNINNSVFKQYFFETKCRDPNPVDSGCRGIDSKHWNSYCTTTHTFVKALTMDGKQAAWRFIRIDTACVCVLSRKAVRRA

SEQ ID NO: 71 - DNA, 2193 bp, synthetic construct
  source 1..2193: mol_type = other DNA
atgaagtgggtgactttcatctctctgctgttcctcttcagcagcgcctacagcagaggcgtgttcagaagggatgcccacaagagcgaggtcgcccatagattcaaggatctgggcgaggagaacttcaaggctctcgtgctcatcgctttcgcccagtatctgcagcagtgccctttcgaagaccatgtgaagctggtgaacgaggtgacagagttcgccaagacatgtgtggccgatgagagcgccgagaactgcgacaagtctctgcacacactgttcggagataagctgtgcacagtcgctactctgagggagacttacggcgaaatggccgactgttgtgccaagcaagagccagagaggaatgagtgcttcctccagcacaaggacgacaaccctaatctgcctagactcgtgaggccagaagtggatgtgatgtgcacagctttccacgacaacgaggagactttcctcaagaagtacctctacgagatcgctaggagacacccttacttctatgccccagagctgctcttcttcgccaagaggtataaagccgctttcacagagtgctgtcaagccgccgacaaagctgcttgtctgctgcctaagctggatgagctgagggatgagggcaaggcctctagcgccaaacaaggcctcaaatgcgcttccctccagaagttcggagagagggcctttaaggcttgggccgtcgctaggctcagccaaagattcccaaaggccgagttcgctgaggtgagcaagctggtcacagacctcactaaggtgcacactgagtgctgtcacggagatctgctcgaatgtgccgacgacagagctgacctcgccaaatacatctgcgagaatcaagattccatcagctccaagctcaaggagtgctgtgagaagccactgctcgagaagagccattgcatcgccgaggtcgagaacgatgagatgccagccgatctgccttctctggctgccgatttcgtgggctccaaagacgtctgcaagaactacgccgaggctaaggacgtctttctgggcatgtttctgtacgagtatgctaggagacatccagattactccgtggtgctgctgctgagactggccaagacttacgagacaacactggaaaagtgctgcgccgctgctgacccacacgagtgctacgccaaggtgtttgacgagttcaagcctctcgtcgaggagccacagaatctgattaagcagaactgtgaactcttcgagcagctgggcgagtacaagttccaaaatgctctgctggtgaggtacactaagaaggtgcctcaagtgtccactcctacactggtggaggtgagcagaaatctcggcaaggtcggcagcaaatgttgcaagcacccagaggccaagagaatgccttgtgctgaggactgtctgagcgtgtttctgaaccagctctgtgtgctgcacgagaagacaccagtcagcgacagagtgactaagtgctgcacagagtctctggtgaacggaaggccatgtttctccgctctggaggtcgacgagacttacgtgcctaaggagttcaacgccgagactttcacattccacgccgacatctgcactctctccgaaaaggaaaggcagatcaagaagcagacagctctggtggagctggtcaagcacaagccaaaggccacaaaggaacagctcaaggctgtcatggacgacttcgccgccttcgtcgagaagtgttgcaaagccgacgacaaggagacatgcttcgccgaggagggcaaaaaactggtcgctgccagccaagccgctctcggcctcggatctagcagctcccacccaattttccacagaggcgagttcagcgtgtgcgattccgtgtccgtctgggtgggcgacaaaactactgccactgacatcaagggcaaagaggtgatggtgctcggcgaggtgaacattaacaacagcgtgttcaagcagtatttcttcgagacaaagtgtagggacccaaacccagtggatagcggctgtaggggcatcgactccaagcactggaacagctactgcacaactactcacactttcgtcaaggctctgacaatggatggcaagcaagccgcttggaggttcatcagaatcgacacagcttgtgtgtgcgtgctgtctaggaaggccgtgaggagggct

SEQ ID NO: 72 - protein, 706 aa, synthetic construct
DAHKSEVAHRFKDLGEENFKALVLIAFAQYLQQCPFEDHVKLVNEVTEFAKTCVADESAENCDKSLHTLFGDKLCTVATLRETYGEMADCCAKQEPERNECFLQHKDDNPNLPRLVRPEVDVMCTAFHDNEETFLKKYLYEIARRHPYFYAPELLFFAKRYKAAFTECCQAADKAACLLPKLDELRDEGKASSAKQGLKCASLQKFGERAFKAWAVARLSQRFPKAEFAEVSKLVTDLTKVHTECCHGDLLECADDRADLAKYICENQDSISSKLKECCEKPLLEKSHCIAEVENDEMPADLPSLAADFVGSKDVCKNYAEAKDVFLGMFLYEYARRHPDYSVVLLLRLAKTYETTLEKCCAAADPHECYAKVFDEFKPLVEEPQNLIKQNCELFEQLGEYKFQNALLVRYTKKVPQVSTPTLVEVSRNLGKVGSKCCKHPEAKRMPCAEDCLSVFLNQLCVLHEKTPVSDRVTKCCTESLVNGRPCFSALEVDETYVPKEFNAETFTFHADICTLSEKERQIKKQTALVELVKHKPKATKEQLKAVMDDFAAFVEKCCKADDKETCFAEEGKKLVAASQAALGLGSYAEHKSHRGEYSVCDSESLWVTDKSSAIDIRGHQVTVLGEIKTGNSPVKQYFYETRCKEARPVKNGCRGIDDKHWNSQCKTSQTYVRALTSENNKLVGWRWIRIDTSCVCALSRKIGRT

SEQ ID NO: 73 - DNA, 2190 bp, synthetic construct
  source 1..2190: mol_type = other DNA
atgaagtgggtgactttcatctctctgctgttcctcttcagcagcgcctacagcagaggcgtgttcagaagggatgcccacaagagcgaggtcgcccatagattcaaggatctgggcgaggagaacttcaaggctctcgtgctcatcgctttcgcccagtatctgcagcagtgccctttcgaagaccatgtgaagctggtgaacgaggtgacagagttcgccaagacatgtgtggccgatgagagcgccgagaactgcgacaagtctctgcacacactgttcggagataagctgtgcacagtcgctactctgagggagacttacggcgaaatggccgactgttgtgccaagcaagagccagagaggaatgagtgcttcctccagcacaaggacgacaaccctaatctgcctagactcgtgaggccagaagtggatgtgatgtgcacagctttccacgacaacgaggagactttcctcaagaagtacctctacgagatcgctaggagacacccttacttctatgccccagagctgctcttcttcgccaagaggtataaagccgctttcacagagtgctgtcaagccgccgacaaagctgcttgtctgctgcctaagctggatgagctgagggatgagggcaaggcctctagcgccaaacaaggcctcaaatgcgcttccctccagaagttcggagagagggcctttaaggcttgggccgtcgctaggctcagccaaagattcccaaaggccgagttcgctgaggtgagcaagctggtcacagacctcactaaggtgcacactgagtgctgtcacggagatctgctcgaatgtgccgacgacagagctgacctcgccaaatacatctgcgagaatcaagattccatcagctccaagctcaaggagtgctgtgagaagccactgctcgagaagagccattgcatcgccgaggtcgagaacgatgagatgccagccgatctgccttctctggctgccgatttcgtgggctccaaagacgtctgcaagaactacgccgaggctaaggacgtctttctgggcatgtttctgtacgagtatgctaggagacatccagattactccgtggtgctgctgctgagactggccaagacttacgagacaacactggaaaagtgctgcgccgctgctgacccacacgagtgctacgccaaggtgtttgacgagttcaagcctctcgtcgaggagccacagaatctgattaagcagaactgtgaactcttcgagcagctgggcgagtacaagttccaaaatgctctgctggtgaggtacactaagaaggtgcctcaagtgtccactcctacactggtggaggtgagcagaaatctcggcaaggtcggcagcaaatgttgcaagcacccagaggccaagagaatgccttgtgctgaggactgtctgagcgtgtttctgaaccagctctgtgtgctgcacgagaagacaccagtcagcgacagagtgactaagtgctgcacagagtctctggtgaacggaaggccatgtttctccgctctggaggtcgacgagacttacgtgcctaaggagttcaacgccgagactttcacattccacgccgacatctgcactctctccgaaaaggaaaggcagatcaagaagcagacagctctggtggagctggtcaagcacaagccaaaggccacaaaggaacagctcaaggctgtcatggacgacttcgccgccttcgtcgagaagtgttgcaaagccgacgacaaggagacatgcttcgccgaggagggcaaaaaactggtcgctgccagccaagccgctctcggcctcggatcttacgctgaacacaagagccataggggagagtacagcgtctgcgattccgagagcctctgggtgactgacaagtcctccgctatcgatattaggggccaccaagtgacagtgctcggcgaaatcaagactggcaactccccagtgaagcagtacttctacgagacaaggtgcaaggaggctaggccagtgaagaacggctgtaggggaattgacgacaagcactggaacagccagtgcaagactagccagacatatgtgagggccctcactagcgagaacaacaagctcgtgggctggagatggattaggatcgacacaagctgtgtctgcgctctgtctaggaagatcggaaggact

SEQ ID NO: 74 - protein, 717 aa, synthetic construct
DAHKSEVAHRFKDLGEENFKALVLIAFAQYLQQCPFEDHVKLVNEVTEFAKTCVADESAENCDKSLHTLFGDKLCTVATLRETYGEMADCCAKQEPERNECFLQHKDDNPNLPRLVRPEVDVMCTAFHDNEETFLKKYLYEIARRHPYFYAPELLFFAKRYKAAFTECCQAADKAACLLPKLDELRDEGKASSAKQGLKCASLQKFGERAFKAWAVARLSQRFPKAEFAEVSKLVTDLTKVHTECCHGDLLECADDRADLAKYICENQDSISSKLKECCEKPLLEKSHCIAEVENDEMPADLPSLAADFVGSKDVCKNYAEAKDVFLGMFLYEYARRHPDYSVVLLLRLAKTYETTLEKCCAAADPHECYAKVFDEFKPLVEEPQNLIKQNCELFEQLGEYKFQNALLVRYTKKVPQVSTPTLVEVSRNLGKVGSKCCKHPEAKRMPCAEDCLSVFLNQLCVLHEKTPVSDRVTKCCTESLVNGRPCFSALEVDETYVPKEFNAETFTFHADICTLSEKERQIKKQTALVELVKHKPKATKEQLKAVMDDFAAFVEKCCKADDKETCFAEEGKKLVAASQAALGLGSGVSETAPASRRGELAVCDAVSGWVTDRRTAVDLRGREVEVLGEVPAAGGSPLRQYFFETRCKADNAEEGGPGAGGGGCRGVDRRHWVSECKAKQSYVRALTADAQGRVGWRWIRIDTACVCTLLSRTGRA

SEQ ID NO: 75 - DNA, 2223 bp, synthetic construct
  source 1..2223: mol_type = other DNA
atgaagtgggtgactttcatctctctgctgttcctcttcagcagcgcctacagcagaggcgtgttcagaagggatgcccacaagagcgaggtcgcccatagattcaaggatctgggcgaggagaacttcaaggctctcgtgctcatcgctttcgcccagtatctgcagcagtgccctttcgaagaccatgtgaagctggtgaacgaggtgacagagttcgccaagacatgtgtggccgatgagagcgccgagaactgcgacaagtctctgcacacactgttcggagataagctgtgcacagtcgctactctgagggagacttacggcgaaatggccgactgttgtgccaagcaagagccagagaggaatgagtgcttcctccagcacaaggacgacaaccctaatctgcctagactcgtgaggccagaagtggatgtgatgtgcacagctttccacgacaacgaggagactttcctcaagaagtacctctacgagatcgctaggagacacccttacttctatgccccagagctgctcttcttcgccaagaggtataaagccgctttcacagagtgctgtcaagccgccgacaaagctgcttgtctgctgcctaagctggatgagctgagggatgagggcaaggcctctagcgccaaacaaggcctcaaatgcgcttccctccagaagttcggagagagggcctttaaggcttgggccgtcgctaggctcagccaaagattcccaaaggccgagttcgctgaggtgagcaagctggtcacagacctcactaaggtgcacactgagtgctgtcacggagatctgctcgaatgtgccgacgacagagctgacctcgccaaatacatctgcgagaatcaagattccatcagctccaagctcaaggagtgctgtgagaagccactgctcgagaagagccattgcatcgccgaggtcgagaacgatgagatgccagccgatctgccttctctggctgccgatttcgtgggctccaaagacgtctgcaagaactacgccgaggctaaggacgtctttctgggcatgtttctgtacgagtatgctaggagacatccagattactccgtggtgctgctgctgagactggccaagacttacgagacaacactggaaaagtgctgcgccgctgctgacccacacgagtgctacgccaaggtgtttgacgagttcaagcctctcgtcgaggagccacagaatctgattaagcagaactgtgaactcttcgagcagctgggcgagtacaagttccaaaatgctctgctggtgaggtacactaagaaggtgcctcaagtgtccactcctacactggtggaggtgagcagaaatctcggcaaggtcggcagcaaatgttgcaagcacccagaggccaagagaatgccttgtgctgaggactgtctgagcgtgtttctgaaccagctctgtgtgctgcacgagaagacaccagtcagcgacagagtgactaagtgctgcacagagtctctggtgaacggaaggccatgtttctccgctctggaggtcgacgagacttacgtgcctaaggagttcaacgccgagactttcacattccacgccgacatctgcactctctccgaaaaggaaaggcagatcaagaagcagacagctctggtggagctggtcaagcacaagccaaaggccacaaaggaacagctcaaggctgtcatggacgacttcgccgccttcgtcgagaagtgttgcaaagccgacgacaaggagacatgcttcgccgaggagggcaaaaaactggtcgctgccagccaagccgctctcggcctcggatctggcgtgtccgagactgctccagccagcagaagaggcgaactggctgtgtgcgatgccgtgagcggctgggtcacagataggaggactgccgtggatctgagaggaagggaggtggaggtgctgggagaagtgccagctgccggaggcagccctctgaggcagtacttcttcgagacaaggtgcaaggccgacaatgccgaagaaggaggccccggcgctggaggcggaggatgtagaggcgtggataggagacattgggtgagcgagtgtaaggccaagcagagctatgtgagagctctgactgctgatgctcaaggcagagtgggatggaggtggatcagaatcgacactgcttgtgtctgcacactgctgtctaggactggcagagct

SEQ ID NO: 76 - protein, 706 aa, synthetic construct
HSDPARRGELSVCDSISEWVTAADKKTAVDMSGGTVTVLEKVPVSKGQLKQYFYETKCNPMGYTKEGCRGIDKRHWNSQCRTTQSYVRALTMDSKKRIGWRFIRIDTSCVCTLTIKRGRGSDAHKSEVAHRFKDLGEENFKALVLIAFAQYLQQCPFEDHVKLVNEVTEFAKTCVADESAENCDKSLHTLFGDKLCTVATLRETYGEMADCCAKQEPERNECFLQHKDDNPNLPRLVRPEVDVMCTAFHDNEETFLKKYLYEIARRHPYFYAPELLFFAKRYKAAFTECCQAADKAACLLPKLDELRDEGKASSAKQGLKCASLQKFGERAFKAWAVARLSQRFPKAEFAEVSKLVTDLTKVHTECCHGDLLECADDRADLAKYICENQDSISSKLKECCEKPLLEKSHCIAEVENDEMPADLPSLAADFVGSKDVCKNYAEAKDVFLGMFLYEYARRHPDYSVVLLLRLAKTYETTLEKCCAAADPHECYAKVFDEFKPLVEEPQNLIKQNCELFEQLGEYKFQNALLVRYTKKVPQVSTPTLVEVSRNLGKVGSKCCKHPEAKRMPCAEDCLSVFLNQLCVLHEKTPVSDRVTKCCTESLVNGRPCFSALEVDETYVPKEFNAETFTFHADICTLSEKERQIKKQTALVELVKHKPKATKEQLKAVMDDFAAFVEKCCKADDKETCFAEEGKKLVAASQAALGL

SEQ ID NO: 77 - DNA, 2502 bp, synthetic construct
  source 1..2502: mol_type = other DNA
atgacaattctgttcctcacaatggtgatcagctacttcggctgcatgaaggccgcccctatgaaggaggctaacatcagaggacaaggcggactcgcctatcccggcgtgaggactcacggcactctggaaagcgtgaatggccctaaggccggaagcagaggactcacatctctggctgacacattcgagcacgtgatcgaagagctgctggatgaggatcagaaggtgaggcctaacgaggagaacaacaaggacgccgatctgtacacatctagggtcatgctgtccagccaagtgccactggagcctcctctcctctttctgctggaggagtacaagaactatctggacgccgccaacatgtccatgagagtgagaaggcacagcgacccagccagaagaggcgagctgagcgtctgcgatagcatctccgaatgggtgactgctgccgataagaagacagccgtcgatatgagcggcggcacagtgacagtgctggaaaaagtcccagtcagcaagggccagctgaagcagtacttctacgagactaagtgcaaccctatgggctacacaaaggaaggctgtaggggcatcgacaaaaggcactggaactcccagtgtaggactactcagagctatgtgagggccctcactatggacagcaagaagaggatcggctggaggtttattaggattgacacaagctgcgtgtgcacactgacaatcaagaggggcagaggatctgatgcccacaagagcgaggtcgcccatagattcaaggatctgggcgaggagaacttcaaggctctcgtgctcatcgctttcgcccagtatctgcagcagtgccctttcgaagaccatgtgaagctggtgaacgaggtgacagagttcgccaagacatgtgtggccgatgagagcgccgagaactgcgacaagtctctgcacacactgttcggagataagctgtgcacagtcgctactctgagggagacttacggcgaaatggccgactgttgtgccaagcaagagccagagaggaatgagtgcttcctccagcacaaggacgacaaccctaatctgcctagactcgtgaggccagaagtggatgtgatgtgcacagctttccacgacaacgaggagactttcctcaagaagtacctctacgagatcgctaggagacacccttacttctatgccccagagctgctcttcttcgccaagaggtataaagccgctttcacagagtgctgtcaagccgccgacaaagctgcttgtctgctgcctaagctggatgagctgagggatgagggcaaggcctctagcgccaaacaaggcctcaaatgcgcttccctccagaagttcggagagagggcctttaaggcttgggccgtcgctaggctcagccaaagattcccaaaggccgagttcgctgaggtgagcaagctggtcacagacctcactaaggtgcacactgagtgctgtcacggcgatctgctcgaatgtgccgacgacagagctgacctcgccaaatacatctgcgagaatcaagattccatcagctccaagctcaaggagtgctgtgagaagccactgctcgagaagagccattgcatcgccgaggtcgagaacgatgagatgccagccgatctgccttctctggctgccgatttcgtgggctccaaagacgtctgcaagaactacgccgaggctaaggacgtctttctgggcatgtttctgtacgagtatgctaggagacatccagattactccgtggtgctgctgctgagactggccaagacttacgagacaacactggaaaagtgctgcgccgctgctgacccacacgagtgctacgccaaggtgtttgacgagttcaagcctctcgtcgaggagccacagaatctgattaagcagaactgtgaactcttcgagcagctgggcgagtacaagttccaaaatgctctgctggtgaggtacactaagaaggtgcctcaagtgtccactcctacactggtggaggtgagcagaaatctcggcaaggtcggcagcaaatgttgcaagcacccagaggccaagagaatgccttgtgctgaggactgtctgagcgtgtttctgaaccagctctgtgtgctgcacgagaagacaccagtcagcgacagagtgactaagtgctgcacagagtctctggtgaacggaaggccatgtttctccgctctggaggtcgacgagacttacgtgcctaaggagttcaacgccgagactttcacattccacgccgacatctgcactctctccgaaaaggaaaggcagatcaagaagcagacagctctggtggagctggtcaagcacaagccaaaggccacaaaggaacagctcaaggctgtcatggacgacttcgccgccttcgtcgagaagtgttgcaaagccgacgacaaggagacatgcttcgccgaggagggcaaaaaactggtcgctgccagccaagccgctctcggcctc

SEQ ID NO: 78 - protein, 707 aa, synthetic construct
SSSHPIFHRGEFSVCDSVSVWVGDKTTATDIKGKEVMVLGEVNINNSVFKQYFFETKCRDPNPVDSGCRGIDSKHWNSYCTTTHTFVKALTMDGKQAAWRFIRIDTACVCVLSRKAVRRAGSDAHKSEVAHRFKDLGEENFKALVLIAFAQYLQQCPFEDHVKLVNEVTEFAKTCVADESAENCDKSLHTLFGDKLCTVATLRETYGEMADCCAKQEPERNECFLQHKDDNPNLPRLVRPEVDVMCTAFHDNEETFLKKYLYEIARRHPYFYAPELLFFAKRYKAAFTECCQAADKAACLLPKLDELRDEGKASSAKQGLKCASLQKFGERAFKAWAVARLSQRFPKAEFAEVSKLVTDLTKVHTECCHGDLLECADDRADLAKYICENQDSISSKLKECCEKPLLEKSHCIAEVENDEMPADLPSLAADFVGSKDVCKNYAEAKDVFLGMFLYEYARRHPDYSVVLLLRLAKTYETTLEKCCAAADPHECYAKVFDEFKPLVEEPQNLIKQNCELFEQLGEYKFQNALLVRYTKKVPQVSTPTLVEVSRNLGKVGSKCCKHPEAKRMPCAEDCLSVFLNQLCVLHEKTPVSDRVTKCCTESLVNGRPCFSALEVDETYVPKEFNAETFTFHADICTLSEKERQIKKQTALVELVKHKPKATKEQLKAVMDDFAAFVEKCCKADDKETCFAEEGKKLVAASQAALGL

SEQ ID NO: 79 - DNA, 2484 bp, synthetic construct
  source 1..2484: mol_type = other DNA
atgagcatgctgttctacacactgatcactgcctttctgatcggcatccaagccgagcctcatagcgagagcaatgtgccagccggccacacaatcccacaagcccactggactaagctgcaacatagcctcgacacagctctgaggagagctaggtccgctccagccgctgctatcgctgctagagtggccggccagacaagaaacatcactgtggaccctaggctcttcaagaagagaaggctgaggtccccaagagtgctcttcagcacacagcctccaagggaggccgctgatacacaagatttggacttcgaggtgggaggcgctgcccctttcaataggactcataggtccaagaggagcagctcccacccaattttccacagaggcgagttcagcgtgtgcgattccgtgtccgtctgggtgggcgacaaaactactgccactgacatcaagggcaaagaggtgatggtgctcggcgaggtgaacattaacaacagcgtgttcaagcagtatttcttcgagacaaagtgtagggacccaaacccagtggatagcggctgtaggggcatcgactccaagcactggaacagctactgcacaactactcacactttcgtcaaggctctgacaatggatggcaagcaagccgcttggaggttcatcagaatcgacacagcttgtgtgtgcgtgctgtctaggaaggccgtgaggagggctggatctgatgcccacaagagcgaggtcgcccatagattcaaggatctgggcgaggagaacttcaaggctctcgtgctcatcgctttcgcccagtatctgcagcagtgccctttcgaagaccatgtgaagctggtgaacgaggtgacagagttcgccaagacatgtgtggccgatgagagcgccgagaactgcgacaagtctctgcacacactgttcggagataagctgtgcacagtcgctactctgagggagacttacggcgaaatggccgactgttgtgccaagcaagagccagagaggaatgagtgcttcctccagcacaaggacgacaaccctaatctgcctagactcgtgaggccagaagtggatgtgatgtgcacagctttccacgacaacgaggagactttcctcaagaagtacctctacgagatcgctaggagacacccttacttctatgccccagagctgctcttcttcgccaagaggtataaagccgctttcacagagtgctgtcaagccgccgacaaagctgcttgtctgctgcctaagctggatgagctgagggatgagggcaaggcctctagcgccaaacaaggcctcaaatgcgcttccctccagaagttcggagagagggcctttaaggcttgggccgtcgctaggctcagccaaagattcccaaaggccgagttcgctgaggtgagcaagctggtcacagacctcactaaggtgcacactgagtgctgtcacggcgatctgctcgaatgtgccgacgacagagctgacctcgccaaatacatctgcgagaatcaagattccatcagctccaagctcaaggagtgctgtgagaagccactgctcgagaagagccattgcatcgccgaggtcgagaacgatgagatgccagccgatctgccttctctggctgccgatttcgtgggctccaaagacgtctgcaagaactacgccgaggctaaggacgtctttctgggcatgtttctgtacgagtatgctaggagacatccagattactccgtggtgctgctgctgagactggccaagacttacgagacaacactggaaaagtgctgcgccgctgctgacccacacgagtgctacgccaaggtgtttgacgagttcaagcctctcgtcgaggagccacagaatctgattaagcagaactgtgaactcttcgagcagctgggcgagtacaagttccaaaatgctctgctggtgaggtacactaagaaggtgcctcaagtgtccactcctacactggtggaggtgagcagaaatctcggcaaggtcggcagcaaatgttgcaagcacccagaggccaagagaatgccttgtgctgaggactgtctgagcgtgtttctgaaccagctctgtgtgctgcacgagaagacaccagtcagcgacagagtgactaagtgctgcacagagtctctggtgaacggaaggccatgtttctccgctctggaggtcgacgagacttacgtgcctaaggagttcaacgccgagactttcacattccacgccgacatctgcactctctccgaaaaggaaaggcagatcaagaagcagacagctctggtggagctggtcaagcacaagccaaaggccacaaaggaacagctcaaggctgtcatggacgacttcgccgccttcgtcgagaagtgttgcaaagccgacgacaaggagacatgcttcgccgaggagggcaaaaaactggtcgctgccagccaagccgctctcggcctc

SEQ ID NO: 80 - protein, 706 aa, synthetic construct
YAEHKSHRGEYSVCDSESLWVTDKSSAIDIRGHQVTVLGEIKTGNSPVKQYFYETRCKEARPVKNGCRGIDDKHWNSQCKTSQTYVRALTSENNKLVGWRWIRIDTSCVCALSRKIGRTGSDAHKSEVAHRFKDLGEENFKALVLIAFAQYLQQCPFEDHVKLVNEVTEFAKTCVADESAENCDKSLHTLFGDKLCTVATLRETYGEMADCCAKQEPERNECFLQHKDDNPNLPRLVRPEVDVMCTAFHDNEETFLKKYLYEIARRHPYFYAPELLFFAKRYKAAFTECCQAADKAACLLPKLDELRDEGKASSAKQGLKCASLQKFGERAFKAWAVARLSQRFPKAEFAEVSKLVTDLTKVHTECCHGDLLECADDRADLAKYICENQDSISSKLKECCEKPLLEKSHCIAEVENDEMPADLPSLAADFVGSKDVCKNYAEAKDVFLGMFLYEYARRHPDYSVVLLLRLAKTYETTLEKCCAAADPHECYAKVFDEFKPLVEEPQNLIKQNCELFEQLGEYKFQNALLVRYTKKVPQVSTPTLVEVSRNLGKVGSKCCKHPEAKRMPCAEDCLSVFLNQLCVLHEKTPVSDRVTKCCTESLVNGRPCFSALEVDETYVPKEFNAETFTFHADICTLSEKERQIKKQTALVELVKHKPKATKEQLKAVMDDFAAFVEKCCKADDKETCFAEEGKKLVAASQAALGL

SEQ ID NO: 81 - DNA, 2532 bp, synthetic construct
  source 1..2532: mol_type = other DNA
atgtccattctgttctacgtcatctttctggcctatctgaggggcatccaaggcaataacatggaccagaggtctctgccagaggactctctgaactctctgatcatcaagctgatccaagccgatattctgaagaacaagctgagcaaacagatggtggacgtcaaggagaactaccagagcacactcccaaaggctgaggcccctagggaaccagaaagaggcggcccagccaaaagcgccttccagccagtgattgctatggacactgagctcctcagacagcagagaaggtacaactccccaagggtgctgctgagcgacagcactcctctggagcctccaccactgtacctcatggaggattacgtgggcagcccagtggtggccaataggacttctaggaggaagaggtacgctgaacacaagagccataggggagagtacagcgtctgcgattccgagagcctctgggtgactgacaagtcctccgctatcgatattaggggccaccaagtgacagtgctcggcgaaatcaagactggcaactccccagtgaagcagtacttctacgagacaaggtgcaaggaggctaggccagtgaagaacggctgtaggggaattgacgacaagcactggaacagccagtgcaagactagccagacatatgtgagggccctcactagcgagaacaacaagctcgtgggctggagatggattaggatcgacacaagctgtgtctgcgctctgtctaggaagatcggaaggactggatctgatgcccacaagagcgaggtcgcccatagattcaaggatctgggcgaggagaacttcaaggctctcgtgctcatcgctttcgcccagtatctgcagcagtgccctttcgaagaccatgtgaagctggtgaacgaggtgacagagttcgccaagacatgtgtggccgatgagagcgccgagaactgcgacaagtctctgcacacactgttcggagataagctgtgcacagtcgctactctgagggagacttacggcgaaatggccgactgttgtgccaagcaagagccagagaggaatgagtgcttcctccagcacaaggacgacaaccctaatctgcctagactcgtgaggccagaagtggatgtgatgtgcacagctttccacgacaacgaggagactttcctcaagaagtacctctacgagatcgctaggagacacccttacttctatgccccagagctgctcttcttcgccaagaggtataaagccgctttcacagagtgctgtcaagccgccgacaaagctgcttgtctgctgcctaagctggatgagctgagggatgagggcaaggcctctagcgccaaacaaggcctcaaatgcgcttccctccagaagttcggagagagggcctttaaggcttgggccgtcgctaggctcagccaaagattcccaaaggccgagttcgctgaggtgagcaagctggtcacagacctcactaaggtgcacactgagtgctgtcacggcgatctgctcgaatgtgccgacgacagagctgacctcgccaaatacatctgcgagaatcaagattccatcagctccaagctcaaggagtgctgtgagaagccactgctcgagaagagccattgcatcgccgaggtcgagaacgatgagatgccagccgatctgccttctctggctgccgatttcgtgggctccaaagacgtctgcaagaactacgccgaggctaaggacgtctttctgggcatgtttctgtacgagtatgctaggagacatccagattactccgtggtgctgctgctgagactggccaagacttacgagacaacactggaaaagtgctgcgccgctgctgacccacacgagtgctacgccaaggtgtttgacgagttcaagcctctcgtcgaggagccacagaatctgattaagcagaactgtgaactcttcgagcagctgggcgagtacaagttccaaaatgctctgctggtgaggtacactaagaaggtgcctcaagtgtccactcctacactggtggaggtgagcagaaatctcggcaaggtcggcagcaaatgttgcaagcacccagaggccaagagaatgccttgtgctgaggactgtctgagcgtgtttctgaaccagctctgtgtgctgcacgagaagacaccagtcagcgacagagtgactaagtgctgcacagagtctctggtgaacggaaggccatgtttctccgctctggaggtcgacgagacttacgtgcctaaggagttcaacgccgagactttcacattccacgccgacatctgcactctctccgaaaaggaaaggcagatcaagaagcagacagctctggtggagctggtcaagcacaagccaaaggccacaaaggaacagctcaaggctgtcatggacgacttcgccgccttcgtcgagaagtgttgcaaagccgacgacaaggagacatgcttcgccgaggagggcaaaaaactggtcgctgccagccaagccgctctcggcctc

SEQ ID NO: 82 - protein, 717 aa, synthetic construct
GVSETAPASRRGELAVCDAVSGWVTDRRTAVDLRGREVEVLGEVPAAGGSPLRQYFFETRCKADNAEEGGPGAGGGGCRGVDRRHWVSECKAKQSYVRALTADAQGRVGWRWIRIDTACVCTLLSRTGRAGSDAHKSEVAHRFKDLGEENFKALVLIAFAQYLQQCPFEDHVKLVNEVTEFAKTCVADESAENCDKSLHTLFGDKLCTVATLRETYGEMADCCAKQEPERNECFLQHKDDNPNLPRLVRPEVDVMCTAFHDNEETFLKKYLYEIARRHPYFYAPELLFFAKRYKAAFTECCQAADKAACLLPKLDELRDEGKASSAKQGLKCASLQKFGERAFKAWAVARLSQRFPKAEFAEVSKLVTDLTKVHTECCHGDLLECADDRADLAKYICENQDSISSKLKECCEKPLLEKSHCIAEVENDEMPADLPSLAADFVGSKDVCKNYAEAKDVFLGMFLYEYARRHPDYSVVLLLRLAKTYETTLEKCCAAADPHECYAKVFDEFKPLVEEPQNLIKQNCELFEQLGEYKFQNALLVRYTKKVPQVSTPTLVEVSRNLGKVGSKCCKHPEAKRMPCAEDCLSVFLNQLCVLHEKTPVSDRVTKCCTESLVNGRPCFSALEVDETYVPKEFNAETFTFHADICTLSEKERQIKKQTALVELVKHKPKATKEQLKAVMDDFAAFVEKCCKADDKETCFAEEGKKLVAASQAALGL

SEQ ID NO: 83 - DNA, 2391 bp, synthetic construct
  source 1..2391: mol_type = other DNA
atgctgccactgccaagctgttctctgcctattctgctgctgtttctgctcccaagcgtgcctatcgagtcccagcctccaccttccacactgcctccatttctggccccagagtgggatctgctgagcccaagggtggtgctcagcagaggcgctccagccggacctccactgctgtttctgctggaagctggcgcctttagagaaagcgccggagctccagccaataggtctaggaggggcgtgtccgagactgctccagccagcagaagaggcgaactggctgtgtgcgatgccgtgagcggctgggtcacagataggaggactgccgtggatctgagaggaagggaggtggaggtgctgggagaagtgccagctgccggaggcagccctctgaggcagtacttcttcgagacaaggtgcaaggccgacaatgccgaagaaggaggccccggcgctggaggcggaggatgtagaggcgtggataggagacattgggtgagcgagtgtaaggccaagcagagctatgtgagagctctgactgctgatgctcaaggcagagtgggatggaggtggatcagaatcgacactgcttgtgtctgcacactgctgtctaggactggcagagctggatctgatgcccacaagagcgaggtcgcccatagattcaaggatctgggcgaggagaacttcaaggctctcgtgctcatcgctttcgcccagtatctgcagcagtgccctttcgaagaccatgtgaagctggtgaacgaggtgacagagttcgccaagacatgtgtggccgatgagagcgccgagaactgcgacaagtctctgcacacactgttcggagataagctgtgcacagtcgctactctgagggagacttacggcgaaatggccgactgttgtgccaagcaagagccagagaggaatgagtgcttcctccagcacaaggacgacaaccctaatctgcctagactcgtgaggccagaagtggatgtgatgtgcacagctttccacgacaacgaggagactttcctcaagaagtacctctacgagatcgctaggagacacccttacttctatgccccagagctgctcttcttcgccaagaggtataaagccgctttcacagagtgctgtcaagccgccgacaaagctgcttgtctgctgcctaagctggatgagctgagggatgagggcaaggcctctagcgccaaacaaggcctcaaatgcgcttccctccagaagttcggagagagggcctttaaggcttgggccgtcgctaggctcagccaaagattcccaaaggccgagttcgctgaggtgagcaagctggtcacagacctcactaaggtgcacactgagtgctgtcacggcgatctgctcgaatgtgccgacgacagagctgacctcgccaaatacatctgcgagaatcaagattccatcagctccaagctcaaggagtgctgtgagaagccactgctcgagaagagccattgcatcgccgaggtcgagaacgatgagatgccagccgatctgccttctctggctgccgatttcgtgggctccaaagacgtctgcaagaactacgccgaggctaaggacgtctttctgggcatgtttctgtacgagtatgctaggagacatccagattactccgtggtgctgctgctgagactggccaagacttacgagacaacactggaaaagtgctgcgccgctgctgacccacacgagtgctacgccaaggtgtttgacgagttcaagcctctcgtcgaggagccacagaatctgattaagcagaactgtgaactcttcgagcagctgggcgagtacaagttccaaaatgctctgctggtgaggtacactaagaaggtgcctcaagtgtccactcctacactggtggaggtgagcagaaatctcggcaaggtcggcagcaaatgttgcaagcacccagaggccaagagaatgccttgtgctgaggactgtctgagcgtgtttctgaaccagctctgtgtgctgcacgagaagacaccagtcagcgacagagtgactaagtgctgcacagagtctctggtgaacggaaggccatgtttctccgctctggaggtcgacgagacttacgtgcctaaggagttcaacgccgagactttcacattccacgccgacatctgcactctctccgaaaaggaaaggcagatcaagaagcagacagctctggtggagctggtcaagcacaagccaaaggccacaaaggaacagctcaaggctgtcatggacgacttcgccgccttcgtcgagaagtgttgcaaagccgacgacaaggagacatgcttcgccgaggagggcaaaaaactggtcgctgccagccaagccgctctcggcctc

SEQ ID NO: 84 - protein, 229 aa, Homo sapiens
APMKEANIRGQGGLAYPGVRTHGTLESVNGPKAGSRGLTSLADTFEHVIEELLDEDQKVRPNEENNKDADLYTSRVMLSSQVPLEPPLLFLLEEYKNYLDAANMSMRVRRHSDPARRGELSVCDSISEWVTAADKKTAVDMSGGTVTVLEKVPVSKGQLKQYFYETKCNPMGYTKEGCRGIDKRHWNSQCRTTQSYVRALTMDSKKRIGWRFIRIDTSCVCTLTIKRGR

SEQ ID NO: 85 - protein, 816 aa, synthetic construct
DAHKSEVAHRFKDLGEENFKALVLIAFAQYLQQCPFEDHVKLVNEVTEFAKTCVADESAENCDKSLHTLFGDKLCTVATLRETYGEMADCCAKQEPERNECFLQHKDDNPNLPRLVRPEVDVMCTAFHDNEETFLKKYLYEIARRHPYFYAPELLFFAKRYKAAFTECCQAADKAACLLPKLDELRDEGKASSAKQGLKCASLQKFGERAFKAWAVARLSQRFPKAEFAEVSKLVTDLTKVHTECCHGDLLECADDRADLAKYICENQDSISSKLKECCEKPLLEKSHCIAEVENDEMPADLPSLAADFVGSKDVCKNYAEAKDVFLGMFLYEYARRHPDYSVVLLLRLAKTYETTLEKCCAAADPHECYAKVFDEFKPLVEEPQNLIKQNCELFEQLGEYKFQNALLVRYTKKVPQVSTPTLVEVSRNLGKVGSKCCKHPEAKRMPCAEDCLSVFLNQLCVLHEKTPVSDRVTKCCTESLVNGRPCFSALEVDETYVPKEFNAETFTFHADICTLSEKERQIKKQTALVELVKHKPKATKEQLKAVMDDFAAFVEKCCKADDKETCFAEEGKKLVAASQAALGLGSAPMKEANIRGQGGLAYPGVRTHGTLESVNGPKAGSRGLTSLADTFEHVIEELLDEDQKVRPNEENNKDADLYTSRVMLSSQVPLEPPLLFLLEEYKNYLDAANMSMRVRRHSDPARRGELSVCDSISEWVTAADKKTAVDMSGGTVTVLEKVPVSKGQLKQYFYETKCNPMGYTKEGCRGIDKRHWNSQCRTTQSYVRALTMDSKKRIGWRFIRIDTSCVCTLTIKRGR

SEQ ID NO: 86 - protein, 816 aa, synthetic construct
APMKEANIRGQGGLAYPGVRTHGTLESVNGPKAGSRGLTSLADTFEHVIEELLDEDQKVRPNEENNKDADLYTSRVMLSSQVPLEPPLLFLLEEYKNYLDAANMSMRVRRHSDPARRGELSVCDSISEWVTAADKKTAVDMSGGTVTVLEKVPVSKGQLKQYFYETKCNPMGYTKEGCRGIDKRHWNSQCRTTQSYVRALTMDSKKRIGWRFIRIDTSCVCTLTIKRGRGSDAHKSEVAHRFKDLGEENFKALVLIAFAQYLQQCPFEDHVKLVNEVTEFAKTCVADESAENCDKSLHTLFGDKLCTVATLRETYGEMADCCAKQEPERNECFLQHKDDNPNLPRLVRPEVDVMCTAFHDNEETFLKKYLYEIARRHPYFYAPELLFFAKRYKAAFTECCQAADKAACLLPKLDELRDEGKASSAKQGLKCASLQKFGERAFKAWAVARLSQRFPKAEFAEVSKLVTDLTKVHTECCHGDLLECADDRADLAKYICENQDSISSKLKECCEKPLLEKSHCIAEVENDEMPADLPSLAADFVGSKDVCKNYAEAKDVFLGMFLYEYARRHPDYSVVLLLRLAKTYETTLEKCCAAADPHECYAKVFDEFKPLVEEPQNLIKQNCELFEQLGEYKFQNALLVRYTKKVPQVSTPTLVEVSRNLGKVGSKCCKHPEAKRMPCAEDCLSVFLNQLCVLHEKTPVSDRVTKCCTESLVNGRPCFSALEVDETYVPKEFNAETFTFHADICTLSEKERQIKKQTALVELVKHKPKATKEQLKAVMDDFAAFVEKCCKADDKETCFAEEGKKLVAASQAALGL

SEQ ID NO: 87 - protein, 223 aa, Homo sapiens
EPHSESNVPAGHTIPQAHWTKLQHSLDTALRRARSAPAAAIAARVAGQTRNITVDPRLFKKRRLRSPRVLFSTQPPREAADTQDLDFEVGGAAPFNRTHRSKRSSSHPIFHRGEFSVCDSVSVWVGDKTTATDIKGKEVMVLGEVNINNSVFKQYFFETKCRDPNPVDSGCRGIDSKHWNSYCTTTHTFVKALTMDGKQAAWRFIRIDTACVCVLSRKAVRRA

SEQ ID NO: 88 - protein, 810 aa, synthetic construct
DAHKSEVAHRFKDLGEENFKALVLIAFAQYLQQCPFEDHVKLVNEVTEFAKTCVADESAENCDKSLHTLFGDKLCTVATLRETYGEMADCCAKQEPERNECFLQHKDDNPNLPRLVRPEVDVMCTAFHDNEETFLKKYLYEIARRHPYFYAPELLFFAKRYKAAFTECCQAADKAACLLPKLDELRDEGKASSAKQGLKCASLQKFGERAFKAWAVARLSQRFPKAEFAEVSKLVTDLTKVHTECCHGDLLECADDRADLAKYICENQDSISSKLKECCEKPLLEKSHCIAEVENDEMPADLPSLAADFVGSKDVCKNYAEAKDVFLGMFLYEYARRHPDYSVVLLLRLAKTYETTLEKCCAAADPHECYAKVFDEFKPLVEEPQNLIKQNCELFEQLGEYKFQNALLVRYTKKVPQVSTPTLVEVSRNLGKVGSKCCKHPEAKRMPCAEDCLSVFLNQLCVLHEKTPVSDRVTKCCTESLVNGRPCFSALEVDETYVPKEFNAETFTFHADICTLSEKERQIKKQTALVELVKHKPKATKEQLKAVMDDFAAFVEKCCKADDKETCFAEEGKKLVAASQAALGLGSEPHSESNVPAGHTIPQAHWTKLQHSLDTALRRARSAPAAAIAARVAGQTRNITVDPRLFKKRRLRSPRVLFSTQPPREAADTQDLDFEVGGAAPFNRTHRSKRSSSHPIFHRGEFSVCDSVSVWVGDKTTATDIKGKEVMVLGEVNINNSVFKQYFFETKCRDPNPVDSGCRGIDSKHWNSYCTTTHTFVKALTMDGKQAAWRFIRIDTACVCVLSRKAVRRA

SEQ ID NO: 89 - protein, 810 aa, synthetic construct
EPHSESNVPAGHTIPQAHWTKLQHSLDTALRRARSAPAAAIAARVAGQTRNITVDPRLFKKRRLRSPRVLFSTQPPREAADTQDLDFEVGGAAPFNRTHRSKRSSSHPIFHRGEFSVCDSVSVWVGDKTTATDIKGKEVMVLGEVNINNSVFKQYFFETKCRDPNPVDSGCRGIDSKHWNSYCTTTHTFVKALTMDGKQAAWRFIRIDTACVCVLSRKAVRRAGSDAHKSEVAHRFKDLGEENFKALVLIAFAQYLQQCPFEDHVKLVNEVTEFAKTCVADESAENCDKSLHTLFGDKLCTVATLRETYGEMADCCAKQEPERNECFLQHKDDNPNLPRLVRPEVDVMCTAFHDNEETFLKKYLYEIARRHPYFYAPELLFFAKRYKAAFTECCQAADKAACLLPKLDELRDEGKASSAKQGLKCASLQKFGERAFKAWAVARLSQRFPKAEFAEVSKLVTDLTKVHTECCHGDLLECADDRADLAKYICENQDSISSKLKECCEKPLLEKSHCIAEVENDEMPADLPSLAADFVGSKDVCKNYAEAKDVFLGMFLYEYARRHPDYSVVLLLRLAKTYETTLEKCCAAADPHECYAKVFDEFKPLVEEPQNLIKQNCELFEQLGEYKFQNALLVRYTKKVPQVSTPTLVEVSRNLGKVGSKCCKHPEAKRMPCAEDCLSVFLNQLCVLHEKTPVSDRVTKCCTESLVNGRPCFSALEVDETYVPKEFNAETFTFHADICTLSEKERQIKKQTALVELVKHKPKATKEQLKAVMDDFAAFVEKCCKADDKETCFAEEGKKLVAASQAALGL

SEQ ID NO: 90 - protein, 239 aa, Homo sapiens
NNMDQRSLPEDSLNSLIIKLIQADILKNKLSKQMVDVKENYQSTLPKAEAPREPERGGPAKSAFQPVIAMDTELLRQQRRYNSPRVLLSDSTPLEPPPLYLMEDYVGSPVVANRTSRRKRYAEHKSHRGEYSVCDSESLWVTDKSSAIDIRGHQVTVLGEIKTGNSPVKQYFYETRCKEARPVKNGCRGIDDKHWNSQCKTSQTYVRALTSENNKLVGWRWIRIDTSCVCALSRKIGRT

SEQ ID NO: 91 - protein, 826 aa, synthetic construct
NNMDQRSLPEDSLNSLIIKLIQADILKNKLSKQMVDVKENYQSTLPKAEAPREPERGGPAKSAFQPVIAMDTELLRQQRRYNSPRVLLSDSTPLEPPPLYLMEDYVGSPVVANRTSRRKRYAEHKSHRGEYSVCDSESLWVTDKSSAIDIRGHQVTVLGEIKTGNSPVKQYFYETRCKEARPVKNGCRGIDDKHWNSQCKTSQTYVRALTSENNKLVGWRWIRIDTSCVCALSRKIGRTGSDAHKSEVAHRFKDLGEENFKALVLIAFAQYLQQCPFEDHVKLVNEVTEFAKTCVADESAENCDKSLHTLFGDKLCTVATLRETYGEMADCCAKQEPERNECFLQHKDDNPNLPRLVRPEVDVMCTAFHDNEETFLKKYLYEIARRHPYFYAPELLFFAKRYKAAFTECCQAADKAACLLPKLDELRDEGKASSAKQGLKCASLQKFGERAFKAWAVARLSQRFPKAEFAEVSKLVTDLTKVHTECCHGDLLECADDRADLAKYICENQDSISSKLKECCEKPLLEKSHCIAEVENDEMPADLPSLAADFVGSKDVCKNYAEAKDVFLGMFLYEYARRHPDYSVVLLLRLAKTYETTLEKCCAAADPHECYAKVFDEFKPLVEEPQNLIKQNCELFEQLGEYKFQNALLVRYTKKVPQVSTPTLVEVSRNLGKVGSKCCKHPEAKRMPCAEDCLSVFLNQLCVLHEKTPVSDRVTKCCTESLVNGRPCFSALEVDETYVPKEFNAETFTFHADICTLSEKERQIKKQTALVELVKHKPKATKEQLKAVMDDFAAFVEKCCKADDKETCFAEEGKKLVAASQAALGL

SEQ ID NO: 92 - protein, 826 aa, synthetic construct
DAHKSEVAHRFKDLGEENFKALVLIAFAQYLQQCPFEDHVKLVNEVTEFAKTCVADESAENCDKSLHTLFGDKLCTVATLRETYGEMADCCAKQEPERNECFLQHKDDNPNLPRLVRPEVDVMCTAFHDNEETFLKKYLYEIARRHPYFYAPELLFFAKRYKAAFTECCQAADKAACLLPKLDELRDEGKASSAKQGLKCASLQKFGERAFKAWAVARLSQRFPKAEFAEVSKLVTDLTKVHTECCHGDLLECADDRADLAKYICENQDSISSKLKECCEKPLLEKSHCIAEVENDEMPADLPSLAADFVGSKDVCKNYAEAKDVFLGMFLYEYARRHPDYSVVLLLRLAKTYETTLEKCCAAADPHECYAKVFDEFKPLVEEPQNLIKQNCELFEQLGEYKFQNALLVRYTKKVPQVSTPTLVEVSRNLGKVGSKCCKHPEAKRMPCAEDCLSVFLNQLCVLHEKTPVSDRVTKCCTESLVNGRPCFSALEVDETYVPKEFNAETFTFHADICTLSEKERQIKKQTALVELVKHKPKATKEQLKAVMDDFAAFVEKCCKADDKETCFAEEGKKLVAASQAALGLGSNNMDQRSLPEDSLNSLIIKLIQADILKNKLSKQMVDVKENYQSTLPKAEAPREPERGGPAKSAFQPVIAMDTELLRQQRRYNSPRVLLSDSTPLEPPPLYLMEDYVGSPVVANRTSRRKRYAEHKSHRGEYSVCDSESLWVTDKSSAIDIRGHQVTVLGEIKTGNSPVKQYFYETRCKEARPVKNGCRGIDDKHWNSQCKTSQTYVRALTSENNKLVGWRWIRIDTSCVCALSRKIGRT

SEQ ID NO: 93 - protein, 186 aa, Homo sapiens
QPPPSTLPPFLAPEWDLLSPRVVLSRGAPAGPPLLFLLEAGAFRESAGAPANRSRRGVSETAPASRRGELAVCDAVSGWVTDRRTAVDLRGREVEVLGEVPAAGGSPLRQYFFETRCKADNAEEGGPGAGGGGCRGVDRRHWVSECKAKQSYVRALTADAQGRVGWRWIRIDTACVCTLLSRTGRA

SEQ ID NO: 94 - protein, 773 aa, synthetic construct
DAHKSEVAHRFKDLGEENFKALVLIAFAQYLQQCPFEDHVKLVNEVTEFAKTCVADESAENCDKSLHTLFGDKLCTVATLRETYGEMADCCAKQEPERNECFLQHKDDNPNLPRLVRPEVDVMCTAFHDNEETFLKKYLYEIARRHPYFYAPELLFFAKRYKAAFTECCQAADKAACLLPKLDELRDEGKASSAKQGLKCASLQKFGERAFKAWAVARLSQRFPKAEFAEVSKLVTDLTKVHTECCHGDLLECADDRADLAKYICENQDSISSKLKECCEKPLLEKSHCIAEVENDEMPADLPSLAADFVGSKDVCKNYAEAKDVFLGMFLYEYARRHPDYSVVLLLRLAKTYETTLEKCCAAADPHECYAKVFDEFKPLVEEPQNLIKQNCELFEQLGEYKFQNALLVRYTKKVPQVSTPTLVEVSRNLGKVGSKCCKHPEAKRMPCAEDCLSVFLNQLCVLHEKTPVSDRVTKCCTESLVNGRPCFSALEVDETYVPKEFNAETFTFHADICTLSEKERQIKKQTALVELVKHKPKATKEQLKAVMDDFAAFVEKCCKADDKETCFAEEGKKLVAASQAALGLGSQPPPSTLPPFLAPEWDLLSPRVVLSRGAPAGPPLLFLLEAGAFRESAGAPANRSRRGVSETAPASRRGELAVCDAVSGWVTDRRTAVDLRGREVEVLGEVPAAGGSPLRQYFFETRCKADNAEEGGPGAGGGGCRGVDRRHWVSECKAKQSYVRALTADAQGRVGWRWIRIDTACVCTLLSRTGRA

SEQ ID NO: 95 - protein, 773 aa, synthetic construct
QPPPSTLPPFLAPEWDLLSPRVVLSRGAPAGPPLLFLLEAGAFRESAGAPANRSRRGVSETAPASRRGELAVCDAVSGWVTDRRTAVDLRGREVEVLGEVPAAGGSPLRQYFFETRCKADNAEEGGPGAGGGGCRGVDRRHWVSECKAKQSYVRALTADAQGRVGWRWIRIDTACVCTLLSRTGRAGSDAHKSEVAHRFKDLGEENFKALVLIAFAQYLQQCPFEDHVKLVNEVTEFAKTCVADESAENCDKSLHTLFGDKLCTVATLRETYGEMADCCAKQEPERNECFLQHKDDNPNLPRLVRPEVDVMCTAFHDNEETFLKKYLYEIARRHPYFYAPELLFFAKRYKAAFTECCQAADKAACLLPKLDELRDEGKASSAKQGLKCASLQKFGERAFKAWAVARLSQRFPKAEFAEVSKLVTDLTKVHTECCHGDLLECADDRADLAKYICENQDSISSKLKECCEKPLLEKSHCIAEVENDEMPADLPSLAADFVGSKDVCKNYAEAKDVFLGMFLYEYARRHPDYSVVLLLRLAKTYETTLEKCCAAADPHECYAKVFDEFKPLVEEPQNLIKQNCELFEQLGEYKFQNALLVRYTKKVPQVSTPTLVEVSRNLGKVGSKCCKHPEAKRMPCAEDCLSVFLNQLCVLHEKTPVSDRVTKCCTESLVNGRPCFSALEVDETYVPKEFNAETFTFHADICTLSEKERQIKKQTALVELVKHKPKATKEQLKAVMDDFAAFVEKCCKADDKETCFAEEGKKLVAASQAALGL

SEQ ID NO: 96 - protein, 11 aa, synthetic construct
QSLVHSNGNTY

SEQ ID NO: 97 - protein, 6 aa, synthetic construct
KVSNRF

SEQ ID NO: 98 - protein, 9 aa, synthetic construct
SQSTHVPWT

SEQ ID NO: 99 - protein, 5 aa, synthetic construct
NYWLG

SEQ ID NO: 100 - protein, 8 aa, synthetic construct
IYPGGDYP

SEQ ID NO: 101 - protein, 9 aa, synthetic construct
SGNYDEVAY

SEQ ID NO: 102 - protein, 8 aa, synthetic construct
GYSFMNYW

SEQ ID NO: 103 - protein, 8 aa, synthetic construct
IYPGGDYP

SEQ ID NO: 104 - protein, 9 aa, synthetic construct
SGNYDEVAY

SEQ ID NO: 105 - protein, 9 aa, synthetic construct
GSIFDIYVM

SEQ ID NO: 106 - protein, 10 aa, synthetic construct
GSIFDIYVMR

SEQ ID NO: 107 - protein, 8 aa, synthetic construct
IYDGGRND

SEQ ID NO: 108 - protein, 12 aa, synthetic construct
IYDGGRNDYDNV

SEQ ID NO: 109 - protein, 8 aa, synthetic construct
LTYAGRPY

SEQ ID NO: 110 - protein, 11 aa, synthetic construct
NVLTYAGRPYW

SEQ ID NO: 111 - protein, 8 aa, synthetic construct
IYAGGRND

SEQ ID NO: 112 - protein, 12 aa, synthetic construct
IYAGGRNDYDNV

SEQ ID NO: 113 - DNA, 145 bp, Adeno-associated dependoparvovirus A
  source 1..145: mol_type = genomic DNA
ttggccactccctctctgcgcgctcgctcgctcactgaggccgggcgaccaaaggtcgcccgacgcccgggctttgcccgggcggcctcagtgagcgagcgagcgcgcagagagggagtggccaactccatcactaggggttcct

SEQ ID NO: 114 - DNA, 145 bp, Adeno-associated dependoparvovirus A
  source 1..145: mol_type = genomic DNA
aggaacccctagtgatggagttggccactccctctctgcgcgctcgctcgctcactgaggccgggcgaccaaaggtcgcccgacgcccgggctttgcccgggcggcctcagtgagcgagcgagcgcgcagagagggagtggccaa

SEQ ID NO: 115 - DNA, 141 bp, synthetic construct
  source 1..141: mol_type = other DNA
cctgcaggcagctgcgcgctcgctcgctcactgaggccgcccgggcaaagcccgggcgtcgggcgacctttggtcgcccggcctcagtgagcgagcgagcgcgcagagagggagtggccaactccatcactaggggttcct

SEQ ID NO: 116 - DNA, 141 bp, synthetic construct
  source 1..141: mol_type = other DNA
aggaacccctagtgatggagttggccactccctctctgcgcgctcgctcgctcactgaggccgggcgaccaaaggtcgcccgacgcccgggctttgcccgggcggcctcagtgagcgagcgagcgcgcagctgcctgcagg

SEQ ID NO: 117 - DNA, 589 bp, synthetic construct
  source 1..589: mol_type = other DNA
tttgaaagaccccacccgtaggtggcaagctagcttaagtaacgccactttgcaaggcatggaaaaatacataactgagaatagaaaagttcagatcaaggtcaggaacaaagaaacagctgaataccaaacaggatatctgtggtaagcggttcctgccccggctcagggccaagaacagatgagacagctgagtgatgggccaaacaggatatctgtggtaagcagttcctgccccggctcggggccaagaacagatggtccccagatgcggtccagccctcagcagtttctagtgaatcatcagatgtttccagggtgccccaaggacctgaaaatgaccctgtaccttatttgaactaaccaatcagttcgcttctcgcttctgttcgcgcgcttccgctctccgagctcaataaaagagcccacaacccctcactcggcgcgccagtcttccgatagactgcgtcgcccgggtacccgtattcccaataaagcctcttgctgtttgcatccgaatcgtggtctcgctgttccttgggagggtctcctctgagtgattgactacccacgacgggggtctttcatt

SEQ ID NO: 118 - DNA, 594 bp, synthetic construct
  source 1..594: mol_type = other DNA
aatgaaagaccccacctgtaggtttggcaagctagcttaagtaacgccattttgcaaggcatggaaaaatacataactgagaatagagaagttcagatcaaggtcaggaacagatggaacagctgaatatgggccaaacaggatatctgtggtaagcagttcctgccccggctcagggccaagaacagatggaacagctgaatatgggccaaacaggatatctgtggtaagcagttcctgccccggctcagggccaagaacagatggtccccagatgcggtccagccctcagcagtttctagagaaccatcagatgtttccagggtgccccaaggacctgaaatgaccctgtgccttatttgaactaaccaatcagttcgcttctcgcttctgttcgcgcgcttctgctccccgagctcaataaaagagcccacaacccctcactcggggcgccagtcctccgattgactgagtcgcccgggtacccgtgtatccaataaaccctcttgcagttgcatccgacttgtggtctcgctgttccttgggagggtctcctctgagtgattgactacccgtcagcgggggtctttcatt

SEQ ID NO: 119 - DNA, 52 bp, synthetic construct
  source 1..52: mol_type = other DNA
accaaacaagagaagaaacttgtttggaatatataatgaagttagacaggat

SEQ ID NO: 120 - DNA, 54 bp, synthetic construct
  source 1..54: mol_type = other DNA
acaaggagacaagaaaatttgaaagaataaatatctcttaaactcttgtctggt

SEQ ID NO: 121 - DNA, 559 bp, synthetic construct
  source 1..559: mol_type = other DNA
agatcattttgatggcagagttcagtttaccgggtcacattgtacctgggaagattcaaggatttatggaaaaagtcaacaacaggagtcagagcagccggaaaagcatggactctgtacttaggactgcgctttgagcaatggcacagcaagctataaccctgtttgcagtcagcacacaaactgtggttcaaagctccactttatctcttcttgtggaattcagatatcagatcagttttgctcaaatgggagacaaagagattaagctcttatgtaaaatttgctgttttacataactttaatgaatggacaaagtcttgtgcatgggggtgggggtggggttagaggggaacagctccagatggcaaacatacgcaagggatttagtcaaacaactttttggcaaagatggtatgattttgtaatggggtaggaaccaatgaaatgcgaggtaagtatggttaataatctacagttattggttaaagaagtatattagagcgagtctttctgcacacagatcaccttcctatcaaccccactagcctctggcaaa

SEQ ID NO: 122 - DNA, 225 bp, synthetic construct
  source 1..225: mol_type = other DNA
ggagtcgctgcgttgccttcgccccgtgccccgctccgcgccgcctcgcgccgcccgccccggctctgactgaccgcgttactcccacaggtgagcgggcgggacggcccttctcctccgggctgtaattagcaagaggtaagggtttaagggatggttggttggtggggtattaatgtttaattacctggagcacctgcctgaaatcactttttttcaggttgg

SEQ ID NO: 123 - DNA, 1866 bp, synthetic construct
  source 1..1866: mol_type = other DNA
acgccggggttttacgagattgtgattaaggtccccagcgaccttgacgagcatctgcccggcatttctgacagctttgtgaactgggtggccgagaaggaatgggagttgccgccagattctgacatggatctgaatctgattgagcaggcacccctgaccgtggccgagaagctgcagcgcgactttctgacggaatggcgccgtgtgagtaaggccccggaggcccttttctttgtgcaatttgagaagggagagagctacttccacatgcacgtgctcgtggaaaccaccggggtgaaatccatggttttgggacgtttcctgagtcagattcgcgaaaaactgattcagagaatttaccgcgggatcgagccgactttgccaaactggttcgcggtcacaaagaccagaaatggcgccggaggcgggaacaaggtggtggatgagtgctacatccccaattacttgctccccaaaacccagcctgagctccagtgggcgtggactaatatggaacagtatttaagcgcctgtttgaatctcacggagcgtaaacggttggtggcgcagcatctgacgcacgtgtcgcagacgcaggagcagaacaaagagaatcagaatcccaattctgatgcgccggtgatcagatcaaaaacttcagccaggtacatggagctggtcgggtggctcgtggacaaggggattacctcggagaagcagtggatccaggaggaccaggcctcatacatctccttcaatgcggcctccaactcgcggtcccaaatcaaggctgccttggacaatgcgggaaagattatgagcctgactaaaaccgcccccgactacctggtgggccagcagcccgtggaggacatttccagcaatcggatttataaaattttggaactaaacgggtacgatccccaatatgcggcttccgtctttctgggatgggccacgaaaaagttcggcaagaggaacaccatctggctgtttgggcctgcaactaccgggaagaccaacatcgcggaggccatagcccacactgtgcccttctacgggtgcgtaaactggaccaatgagaactttcccttcaacgactgtgtcgacaagatggtgatctggtgggaggaggggaagatgaccgccaaggtcgtggagtcggccaaagccattctcggaggaagcaaggtgcgcgtggaccagaaatgcaagtcctcggcccagatagacccgactcccgtgatcgtcacctccaacaccaacatgtgcgccgtgattgacgggaactcaacgaccttcgaacaccagcagccgttgcaagaccggatgttcaaatttgaactcacccgccgtctggatcatgactttgggaaggtcaccaagcaggaagtcaaagactttttccggtgggcaaaggatcacgtggttgaggtggagcatgaattctacgtcaaaaagggtggagccaagaaaagacccgcccccagtgacgcagatataagtgagcccaaacgggtgcgcgagtcagttgcgcagccatcgacgtcagacgcggaagcttcgatcaactacgcagacaggtaccaaaacaaatgttctcgtcacgtgggcatgaatctgatgctgtttccctgcagacaatgcgagagaatgaatcagaattcaaatatctgcttcactcacggacagaaagactgtttagagtgctttcccgtgtcagaatctcaacccgtttctgtcgtcaaaaaggcgtatcagaaactgtgctacattcatcatatcatgggaaaggtgccagacgcttgcactgcctgcgatctggtcaatgtggatttggatgactgcatctttgaacaataa

SEQ ID NO: 124 - DNA, 2214 bp, Adeno-associated dependoparvovirus A
  source 1..2214: mol_type = genomic DNA
atggctgccgatggttatcttccagattggctcgaggacaacctctctgagggcattcgcgagtggtgggcgctgaaacctggagccccgaagcccaaagccaaccagcaaaagcaggacgacggccggggtctggtgcttcctggctacaagtacctcggacccttcaacggactcgacaagggggagcccgtcaacgcggcggacgcagcggccctcgagcacgacaaggcctacgaccagcagctgcaggcgggtgacaatccgtacctgcggtataaccacgccgacgccgagtttcaggagcgtctgcaagaagatacgtcttttgggggcaacctcgggcgagcagtcttccaggccaagaagcgggttctcgaacctctcggtctggttgaggaaggcgctaagacggctcctggaaagaagagaccggtagagccatcaccccagcgttctccagactcctctacgggcatcggcaagaaaggccaacagcccgccagaaaaagactcaattttggtcagactggcgactcagagtcagttccagaccctcaacctctcggagaacctccagcagcgccctctggtgtgggacctaatacaatggctgcaggcggtggcgcaccaatggcagacaataacgaaggcgccgacggagtgggtagttcctcgggaaattggcattgcgattccacatggctgggcgacagagtcatcaccaccagcacccgaacctgggccctgcccacctacaacaaccacctctacaagcaaatctccaacgggacatcgggaggagccaccaacgacaacacctacttcggctacagcaccccctgggggtattttgactttaacagattccactgccacttttcaccacgtgactggcagcgactcatcaacaacaactggggattccggcccaagagactcagcttcaagctcttcaacatccaggtcaaggaggtcacgcagaatgaaggcaccaagaccatcgccaataacctcaccagcaccatccaggtgtttacggactcggagtaccagctgccgtacgttctcggctctgcccaccagggctgcctgcctccgttcccggcggacgtgttcatgattccccagtacggctacctaacactcaacaacggtagtcaggccgtgggacgctcctccttctactgcctggaatactttccttcgcagatgctgagaaccggcaacaacttccagtttacttacaccttcgaggacgtgcctttccacagcagctacgcccacagccagagcttggaccggctgatgaatcctctgattgaccagtacctgtactacttgtctcggactcaaacaacaggaggcacggcaaatacgcagactctgggcttcagccaaggtgggcctaatacaatggccaatcaggcaaagaactggctgccaggaccctgttaccgccaacaacgcgtctcaacgacaaccgggcaaaacaacaatagcaactttgcctggactgctgggaccaaataccatctgaatggaagaaattcattggctaatcctggcatcgctatggcaacacacaaagacgacgaggagcgtttttttcccagtaacgggatcctgatttttggcaaacaaaatgctgccagagacaatgcggattacagcgatgtcatgctcaccagcgaggaagaaatcaaaaccactaaccctgtggctacagaggaatacggtatcgtggcagataacttgcagcagcaaaacacggctcctcaaattggaactgtcaacagccagggggccttacccggtatggtctggcagaaccgggacgtgtacctgcagggtcccatctgggccaagattcctcacacggacggcaacttccacccgtctccgctgatgggcggctttggcctgaaacatcctccgcctcagatcctgatcaagaacacgcctgtacctgcggatcctccgaccaccttcaaccagtcaaagctgaactctttcatcacgcaatacagcaccggacaggtcagcgtggaaattgaatgggagctgcagaaggaaaacagcaagcgctggaaccccgagatccagtacacctccaactactacaaatctacaagtgtggactttgctgttaatacagaaggcgtgtactctgaaccccgccccattggcacccgttacctcacccgtaatctg

SEQ ID NO: 125 - protein, 584 aa, synthetic construct
EAHKSEIAHRYNDLGEQHFKGLVLIAFSQYLQKCSYDEHAKLVQEVTDFAKTCVADESAANCDKSLHTLFGDKLCAIPNLRENYGELADCCTKQEPERNECFLQHKDDNPSLPPFERPEAEAMCTSFKENPTTFMGHYLHEVARRHPYFYAPELLYYAEQYNEILTQCCAEADKESCLTPKLDGVKEKALVSSVRQRMKCSSMQKFGERAFKAWAVARLSQTFPNADFAEITKLATDLTKVNKECCHGDLLECADDRAELAKYMCENQATISSKLQTCCDKPLLKKAHCLSEVEHDTMPADLPAIAADFVEDQEVCKNYTEAKDVFLGTFLYEYSRRHPDYSVSLLLRLAKKYEATLEKCCAEANPPACYGTVLAEFQPLVEEPKNLVKTNCDLYEKLGEYGFQNAILVRYTQKAPQVSTPTLVEAARNLGRVGTKCCTLPEDQRLPCVEDYLSAILNRVCLLHEKTPVSEHVTKCCSGSLVERRPCFSALTVDETYVPKEFKAETFTFHSDICTLPEKEKQIKKQTALAELVKHKPKATAEQLKTVMDDFAQFLDTCCKAADKDTCFSTEGPNLVTRCKDALA

SEQ ID NO: 126 - protein, 160 aa, Mus musculus
SRGQYSREDNNCTHFPVGQSHMLLELRTAFSQVKTFFQTKDQLDNILLTDSLMQDFKGYLGCQALSEMIQFYLVEVMPQAEKHGPEIKEHLNSLGEKLKTLRMRLRRCHRFLPCENKSKAVEQVKSDFNKLQDQGVYKAMNEFDIFINCIEAYMMIKMKS

SEQ ID NO: 127 - DNA, 560 bp, synthetic construct
  source 1..560: mol_type = other DNA
acgcgtgccgccaccatgcccggttccgctctgctgtgctgtttactgctgctgaccggaatgcggatttctcgtggccaatacagccgggaagataacaactgcacccatttccccgttggccagagccacatgttattagagctgcggaccgccttttcccaagtgaagaccttcttccagaccaaagaccagctcgacaacattctgctgaccgactccctcatgcaagatttcaagggctatttaggatgccaagctttatccgagatgatccagttttacctcgtggaggtgatgccccaagctgagaagcacggccccgaaatcaaggagcatttaaattctttaggagaaaagctgaagaccctccggatgaggttacgtaggtgccatcgttttttaccttgcgaaaacaagagcaaggccgtggagcaagtgaagagcgacttcaataagctgcaagatcaaggtgtgtataaggccatgaatgagtttgacatctttatcaactgcattgaagcctacatgatgattaaaatgaagagctaagcggccgc

SEQ ID NO: 128 - protein, 744 aa, synthetic construct
SRGQYSREDNNCTHFPVGQSHMLLELRTAFSQVKTFFQTKDQLDNILLTDSLMQDFKGYLGCQALSEMIQFYLVEVMPQAEKHGPEIKEHLNSLGEKLKTLRMRLRRCHRFLPCENKSKAVEQVKSDFNKLQDQGVYKAMNEFDIFINCIEAYMMIKMKSEAHKSEIAHRYNDLGEQHFKGLVLIAFSQYLQKCSYDEHAKLVQEVTDFAKTCVADESAANCDKSLHTLFGDKLCAIPNLRENYGELADCCTKQEPERNECFLQHKDDNPSLPPFERPEAEAMCTSFKENPTTFMGHYLHEVARRHPYFYAPELLYYAEQYNEILTQCCAEADKESCLTPKLDGVKEKALVSSVRQRMKCSSMQKFGERAFKAWAVARLSQTFPNADFAEITKLATDLTKVNKECCHGDLLECADDRAELAKYMCENQATISSKLQTCCDKPLLKKAHCLSEVEHDTMPADLPAIAADFVEDQEVCKNYTEAKDVFLGTFLYEYSRRHPDYSVSLLLRLAKKYEATLEKCCAEANPPACYGTVLAEFQPLVEEPKNLVKTNCDLYEKLGEYGFQNAILVRYTQKAPQVSTPTLVEAARNLGRVGTKCCTLPEDQRLPCVEDYLSAILNRVCLLHEKTPVSEHVTKCCSGSLVERRPCFSALTVDETYVPKEFKAETFTFHSDICTLPEKEKQIKKQTALAELVKHKPKATAEQLKTVMDDFAQFLDTCCKAADKDTCFSTEGPNLVTRCKDALA

SEQ ID NO: 129 - DNA, 2312 bp, synthetic construct
  source 1..2312: mol_type = other DNA
acgcgtgccgccaccatgcccggttccgctctgctgtgctgtttactgctgctgaccggaatgcggatttctcgtggccaatacagccgggaagataacaactgcacccatttccccgttggccagagccacatgttattagagctgcggaccgccttttcccaagtgaagaccttcttccagaccaaagaccagctcgacaacattctgctgaccgactccctcatgcaagatttcaagggctatttaggatgccaagctttatccgagatgatccagttttacctcgtggaggtgatgccccaagctgagaagcacggccccgaaatcaaggagcatttaaattctttaggagaaaagctgaagaccctccggatgaggttacgtaggtgccatcgttttttaccttgcgaaaacaagagcaaggccgtggagcaagtgaagagcgacttcaataagctgcaagatcaaggtgtgtataaggccatgaatgagtttgacatctttatcaactgcattgaagcctacatgatgattaaaatgaagagcgaggcccataagtccgagatcgcccaccggtacaacgatttaggcgagcaacatttcaagggactggtgctcatcgccttctcccagtatctgcagaaatgctcctatgacgagcacgccaagctcgtccaagaagtgacagacttcgctaagacttgtgtcgctgacgagagcgccgccaattgcgacaaatctttacatactttattcggcgataaactctgcgccatccccaatctgcgggagaactacggagagctcgccgactgctgtaccaagcaagaacccgaacggaacgagtgtttcctccagcacaaggatgacaacccttctttacctccttttgagcggcccgaagccgaggccatgtgcacaagcttcaaggagaaccccacaacctttatgggccactatctgcacgaggtggcccggaggcacccttatttctacgcccccgagctgctgtactacgctgagcagtacaacgagattttaacacagtgttgtgctgaagccgacaaggagagctgtctgacacccaagctcgacggagtcaaggagaaggccctcgtgagctccgtgaggcagcggatgaaatgcagctccatgcagaagttcggagaaagggccttcaaggcttgggccgtggctaggctgagccagacattccccaatgctgacttcgccgagattacaaaactggccaccgatttaaccaaggtcaacaaagaatgctgccacggagatttactggaatgcgccgatgatcgggccgagctggccaaatatatgtgcgagaaccaagctaccatctccagcaagctccaaacatgctgcgacaaacctttactcaagaaggcccactgcctctccgaagtggagcacgacaccatgcccgccgatctccccgctatcgctgccgatttcgtggaggaccaagaagtgtgcaagaattataccgaagctaaggatgtctttctgggcacatttctgtacgagtattctcgtaggcaccccgactatagcgtgtctttactgctccggctcgccaaaaagtatgaggccacactggagaaatgctgtgccgaagccaaccctcccgcttgctacggcaccgtgctcgccgagttccagcccctcgtggaggagcctaaaaatttagtgaagaccaactgtgatttatacgagaaactgggagagtacggattccagaacgccattttagtccggtacacacagaaggctccccaagtttccacacccacactggtcgaggccgctcgtaatctgggtcgtgtgggaacaaagtgttgtaccctccccgaagaccagaggctgccttgtgtggaggactatttaagcgccattctgaatcgggtctgtttactgcacgagaagacccccgtttccgagcacgtgacaaagtgttgctccggaagcctcgtggagaggaggccttgtttcagcgctttaaccgtcgacgaaacatatgtccccaaggagtttaaggccgagaccttcaccttccacagcgacatctgcactttacccgagaaagagaaacaaatcaagaagcagaccgctttagctgagctggtgaaacataagcccaaggccaccgccgagcagctgaaaaccgtgatggacgactttgcccagtttctcgacacttgttgtaaagccgccgacaaggacacttgtttctccaccgagggccccaatttagtgacaaggtgcaaagacgctttagcttaagcggccgc

SEQ ID NO: 130 - protein, 744 aa, synthetic construct
EAHKSEIAHRYNDLGEQHFKGLVLIAFSQYLQKCSYDEHAKLVQEVTDFAKTCVADESAANCDKSLHTLFGDKLCAIPNLRENYGELADCCTKQEPERNECFLQHKDDNPSLPPFERPEAEAMCTSFKENPTTFMGHYLHEVARRHPYFYAPELLYYAEQYNEILTQCCAEADKESCLTPKLDGVKEKALVSSVRQRMKCSSMQKFGERAFKAWAVARLSQTFPNADFAEITKLATDLTKVNKECCHGDLLECADDRAELAKYMCENQATISSKLQTCCDKPLLKKAHCLSEVEHDTMPADLPAIAADFVEDQEVCKNYTEAKDVFLGTFLYEYSRRHPDYSVSLLLRLAKKYEATLEKCCAEANPPACYGTVLAEFQPLVEEPKNLVKTNCDLYEKLGEYGFQNAILVRYTQKAPQVSTPTLVEAARNLGRVGTKCCTLPEDQRLPCVEDYLSAILNRVCLLHEKTPVSEHVTKCCSGSLVERRPCFSALTVDETYVPKEFKAETFTFHSDICTLPEKEKQIKKQTALAELVKHKPKATAEQLKTVMDDFAQFLDTCCKAADKDTCFSTEGPNLVTRCKDALASRGQYSREDNNCTHFPVGQSHMLLELRTAFSQVKTFFQTKDQLDNILLTDSLMQDFKGYLGCQALSEMIQFYLVEVMPQAEKHGPEIKEHLNSLGEKLKTLRMRLRRCHRFLPCENKSKAVEQVKSDFNKLQDQGVYKAMNEFDIFINCIEAYMMIKMKS

SEQ ID NO: 131 - DNA, 2330 bp, synthetic construct
  source 1..2330: mol_type = other DNA
acgcgtgccgccaccatgaaatgggtgaccttcctcttattactgtttgtcagcggcagcgccttttctcgtggagtgttccggagggaggctcacaagagcgaaatcgctcatcgttacaacgatttaggcgagcagcacttcaagggtttagttttaatcgctttctcccagtacctccagaagtgctcctacgacgagcatgccaagctcgtgcaagaggtgaccgactttgctaagacttgtgtggccgatgagtccgccgctaactgcgataagtctttacacaccctctttggagacaaactgtgcgccatccctaatctgcgggagaactacggcgagctggccgattgctgcacaaagcaagaacccgaaaggaacgagtgtttcctccagcacaaagacgacaacccttctttacctccctttgagaggcccgaggccgaggctatgtgtacctccttcaaggaaaaccccacaacattcatgggacattatttacatgaggtcgctcggcggcacccttacttctacgcccccgagctgctgtattacgccgagcagtacaacgagattctgacccagtgttgtgccgaagctgataaagagagctgtttaacacccaagctggatggcgtgaaggaaaaggctttagtcagcagcgtgaggcagaggatgaaatgctcctccatgcaaaagttcggcgaacgggcctttaaggcttgggctgtggctcgtctgagccagacattccccaacgccgacttcgccgagattaccaaactcgccaccgatctgacaaaggtcaacaaggagtgctgccatggtgatttactggagtgcgccgacgatagggccgaactcgctaaatacatgtgcgagaaccaagctaccatctccagcaagctgcagacttgttgtgataaacccctcctcaagaaggctcactgtttatccgaggtcgagcacgacacaatgcccgctgatctgcccgctatcgccgctgattttgtggaagaccaagaagtctgtaagaattacacagaggctaaggatgtgtttctcggcacctttttatacgaatatagccggaggcaccccgattatagcgtcagcctcttattacggctggctaagaagtatgaggccacactggaaaagtgctgtgccgaggctaaccctcccgcttgttacggaaccgtgctggctgaatttcagcctttagtcgaggagcccaagaatctggtgaagaccaactgtgatctgtacgaaaagctgggcgagtatggcttccaaaacgccattttagtgcggtatacacagaaggccccccaagtttccacccccacactggtcgaagctgcccggaatctgggacgggtgggcaccaagtgttgcactttacccgaggaccagaggctgccttgcgtggaggactacctcagcgctatcctcaatcgtgtctgtttactgcacgaaaagacacccgttagcgaacacgtgacaaagtgctgctccggctctttagtggaacggaggccttgctttagcgctttaacagtggacgaaacctacgtgcctaaggagtttaaggccgagaccttcacctttcactccgacatctgcactttacccgaaaaagagaagcagatcaaaaagcagaccgccctcgccgagctcgtcaaacataagcctaaggctaccgccgaacagctcaaaaccgtgatggacgacttcgcccaatttttagatacatgctgcaaggccgccgacaaggacacttgtttttccaccgagggccccaatttagtcactcgttgcaaggatgctttagcttctcgtggccagtactctcgtgaggacaataactgcacacattttcccgtgggccagagccatatgctgctcgagttacgtacagccttctcccaagttaagacattctttcagacaaaggaccagctggataacattctgctgacagacagcctcatgcaagatttcaaaggatatttaggatgccaagctctcagcgagatgatccagttctatttagtcgaagtgatgcctcaagctgaaaagcacggccccgagattaaggagcatctcaactctttaggcgagaagctgaagacactccggatgcggctgaggcggtgtcataggtttttaccttgtgagaataagagcaaagccgtggagcaagttaagtccgatttcaacaagctgcaagatcaaggcgtctataaggccatgaacgagtttgacatttttatcaattgcattgaggcctacatgatgatcaaaatgaagagctaagcggccgc

SEQ ID NO: 132 - protein, 127 aa, synthetic construct
HSDPARRGELSVCDSISEWVTAADKKTAVDMSGGTVTVLEKVPVSKGQLKQYFYETKCNPMGYTKEGCRGIDKRHWNSQCRTTQSYVRALTMDSKKRIGWRFIRIDTSCVCTLTIKRGRGSHHHHHH

SEQ ID NO: 133 - DNA, 794 bp, synthetic construct
  source 1..794: mol_type = other DNA
acgcgtgccgccaccatgacaattctgttcctcacaatggtgatcagctacttcggctgcatgaaggccgcccctatgaaggaggctaacatcagaggacaaggcggactcgcctatcccggcgtgaggactcacggcactctggaaagcgtgaatggccctaaggccggaagcagaggactcacatctctggctgacacattcgagcacgtgatcgaagagctgctggatgaggatcagaaggtgaggcctaacgaggagaacaacaaggacgccgatctgtacacatctagggtcatgctgtccagccaagtgccactggagcctcctctcctctttctgctggaggagtacaagaactatctggacgccgccaacatgtccatgagagtgagaaggcacagcgacccagccagaagaggcgagctgagcgtctgcgatagcatctccgaatgggtgactgctgccgataagaagacagccgtcgatatgagcggcggcacagtgacagtgctggaaaaagtcccagtcagcaagggccagctgaagcagtacttctacgagactaagtgcaaccctatgggctacacaaaggaaggctgtaggggcatcgacaaaaggcactggaactcccagtgtaggactactcagagctatgtgagggccctcactatggacagcaagaagaggatcggctggaggtttattaggattgacacaagctgcgtgtgcacactgacaatcaagaggggcagaggatcccatcaccatcaccatcactaataagcggccgc

SEQ ID NO: 134 - protein, 128 aa, synthetic construct
SSSHPIFHRGEFSVCDSVSVWVGDKTTATDIKGKEVMVLGEVNINNSVFKQYFFETKCRDPNPVDSGCRGIDSKHWNSYCTTTHTFVKALTMDGKQAAWRFIRIDTACVCVLSRKAVRRAGSHHHHHH

SEQ ID NO: 135 - DNA, 776 bp, synthetic construct
  source 1..776: mol_type = other DNA
acgcgtgccgccaccatgagcatgctgttctacacactgatcactgcctttctgatcggcatccaagccgagcctcatagcgagagcaatgtgccagccggccacacaatcccacaagcccactggactaagctgcaacatagcctcgacacagctctgaggagagctaggtccgctccagccgctgctatcgctgctagagtggccggccagacaagaaacatcactgtggaccctaggctcttcaagaagagaaggctgaggtccccaagagtgctcttcagcacacagcctccaagggaggccgctgatacacaagatttggacttcgaggtgggaggcgctgcccctttcaataggactcataggtccaagaggagcagctcccacccaattttccacagaggcgagttcagcgtgtgcgattccgtgtccgtctgggtgggcgacaaaactactgccactgacatcaagggcaaagaggtgatggtgctcggcgaggtgaacattaacaacagcgtgttcaagcagtatttcttcgagacaaagtgtagggacccaaacccagtggatagcggctgtaggggcatcgactccaagcactggaacagctactgcacaactactcacactttcgtcaaggctctgacaatggatggcaagcaagccgcttggaggttcatcagaatcgacacagcttgtgtgtgcgtgctgtctaggaaggccgtgaggagggctggatcccatcaccatcaccatcactaataagcggccgc

SEQ ID NO: 136 - protein, 138 aa, synthetic construct
GVSETAPASRRGELAVCDAVSGWVTDRRTAVDLRGREVEVLGEVPAAGGSPLRQYFFETRCKADNAEEGGPGAGGGGCRGVDRRHWVSECKAKQSYVRALTADAQGRVGWRWIRIDTACVCTLLSRTGRAGSHHHHHH

SEQ ID NO: 137 - DNA, 683 bp, synthetic construct
  source 1..683: mol_type = other DNA
acgcgtgccgccaccatgctgccactgccaagctgttctctgcctattctgctgctgtttctgctcccaagcgtgcctatcgagtcccagcctccaccttccacactgcctccatttctggccccagagtgggatctgctgagcccaagggtggtgctcagcagaggcgctccagccggacctccactgctgtttctgctggaagctggcgcctttagagaaagcgccggagctccagccaataggtctaggaggggcgtgtccgagactgctccagccagcagaagaggcgaactggctgtgtgcgatgccgtgagcggctgggtcacagataggaggactgccgtggatctgagaggaagggaggtggaggtgctgggagaagtgccagctgccggaggcagccctctgaggcagtacttcttcgagacaaggtgcaaggccgacaatgccgaagaaggaggccccggcgctggaggcggaggatgtagaggcgtggataggagacattgggtgagcgagtgtaaggccaagcagagctatgtgagagctctgactgctgatgctcaaggcagagtgggatggaggtggatcagaatcgacactgcttgtgtctgcacactgctgtctaggactggcagagctggatcccatcaccatcaccatcactaataagcggccgc

SEQ ID NO: 138 - protein, 127 aa, synthetic construct
YAEHKSHRGEYSVCDSESLWVTDKSSAIDIRGHQVTVLGEIKTGNSPVKQYFYETRCKEARPVKNGCRGIDDKHWNSQCKTSQTYVRALTSENNKLVGWRWIRIDTSCVCALSRKIGRTGSHHHHHH

SEQ ID NO: 139 - DNA, 824 bp, synthetic construct
  source 1..824: mol_type = other DNA
acgcgtgccgccaccatgtccattctgttctacgtcatctttctggcctatctgaggggcatccaaggcaataacatggaccagaggtctctgccagaggactctctgaactctctgatcatcaagctgatccaagccgatattctgaagaacaagctgagcaaacagatggtggacgtcaaggagaactaccagagcacactcccaaaggctgaggcccctagggaaccagaaagaggcggcccagccaaaagcgccttccagccagtgattgctatggacactgagctcctcagacagcagagaaggtacaactccccaagggtgctgctgagcgacagcactcctctggagcctccaccactgtacctcatggaggattacgtgggcagcccagtggtggccaataggacttctaggaggaagaggtacgctgaacacaagagccataggggagagtacagcgtctgcgattccgagagcctctgggtgactgacaagtcctccgctatcgatattaggggccaccaagtgacagtgctcggcgaaatcaagactggcaactccccagtgaagcagtacttctacgagacaaggtgcaaggaggctaggccagtgaagaacggctgtaggggaattgacgacaagcactggaacagccagtgcaagactagccagacatatgtgagggccctcactagcgagaacaacaagctcgtgggctggagatggattaggatcgacacaagctgtgtctgcgctctgtctaggaagatcggaaggactggatcccatcaccatcaccatcactaataagcggccgc

SEQ ID NO: 140 - protein, 593 aa, synthetic construct
DAHKSEVAHRFKDLGEENFKALVLIAFAQYLQQCPFEDHVKLVNEVTEFAKTCVADESAENCDKSLHTLFGDKLCTVATLRETYGEMADCCAKQEPERNECFLQHKDDNPNLPRLVRPEVDVMCTAFHDNEETFLKKYLYEIARRHPYFYAPELLFFAKRYKAAFTECCQAADKAACLLPKLDELRDEGKASSAKQGLKCASLQKFGERAFKAWAVARLSQRFPKAEFAEVSKLVTDLTKVHTECCHGDLLECADDRADLAKYICENQDSISSKLKECCEKPLLEKSHCIAEVENDEMPADLPSLAADFVGSKDVCKNYAEAKDVFLGMFLYEYARRHPDYSVVLLLRLAKTYETTLEKCCAAADPHECYAKVFDEFKPLVEEPQNLIKQNCELFEQLGEYKFQNALLVRYTKKVPQVSTPTLVEVSRNLGKVGSKCCKHPEAKRMPCAEDCLSVFLNQLCVLHEKTPVSDRVTKCCTESLVNGRPCFSALEVDETYVPKEFNAETFTFHADICTLSEKERQIKKQTALVELVKHKPKATKEQLKAVMDDFAAFVEKCCKADDKETCFAEEGKKLVAASQAALGLGSHHHHHH

SEQ ID NO: 141 - DNA, 1880 bp, synthetic construct
  source 1..1880: mol_type = other DNA
acgcgtgccgccaccatgaagtgggtgactttcatctctctgctgttcctcttcagcagcgcctacagcagaggcgtgttcagaagggatgcccacaagagcgaggtcgcccatagattcaaggatctgggcgaggagaacttcaaggctctcgtgctcatcgctttcgcccagtatctgcagcagtgccctttcgaagaccatgtgaagctggtgaacgaggtgacagagttcgccaagacatgtgtggccgatgagagcgccgagaactgcgacaagtctctgcacacactgttcggagataagctgtgcacagtcgctactctgagggagacttacggcgaaatggccgactgttgtgccaagcaagagccagagaggaatgagtgcttcctccagcacaaggacgacaaccctaatctgcctagactcgtgaggccagaagtggatgtgatgtgcacagctttccacgacaacgaggagactttcctcaagaagtacctctacgagatcgctaggagacacccttacttctatgccccagagctgctcttcttcgccaagaggtataaagccgctttcacagagtgctgtcaagccgccgacaaagctgcttgtctgctgcctaagctggatgagctgagggatgagggcaaggcctctagcgccaaacaaggcctcaaatgcgcttccctccagaagttcggagagagggcctttaaggcttgggccgtcgctaggctcagccaaagattcccaaaggccgagttcgctgaggtgagcaagctggtcacagacctcactaaggtgcacactgagtgctgtcacggcgatctgctcgaatgtgccgacgacagagctgacctcgccaaatacatctgcgagaatcaagattccatcagctccaagctcaaggagtgctgtgagaagccactgctcgagaagagccattgcatcgccgaggtcgagaacgatgagatgccagccgatctgccttctctggctgccgatttcgtgggctccaaagacgtctgcaagaactacgccgaggctaaggacgtctttctgggcatgtttctgtacgagtatgctaggagacatccagattactccgtggtgctgctgctgagactggccaagacttacgagacaacactggaaaagtgctgcgccgctgctgacccacacgagtgctacgccaaggtgtttgacgagttcaagcctctcgtcgaggagccacagaatctgattaagcagaactgtgaactcttcgagcagctgggcgagtacaagttccaaaatgctctgctggtgaggtacactaagaaggtgcctcaagtgtccactcctacactggtggaggtgagcagaaatctcggcaaggtcggcagcaaatgttgcaagcacccagaggccaagagaatgccttgtgctgaggactgtctgagcgtgtttctgaaccagctctgtgtgctgcacgagaagacaccagtcagcgacagagtgactaagtgctgcacagagtctctggtgaacggaaggccatgtttctccgctctggaggtcgacgagacttacgtgcctaaggagttcaacgccgagactttcacattccacgccgacatctgcactctctccgaaaaggaaaggcagatcaagaagcagacagctctggtggagctggtcaagcacaagccaaaggccacaaaggaacagctcaaggctgtcatggacgacttcgccgccttcgtcgagaagtgttgcaaagccgacgacaaggagacatgcttcgccgaggagggcaaaaaactggtcgctgccagccaagccgctctcggcctcggatcccatcaccatcaccatcactaataagcggccgc

SEQ ID NO: 142 - DNA, 32 bp, synthetic construct
  source 1..32: mol_type = other DNA
tttttagatctgatgcccacaagagcgaggtc

SEQ ID NO: 143 - DNA, 32 bp, synthetic construct
  source 1..32: mol_type = other DNA
tttttagatctgcccctatgaaggaggctaac

SEQ ID NO: 144 - DNA, 33 bp, synthetic construct
  source 1..33: mol_type = other DNA
ttgttagatctgagcctcatagcgagagcaatg

SEQ ID NO: 145 - DNA, 30 bp, synthetic construct
  source 1..30: mol_type = other DNA
ttgttagatctcagcctccaccttccacac

SEQ ID NO: 146 - DNA, 33 bp, synthetic construct
  source 1..33: mol_type = other DNA
ttgttagatctaataacatggaccagaggtctc

SEQ ID NO: 147 - DNA, 33 bp, synthetic construct
  source 1..33: mol_type = other DNA
ttctgtctttgcggccgcttattagtgatggtg

SEQ ID NO: 148 - protein, 714 aa, synthetic construct
HSDPARRGELSVCDSISEWVTAADKKTAVDMSGGTVTVLEKVPVSKGQLKQYFYETKCNPMGYTKEGCRGIDKRHWNSQCRTTQSYVRALTMDSKKRIGWRFIRIDTSCVCTLTIKRGRGSDAHKSEVAHRFKDLGEENFKALVLIAFAQYLQQCPFEDHVKLVNEVTEFAKTCVADESAENCDKSLHTLFGDKLCTVATLRETYGEMADCCAKQEPERNECFLQHKDDNPNLPRLVRPEVDVMCTAFHDNEETFLKKYLYEIARRHPYFYAPELLFFAKRYKAAFTECCQAADKAACLLPKLDELRDEGKASSAKQGLKCASLQKFGERAFKAWAVARLSQRFPKAEFAEVSKLVTDLTKVHTECCHGDLLECADDRADLAKYICENQDSISSKLKECCEKPLLEKSHCIAEVENDEMPADLPSLAADFVGSKDVCKNYAEAKDVFLGMFLYEYARRHPDYSVVLLLRLAKTYETTLEKCCAAADPHECYAKVFDEFKPLVEEPQNLIKQNCELFEQLGEYKFQNALLVRYTKKVPQVSTPTLVEVSRNLGKVGSKCCKHPEAKRMPCAEDCLSVFLNQLCVLHEKTPVSDRVTKCCTESLVNGRPCFSALEVDETYVPKEFNAETFTFHADICTLSEKERQIKKQTALVELVKHKPKATKEQLKAVMDDFAAFVEKCCKADDKETCFAEEGKKLVAASQAALGLGSHHHHHH

SEQ ID NO: 149 - protein, 715 aa, synthetic construct
SSSHPIFHRGEFSVCDSVSVWVGDKTTATDIKGKEVMVLGEVNINNSVFKQYFFETKCRDPNPVDSGCRGIDSKHWNSYCTTTHTFVKALTMDGKQAAWRFIRIDTACVCVLSRKAVRRAGSDAHKSEVAHRFKDLGEENFKALVLIAFAQYLQQCPFEDHVKLVNEVTEFAKTCVADESAENCDKSLHTLFGDKLCTVATLRETYGEMADCCAKQEPERNECFLQHKDDNPNLPRLVRPEVDVMCTAFHDNEETFLKKYLYEIARRHPYFYAPELLFFAKRYKAAFTECCQAADKAACLLPKLDELRDEGKASSAKQGLKCASLQKFGERAFKAWAVARLSQRFPKAEFAEVSKLVTDLTKVHTECCHGDLLECADDRADLAKYICENQDSISSKLKECCEKPLLEKSHCIAEVENDEMPADLPSLAADFVGSKDVCKNYAEAKDVFLGMFLYEYARRHPDYSVVLLLRLAKTYETTLEKCCAAADPHECYAKVFDEFKPLVEEPQNLIKQNCELFEQLGEYKFQNALLVRYTKKVPQVSTPTLVEVSRNLGKVGSKCCKHPEAKRMPCAEDCLSVFLNQLCVLHEKTPVSDRVTKCCTESLVNGRPCFSALEVDETYVPKEFNAETFTFHADICTLSEKERQIKKQTALVELVKHKPKATKEQLKAVMDDFAAFVEKCCKADDKETCFAEEGKKLVAASQAALGLGSHHHHHH

SEQ ID NO: 150 - protein, 725 aa, synthetic construct
GVSETAPASRRGELAVCDAVSGWVTDRRTAVDLRGREVEVLGEVPAAGGSPLRQYFFETRCKADNAEEGGPGAGGGGCRGVDRRHWVSECKAKQSYVRALTADAQGRVGWRWIRIDTACVCTLLSRTGRAGSDAHKSEVAHRFKDLGEENFKALVLIAFAQYLQQCPFEDHVKLVNEVTEFAKTCVADESAENCDKSLHTLFGDKLCTVATLRETYGEMADCCAKQEPERNECFLQHKDDNPNLPRLVRPEVDVMCTAFHDNEETFLKKYLYEIARRHPYFYAPELLFFAKRYKAAFTECCQAADKAACLLPKLDELRDEGKASSAKQGLKCASLQKFGERAFKAWAVARLSQRFPKAEFAEVSKLVTDLTKVHTECCHGDLLECADDRADLAKYICENQDSISSKLKECCEKPLLEKSHCIAEVENDEMPADLPSLAADFVGSKDVCKNYAEAKDVFLGMFLYEYARRHPDYSVVLLLRLAKTYETTLEKCCAAADPHECYAKVFDEFKPLVEEPQNLIKQNCELFEQLGEYKFQNALLVRYTKKVPQVSTPTLVEVSRNLGKVGSKCCKHPEAKRMPCAEDCLSVFLNQLCVLHEKTPVSDRVTKCCTESLVNGRPCFSALEVDETYVPKEFNAETFTFHADICTLSEKERQIKKQTALVELVKHKPKATKEQLKAVMDDFAAFVEKCCKADDKETCFAEEGKKLVAASQAALGLGSHHHHHH

SEQ ID NO: 151 - protein, 714 aa, synthetic construct
YAEHKSHRGEYSVCDSESLWVTDKSSAIDIRGHQVTVLGEIKTGNSPVKQYFYETRCKEARPVKNGCRGIDDKHWNSQCKTSQTYVRALTSENNKLVGWRWIRIDTSCVCALSRKIGRTGSDAHKSEVAHRFKDLGEENFKALVLIAFAQYLQQCPFEDHVKLVNEVTEFAKTCVADESAENCDKSLHTLFGDKLCTVATLRETYGEMADCCAKQEPERNECFLQHKDDNPNLPRLVRPEVDVMCTAFHDNEETFLKKYLYEIARRHPYFYAPELLFFAKRYKAAFTECCQAADKAACLLPKLDELRDEGKASSAKQGLKCASLQKFGERAFKAWAVARLSQRFPKAEFAEVSKLVTDLTKVHTECCHGDLLECADDRADLAKYICENQDSISSKLKECCEKPLLEKSHCIAEVENDEMPADLPSLAADFVGSKDVCKNYAEAKDVFLGMFLYEYARRHPDYSVVLLLRLAKTYETTLEKCCAAADPHECYAKVFDEFKPLVEEPQNLIKQNCELFEQLGEYKFQNALLVRYTKKVPQVSTPTLVEVSRNLGKVGSKCCKHPEAKRMPCAEDCLSVFLNQLCVLHEKTPVSDRVTKCCTESLVNGRPCFSALEVDETYVPKEFNAETFTFHADICTLSEKERQIKKQTALVELVKHKPKATKEQLKAVMDDFAAFVEKCCKADDKETCFAEEGKKLVAASQAALGLGSHHHHHH

SEQ ID NO: 152 - protein, 824 aa, synthetic construct
DAHKSEVAHRFKDLGEENFKALVLIAFAQYLQQCPFEDHVKLVNEVTEFAKTCVADESAENCDKSLHTLFGDKLCTVATLRETYGEMADCCAKQEPERNECFLQHKDDNPNLPRLVRPEVDVMCTAFHDNEETFLKKYLYEIARRHPYFYAPELLFFAKRYKAAFTECCQAADKAACLLPKLDELRDEGKASSAKQGLKCASLQKFGERAFKAWAVARLSQRFPKAEFAEVSKLVTDLTKVHTECCHGDLLECADDRADLAKYICENQDSISSKLKECCEKPLLEKSHCIAEVENDEMPADLPSLAADFVGSKDVCKNYAEAKDVFLGMFLYEYARRHPDYSVVLLLRLAKTYETTLEKCCAAADPHECYAKVFDEFKPLVEEPQNLIKQNCELFEQLGEYKFQNALLVRYTKKVPQVSTPTLVEVSRNLGKVGSKCCKHPEAKRMPCAEDCLSVFLNQLCVLHEKTPVSDRVTKCCTESLVNGRPCFSALEVDETYVPKEFNAETFTFHADICTLSEKERQIKKQTALVELVKHKPKATKEQLKAVMDDFAAFVEKCCKADDKETCFAEEGKKLVAASQAALGLGSAPMKEANIRGQGGLAYPGVRTHGTLESVNGPKAGSRGLTSLADTFEHVIEELLDEDQKVRPNEENNKDADLYTSRVMLSSQVPLEPPLLFLLEEYKNYLDAANMSMRVRRHSDPARRGELSVCDSISEWVTAADKKTAVDMSGGTVTVLEKVPVSKGQLKQYFYETKCNPMGYTKEGCRGIDKRHWNSQCRTTQSYVRALTMDSKKRIGWRFIRIDTSCVCTLTIKRGRGSHHHHHH

SEQ ID NO: 153 - protein, 818 aa, synthetic construct
DAHKSEVAHRFKDLGEENFKALVLIAFAQYLQQCPFEDHVKLVNEVTEFAKTCVADESAENCDKSLHTLFGDKLCTVATLRETYGEMADCCAKQEPERNECFLQHKDDNPNLPRLVRPEVDVMCTAFHDNEETFLKKYLYEIARRHPYFYAPELLFFAKRYKAAFTECCQAADKAACLLPKLDELRDEGKASSAKQGLKCASLQKFGERAFKAWAVARLSQRFPKAEFAEVSKLVTDLTKVHTECCHGDLLECADDRADLAKYICENQDSISSKLKECCEKPLLEKSHCIAEVENDEMPADLPSLAADFVGSKDVCKNYAEAKDVFLGMFLYEYARRHPDYSVVLLLRLAKTYETTLEKCCAAADPHECYAKVFDEFKPLVEEPQNLIKQNCELFEQLGEYKFQNALLVRYTKKVPQVSTPTLVEVSRNLGKVGSKCCKHPEAKRMPCAEDCLSVFLNQLCVLHEKTPVSDRVTKCCTESLVNGRPCFSALEVDETYVPKEFNAETFTFHADICTLSEKERQIKKQTALVELVKHKPKATKEQLKAVMDDFAAFVEKCCKADDKETCFAEEGKKLVAASQAALGLGSEPHSESNVPAGHTIPQAHWTKLQHSLDTALRRARSAPAAAIAARVAGQTRNITVDPRLFKKRRLRSPRVLFSTQPPREAADTQDLDFEVGGAAPFNRTHRSKRSSSHPIFHRGEFSVCDSVSVWVGDKTTATDIKGKEVMVLGEVNINNSVFKQYFFETKCRDPNPVDSGCRGIDSKHWNSYCTTTHTFVKALTMDGKQAAWRFIRIDTACVCVLSRKAVRRAGSHHHHHH

SEQ ID NO: 154 - protein, 780 aa, synthetic construct
DAHKSEVAHRFKDLGEENFKALVLIAFAQYLQQCPFEDHVKLVNEVTEFAKTCVADESAENCDKSLHTLFGDKLCTVATLRETYGEMADCCAKQEPERNECFLQHKDDNPNLPRLVRPEVDVMCTAFHDNEETFLKKYLYEIARRHPYFYAPELLFFAKRYKAAFTECCQAADKAACLLPKLDELRDEGKASSAKQGLKCASLQKFGERAFKAWAVARLSQRFPKAEFAEVSKLVTDLTKVHTECCHGDLLECADDRADLAKYICENQDSISSKLKECCEKPLLEKSHCIAEVENDEMPADLPSLAADFVGSKDVCKNYAEAKDVFLGMFLYEYARRHPDYSVVLLLRLAKTYETTLEKCCAAADPHECYAKVFDEFKPLVEEPQNLIKQNCELFEQLGEYKFQNALLVRYTKKVPQVSTPTLVEVSRNLGKVGSKCCKHPEAKRMPCAEDCLSVFLNQLCVLHEKTPVSDRVTKCCTESLVNGRPCFSALEVDETYVPKEFNAETFTFHADICTLSEKERQIKKQTALVELVKHKPKATKEQLKAVMDDFAAFVEKCCKADDKETCFAEEGKKLVAASQAALGLGSQPPPSTLPPFLAPEWDLLSPRVVLSRGAPAGPPLLFLLEAGAFRESAGAPANRSRRGVSETAPASRRGELAVCDAVSGWVTDRRTAVDLRGREVEVLGEVPAAGGSPLRQYFFETRCKADNAEEGGPGAGGGGCRGVDRRHWVSECKAKQSYVRALTADAQGRVGWRWIRIDTACVCTLLSRTGRAGSHHHHH

SEQ ID NO: 155 - protein, 834 aa, synthetic construct
DAHKSEVAHRFKDLGEENFKALVLIAFAQYLQQCPFEDHVKLVNEVTEFAKTCVADESAENCDKSLHTLFGDKLCTVATLRETYGEMADCCAKQEPERNECFLQHKDDNPNLPRLVRPEVDVMCTAFHDNEETFLKKYLYEIARRHPYFYAPELLFFAKRYKAAFTECCQAADKAACLLPKLDELRDEGKASSAKQGLKCASLQKFGERAFKAWAVARLSQRFPKAEFAEVSKLVTDLTKVHTECCHGDLLECADDRADLAKYICENQDSISSKLKECCEKPLLEKSHCIAEVENDEMPADLPSLAADFVGSKDVCKNYAEAKDVFLGMFLYEYARRHPDYSVVLLLRLAKTYETTLEKCCAAADPHECYAKVFDEFKPLVEEPQNLIKQNCELFEQLGEYKFQNALLVRYTKKVPQVSTPTLVEVSRNLGKVGSKCCKHPEAKRMPCAEDCLSVFLNQLCVLHEKTPVSDRVTKCCTESLVNGRPCFSALEVDETYVPKEFNAETFTFHADICTLSEKERQIKKQTALVELVKHKPKATKEQLKAVMDDFAAFVEKCCKADDKETCFAEEGKKLVAASQAALGLGSNNMDQRSLPEDSLNSLIIKLIQADILKNKLSKQMVDVKENYQSTLPKAEAPREPERGGPAKSAFQPVIAMDTELLRQQRRYNSPRVLLSDSTPLEPPPLYLMEDYVGSPVVANRTSRRKRYAEHKSHRGEYSVCDSESLWVTDKSSAIDIRGHQVTVLGEIKTGNSPVKQYFYETRCKEARPVKNGCRGIDDKHWNSQCKTSQTYVRALTSENNKLVGWRWIRIDTSCVCALSRKIGRTGSHHHHHH

SEQ ID NO: 156 - protein, 171 aa, synthetic construct
QGQEAGGRPGADCEVCKEFLNRFYKSLIDRGVNFSLDTIEKELISFCLDTKGKENRLCYYLGATKDAATKILSEVTRPMSVHMPAMKICEKLKKLDSQICELKYEKTLDLASVDLRKMRVAELKQILHSWGEECRACAEKTDYVNLIQELAPKYAATHPKTELGSHHHHHH

SEQ ID NO: 157 - DNA, 614 bp, synthetic construct
  source 1..614: mol_type = other DNA
acgcgtgccgccaccatgtggtgcgctagccctgtggccgtggtggccttctgcgccggcctcctggtatctcaccctgtgctgacacaaggccaagaggccggcggtagacctggcgccgactgcgaggtgtgcaaggagttcctgaacagattctacaagagcctgatcgacagaggcgtgaacttctccctggacaccatcgagaaggagctgatcagcttctgtctggacaccaagggcaaggagaacagactgtgctactacctgggcgccaccaaggacgccgccaccaagatcctgagcgaggtgacaagacctatgagcgtgcacatgcctgccatgaaaatctgcgagaagctgaagaagctggactctcaaatctgcgagctgaagtacgagaagaccctggacctggctagcgtggacctgagaaagatgagagtggccgagctgaagcagatcctgcacagctggggcgaggagtgcagagcctgcgccgagaagaccgactacgtgaacctgatccaagagctggcccctaagtacgccgccacccaccctaagaccgagctgggatcccatcaccatcaccatcactaataagcggccgc

SEQ ID NO: 158 - protein, 758 aa, synthetic construct
QGQEAGGRPGADCEVCKEFLNRFYKSLIDRGVNFSLDTIEKELISFCLDTKGKENRLCYYLGATKDAATKILSEVTRPMSVHMPAMKICEKLKKLDSQICELKYEKTLDLASVDLRKMRVAELKQILHSWGEECRACAEKTDYVNLIQELAPKYAATHPKTELGSDAHKSEVAHRFKDLGEENFKALVLIAFAQYLQQCPFEDHVKLVNEVTEFAKTCVADESAENCDKSLHTLFGDKLCTVATLRETYGEMADCCAKQEPERNECFLQHKDDNPNLPRLVRPEVDVMCTAFHDNEETFLKKYLYEIARRHPYFYAPELLFFAKRYKAAFTECCQAADKAACLLPKLDELRDEGKASSAKQGLKCASLQKFGERAFKAWAVARLSQRFPKAEFAEVSKLVTDLTKVHTECCHGDLLECADDRADLAKYICENQDSISSKLKECCEKPLLEKSHCIAEVENDEMPADLPSLAADFVGSKDVCKNYAEAKDVFLGMFLYEYARRHPDYSVVLLLRLAKTYETTLEKCCAAADPHECYAKVFDEFKPLVEEPQNLIKQNCELFEQLGEYKFQNALLVRYTKKVPQVSTPTLVEVSRNLGKVGSKCCKHPEAKRMPCAEDCLSVFLNQLCVLHEKTPVSDRVTKCCTESLVNGRPCFSALEVDETYVPKEFNAETFTFHADICTLSEKERQIKKQTALVELVKHKPKATKEQLKAVMDDFAAFVEKCCKADDKETCFAEEGKKLVAASQAALGLGSHHHHHH

SEQ ID NO: 159 - DNA, 2375 bp, synthetic construct
  source 1..2375: mol_type = other DNA
acgcgtgccgccaccatgtggtgcgctagccctgtggccgtggtggccttctgcgccggcctcctggtatctcaccctgtgctgacacaaggccaagaggccggcggtagacctggcgccgactgcgaggtgtgcaaggagttcctgaacagattctacaagagcctgatcgacagaggcgtgaacttctccctggacaccatcgagaaggagctgatcagcttctgtctggacaccaagggcaaggagaacagactgtgctactacctgggcgccaccaaggacgccgccaccaagatcctgagcgaggtgacaagacctatgagcgtgcacatgcctgccatgaaaatctgcgagaagctgaagaagctggactctcaaatctgcgagctgaagtacgagaagaccctggacctggctagcgtggacctgagaaagatgagagtggccgagctgaagcagatcctgcacagctggggcgaggagtgcagagcctgcgccgagaagaccgactacgtgaacctgatccaagagctggcccctaagtacgccgccacccaccctaagaccgagctgggatctgatgcccacaagagcgaggtcgcccatagattcaaggatctgggcgaggagaacttcaaggctctcgtgctcatcgctttcgcccagtatctgcagcagtgccctttcgaagaccatgtgaagctggtgaacgaggtgacagagttcgccaagacatgtgtggccgatgagagcgccgagaactgcgacaagtctctgcacacactgttcggagataagctgtgcacagtcgctactctgagggagacttacggcgaaatggccgactgttgtgccaagcaagagccagagaggaatgagtgcttcctccagcacaaggacgacaaccctaatctgcctagactcgtgaggccagaagtggatgtgatgtgcacagctttccacgacaacgaggagactttcctcaagaagtacctctacgagatcgctaggagacacccttacttctatgccccagagctgctcttcttcgccaagaggtataaagccgctttcacagagtgctgtcaagccgccgacaaagctgcttgtctgctgcctaagctggatgagctgagggatgagggcaaggcctctagcgccaaacaaggcctcaaatgcgcttccctccagaagttcggagagagggcctttaaggcttgggccgtcgctaggctcagccaaagattcccaaaggccgagttcgctgaggtgagcaagctggtcacagacctcactaaggtgcacactgagtgctgtcacggcgatctgctcgaatgtgccgacgacagagctgacctcgccaaatacatctgcgagaatcaagattccatcagctccaagctcaaggagtgctgtgagaagccactgctcgagaagagccattgcatcgccgaggtcgagaacgatgagatgccagccgatctgccttctctggctgccgatttcgtgggctccaaagacgtctgcaagaactacgccgaggctaaggacgtctttctgggcatgtttctgtacgagtatgctaggagacatccagattactccgtggtgctgctgctgagactggccaagacttacgagacaacactggaaaagtgctgcgccgctgctgacccacacgagtgctacgccaaggtgtttgacgagttcaagcctctcgtcgaggagccacagaatctgattaagcagaactgtgaactcttcgagcagctgggcgagtacaagttccaaaatgctctgctggtgaggtacactaagaaggtgcctcaagtgtccactcctacactggtggaggtgagcagaaatctcggcaaggtcggcagcaaatgttgcaagcacccagaggccaagagaatgccttgtgctgaggactgtctgagcgtgtttctgaaccagctctgtgtgctgcacgagaagacaccagtcagcgacagagtgactaagtgctgcacagagtctctggtgaacggaaggccatgtttctccgctctggaggtcgacgagacttacgtgcctaaggagttcaacgccgagactttcacattccacgccgacatctgcactctctccgaaaaggaaaggcagatcaagaagcagacagctctggtggagctggtcaagcacaagccaaaggccacaaaggaacagctcaaggctgtcatggacgacttcgccgccttcgtcgagaagtgttgcaaagccgacgacaaggagacatgcttcgccgaggagggcaaaaaactggtcgctgccagccaagccgctctcggcctcggatcccatcaccatcaccatcactgataagcggccgc

SEQ ID NO: 160 - protein, 758 aa, synthetic construct
DAHKSEVAHRFKDLGEENFKALVLIAFAQYLQQCPFEDHVKLVNEVTEFAKTCVADESAENCDKSLHTLFGDKLCTVATLRETYGEMADCCAKQEPERNECFLQHKDDNPNLPRLVRPEVDVMCTAFHDNEETFLKKYLYEIARRHPYFYAPELLFFAKRYKAAFTECCQAADKAACLLPKLDELRDEGKASSAKQGLKCASLQKFGERAFKAWAVARLSQRFPKAEFAEVSKLVTDLTKVHTECCHGDLLECADDRADLAKYICENQDSISSKLKECCEKPLLEKSHCIAEVENDEMPADLPSLAADFVGSKDVCKNYAEAKDVFLGMFLYEYARRHPDYSVVLLLRLAKTYETTLEKCCAAADPHECYAKVFDEFKPLVEEPQNLIKQNCELFEQLGEYKFQNALLVRYTKKVPQVSTPTLVEVSRNLGKVGSKCCKHPEAKRMPCAEDCLSVFLNQLCVLHEKTPVSDRVTKCCTESLVNGRPCFSALEVDETYVPKEFNAETFTFHADICTLSEKERQIKKQTALVELVKHKPKATKEQLKAVMDDFAAFVEKCCKADDKETCFAEEGKKLVAASQAALGLGSQGQEAGGRPGADCEVCKEFLNRFYKSLIDRGVNFSLDTIEKELISFCLDTKGKENRLCYYLGATKDAATKILSEVTRPMSVHMPAMKICEKLKKLDSQICELKYEKTLDLASVDLRKMRVAELKQILHSWGEECRACAEKTDYVNLIQELAPKYAATHPKTELGSHHHHHH

SEQ ID NO: 161 - DNA, 2375 bp, synthetic construct
  source 1..2375: mol_type = other DNA
acgcgtgccgccaccatgaagtgggtgactttcatctctctgctgttcctcttcagcagcgcctacagcagaggcgtgttcagaagggatgcccacaagagcgaggtcgcccatagattcaaggatctgggcgaggagaacttcaaggctctcgtgctcatcgctttcgcccagtatctgcagcagtgccctttcgaagaccatgtgaagctggtgaacgaggtgacagagttcgccaagacatgtgtggccgatgagagcgccgagaactgcgacaagtctctgcacacactgttcggagataagctgtgcacagtcgctactctgagggagacttacggcgaaatggccgactgttgtgccaagcaagagccagagaggaatgagtgcttcctccagcacaaggacgacaaccctaatctgcctagactcgtgaggccagaagtggatgtgatgtgcacagctttccacgacaacgaggagactttcctcaagaagtacctctacgagatcgctaggagacacccttacttctatgccccagagctgctcttcttcgccaagaggtataaagccgctttcacagagtgctgtcaagccgccgacaaagctgcttgtctgctgcctaagctggatgagctgagggatgagggcaaggcctctagcgccaaacaaggcctcaaatgcgcttccctccagaagttcggagagagggcctttaaggcttgggccgtcgctaggctcagccaaagattcccaaaggccgagttcgctgaggtgagcaagctggtcacagacctcactaaggtgcacactgagtgctgtcacggagatctgctcgaatgtgccgacgacagagctgacctcgccaaatacatctgcgagaatcaagattccatcagctccaagctcaaggagtgctgtgagaagccactgctcgagaagagccattgcatcgccgaggtcgagaacgatgagatgccagccgatctgccttctctggctgccgatttcgtgggctccaaagacgtctgcaagaactacgccgaggctaaggacgtctttctgggcatgtttctgtacgagtatgctaggagacatccagattactccgtggtgctgctgctgagactggccaagacttacgagacaacactggaaaagtgctgcgccgctgctgacccacacgagtgctacgccaaggtgtttgacgagttcaagcctctcgtcgaggagccacagaatctgattaagcagaactgtgaactcttcgagcagctgggcgagtacaagttccaaaatgctctgctggtgaggtacactaagaaggtgcctcaagtgtccactcctacactggtggaggtgagcagaaatctcggcaaggtcggcagcaaatgttgcaagcacccagaggccaagagaatgccttgtgctgaggactgtctgagcgtgtttctgaaccagctctgtgtgctgcacgagaagacaccagtcagcgacagagtgactaagtgctgcacagagtctctggtgaacggaaggccatgtttctccgctctggaggtcgacgagacttacgtgcctaaggagttcaacgccgagactttcacattccacgccgacatctgcactctctccgaaaaggaaaggcagatcaagaagcagacagctctggtggagctggtcaagcacaagccaaaggccacaaaggaacagctcaaggctgtcatggacgacttcgccgccttcgtcgagaagtgttgcaaagccgacgacaaggagacatgcttcgccgaggagggcaaaaaactggtcgctgccagccaagccgctctcggcctcggatctcaaggccaagaggccggcggtagacctggcgccgactgcgaggtgtgcaaggagttcctgaacagattctacaagagcctgatcgacagaggcgtgaacttctccctggacaccatcgagaaggagctgatcagcttctgtctggacaccaagggcaaggagaacagactgtgctactacctgggcgccaccaaggacgccgccaccaagatcctgagcgaggtgacaagacctatgagcgtgcacatgcctgccatgaaaatctgcgagaagctgaagaagctggactctcaaatctgcgagctgaagtacgagaagaccctggacctggctagcgtggacctgagaaagatgagagtggccgagctgaagcagatcctgcacagctggggcgaggagtgcagagcctgcgccgagaagaccgactacgtgaacctgatccaagagctggcccctaagtacgccgccacccaccctaagaccgagctgggatcccatcaccatcaccatcactaataagcggccgc

SEQ ID NO: 162 - protein, 142 aa, synthetic construct
SPDKQMAVLPRRERNRQAAAANPENSRGKGRRGQRGKNRGCVLTAIHLNVTDLGLGYETKEELIFRYCSGSCDAAETTYDKILKNLSRNRRLVSDKVGQACCRPIAFDDDLSFLDDNLVYHILRKHSAKRCGCIGSHHHHHH

SEQ ID NO: 163 - DNA, 730 bp, synthetic construct
  source 1..730: mol_type = other DNA
acgcgttctagagtgtcgtgaaaactacccctaaaagccaaagccgccaccatgaagctgtgggacgtggtggccgtgtgcctggtgctgctgcacaccgctagcgccttccctctgcctgccggcaagaggcctcctgaggcccctgccgaggacagaagcctgggcagaagaagagcccctttcgccctgagcagcgacagcaacatgcctgaggactaccctgatcagttcgacgacgtgatggacttcatccaagccaccatcaagagactgaagagaagccctgacaagcagatggccgtgctgcctagaagagagagaaacagacaagccgccgccgccaaccctgagaacagcagaggcaagggcagaagaggacagagaggcaagaacagaggctgcgtgctgaccgccatccacctgaacgtgaccgacctgggcctgggctacgagaccaaggaggagctgatcttcagatactgcagcggcagctgcgacgccgccgagaccacctacgacaagatcctgaagaacctgagcagaaacagaagactggtgagcgacaaggtgggccaagcctgctgcagacctatcgccttcgacgacgacctgagcttcctggacgacaacctggtgtaccacatcctgagaaagcacagcgccaagagatgcggctgcatcggatcccatcaccatcaccatcactaataaggcgcgccgcggccgc

SEQ ID NO: 164 - protein, 729 aa, synthetic construct
SPDKQMAVLPRRERNRQAAAANPENSRGKGRRGQRGKNRGCVLTAIHLNVTDLGLGYETKEELIFRYCSGSCDAAETTYDKILKNLSRNRRLVSDKVGQACCRPIAFDDDLSFLDDNLVYHILRKHSAKRCGCIGSDAHKSEVAHRFKDLGEENFKALVLIAFAQYLQQCPFEDHVKLVNEVTEFAKTCVADESAENCDKSLHTLFGDKLCTVATLRETYGEMADCCAKQEPERNECFLQHKDDNPNLPRLVRPEVDVMCTAFHDNEETFLKKYLYEIARRHPYFYAPELLFFAKRYKAAFTECCQAADKAACLLPKLDELRDEGKASSAKQGLKCASLQKFGERAFKAWAVARLSQRFPKAEFAEVSKLVTDLTKVHTECCHGDLLECADDRADLAKYICENQDSISSKLKECCEKPLLEKSHCIAEVENDEMPADLPSLAADFVGSKDVCKNYAEAKDVFLGMFLYEYARRHPDYSVVLLLRLAKTYETTLEKCCAAADPHECYAKVFDEFKPLVEEPQNLIKQNCELFEQLGEYKFQNALLVRYTKKVPQVSTPTLVEVSRNLGKVGSKCCKHPEAKRMPCAEDCLSVFLNQLCVLHEKTPVSDRVTKCCTESLVNGRPCFSALEVDETYVPKEFNAETFTFHADICTLSEKERQIKKQTALVELVKHKPKATKEQLKAVMDDFAAFVEKCCKADDKETCFAEEGKKLVAASQAALGLGSHHHHHH

SEQ ID NO: 165 - DNA, 2483 bp, synthetic construct
  source 1..2483: mol_type = other DNA
acgcgttctagagtgtcgtgaaaactacccctaaaagccaaagccgccaccatgaagctgtgggacgtggtggccgtgtgcctggtgctgctgcacaccgctagcgccttccctctgcctgccggcaagaggcctcctgaggcccctgccgaggacagaagcctgggcagaagaagagcccctttcgccctgagcagcgacagcaacatgcctgaggactaccctgatcagttcgacgacgtgatggacttcatccaagccaccatcaagagactgaagagaagccctgacaagcagatggccgtgctgcctagaagagagagaaacagacaagccgccgccgccaaccctgagaacagcagaggcaagggcagaagaggacagagaggcaagaacagaggctgcgtgctgaccgccatccacctgaacgtgaccgacctgggcctgggctacgagaccaaggaggagctgatcttcagatactgcagcggcagctgcgacgccgccgagaccacctacgacaagatcctgaagaacctgagcagaaacagaagactggtgagcgacaaggtgggccaagcctgctgcagacctatcgccttcgacgacgacctgagcttcctggacgacaacctggtgtaccacatcctgagaaagcacagcgccaagagatgcggctgcatcggatctgatgcccacaagagcgaggtcgcccatagattcaaggatctgggcgaggagaacttcaaggctctcgtgctcatcgctttcgcccagtatctgcagcagtgccctttcgaagaccatgtgaagctggtgaacgaggtgacagagttcgccaagacatgtgtggccgatgagagcgccgagaactgcgacaagtctctgcacacactgttcggagataagctgtgcacagtcgctactctgagggagacttacggcgaaatggccgactgttgtgccaagcaagagccagagaggaatgagtgcttcctccagcacaaggacgacaaccctaatctgcctagactcgtgaggccagaagtggatgtgatgtgcacagctttccacgacaacgaggagactttcctcaagaagtacctctacgagatcgctaggagacacccttacttctatgccccagagctgctcttcttcgccaagaggtataaagccgctttcacagagtgctgtcaagccgccgacaaagctgcttgtctgctgcctaagctggatgagctgagggatgagggcaaggcctctagcgccaaacaaggcctcaaatgcgcttccctccagaagttcggagagagggcctttaaggcttgggccgtcgctaggctcagccaaagattcccaaaggccgagttcgctgaggtgagcaagctggtcacagacctcactaaggtgcacactgagtgctgtcacggcgatctgctcgaatgtgccgacgacagagctgacctcgccaaatacatctgcgagaatcaagattccatcagctccaagctcaaggagtgctgtgagaagccactgctcgagaagagccattgcatcgccgaggtcgagaacgatgagatgccagccgatctgccttctctggctgccgatttcgtgggctccaaagacgtctgcaagaactacgccgaggctaaggacgtctttctgggcatgtttctgtacgagtatgctaggagacatccagattactccgtggtgctgctgctgagactggccaagacttacgagacaacactggaaaagtgctgcgccgctgctgacccacacgagtgctacgccaaggtgtttgacgagttcaagcctctcgtcgaggagccacagaatctgattaagcagaactgtgaactcttcgagcagctgggcgagtacaagttccaaaatgctctgctggtgaggtacactaagaaggtgcctcaagtgtccactcctacactggtggaggtgagcagaaatctcggcaaggtcggcagcaaatgttgcaagcacccagaggccaagagaatgccttgtgctgaggactgtctgagcgtgtttctgaaccagctctgtgtgctgcacgagaagacaccagtcagcgacagagtgactaagtgctgcacagagtctctggtgaacggaaggccatgtttctccgctctggaggtcgacgagacttacgtgcctaaggagttcaacgccgagactttcacattccacgccgacatctgcactctctccgaaaaggaaaggcagatcaagaagcagacagctctggtggagctggtcaagcacaagccaaaggccacaaaggaacagctcaaggctgtcatggacgacttcgccgccttcgtcgagaagtgttgcaaagccgacgacaaggagacatgcttcgccgaggagggcaaaaaactggtcgctgccagccaagccgctctcggcctcggatcccatcaccatcaccatcactgataagcggccgc

SEQ ID NO: 166 - protein, 787 aa, synthetic construct
DAHKSEVAHRFKDLGEENFKALVLIAFAQYLQQCPFEDHVKLVNEVTEFAKTCVADESAENCDKSLHTLFGDKLCTVATLRETYGEMADCCAKQEPERNECFLQHKDDNPNLPRLVRPEVDVMCTAFHDNEETFLKKYLYEIARRHPYFYAPELLFFAKRYKAAFTECCQAADKAACLLPKLDELRDEGKASSAKQGLKCASLQKFGERAFKAWAVARLSQRFPKAEFAEVSKLVTDLTKVHTECCHGDLLECADDRADLAKYICENQDSISSKLKECCEKPLLEKSHCIAEVENDEMPADLPSLAADFVGSKDVCKNYAEAKDVFLGMFLYEYARRHPDYSVVLLLRLAKTYETTLEKCCAAADPHECYAKVFDEFKPLVEEPQNLIKQNCELFEQLGEYKFQNALLVRYTKKVPQVSTPTLVEVSRNLGKVGSKCCKHPEAKRMPCAEDCLSVFLNQLCVLHEKTPVSDRVTKCCTESLVNGRPCFSALEVDETYVPKEFNAETFTFHADICTLSEKERQIKKQTALVELVKHKPKATKEQLKAVMDDFAAFVEKCCKADDKETCFAEEGKKLVAASQAALGLGSFPLPAGKRPPEAPAEDRSLGRRRAPFALSSDSNMPEDYPDQFDDVMDFIQATIKRLKRSPDKQMAVLPRRERNRQAAAANPENSRGKGRRGQRGKNRGCVLTAIHLNVTDLGLGYETKEELIFRYCSGSCDAAETTYDKILKNLSRNRRLVSDKVGQACCRPIAFDDDLSFLDDNLVYHILRKHSAKRCGCIGSHHHHHH

SEQ ID NO: 167 - DNA, 2470 bp, synthetic construct
  source 1..2470: mol_type = other DNA
acgcgtgccgccaccatgaagtgggtgactttcatctctctgctgttcctcttcagcagcgcctacagcagaggcgtgttcagaagggatgcccacaagagcgaggtcgcccatagattcaaggatctgggcgaggagaacttcaaggctctcgtgctcatcgctttcgcccagtatctgcagcagtgccctttcgaagaccatgtgaagctggtgaacgaggtgacagagttcgccaagacatgtgtggccgatgagagcgccgagaactgcgacaagtctctgcacacactgttcggagataagctgtgcacagtcgctactctgagggagacttacggcgaaatggccgactgttgtgccaagcaagagccagagaggaatgagtgcttcctccagcacaaggacgacaaccctaatctgcctagactcgtgaggccagaagtggatgtgatgtgcacagctttccacgacaacgaggagactttcctcaagaagtacctctacgagatcgctaggagacacccttacttctatgccccagagctgctcttcttcgccaagaggtataaagccgctttcacagagtgctgtcaagccgccgacaaagctgcttgtctgctgcctaagctggatgagctgagggatgagggcaaggcctctagcgccaaacaaggcctcaaatgcgcttccctccagaagttcggagagagggcctttaaggcttgggccgtcgctaggctcagccaaagattcccaaaggccgagttcgctgaggtgagcaagctggtcacagacctcactaaggtgcacactgagtgctgtcacggagatctgctcgaatgtgccgacgacagagctgacctcgccaaatacatctgcgagaatcaagattccatcagctccaagctcaaggagtgctgtgagaagccactgctcgagaagagccattgcatcgccgaggtcgagaacgatgagatgccagccgatctgccttctctggctgccgatttcgtgggctccaaagacgtctgcaagaactacgccgaggctaaggacgtctttctgggcatgtttctgtacgagtatgctaggagacatccagattactccgtggtgctgctgctgagactggccaagacttacgagacaacactggaaaagtgctgcgccgctgctgacccacacgagtgctacgccaaggtgtttgacgagttcaagcctctcgtcgaggagccacagaatctgattaagcagaactgtgaactcttcgagcagctgggcgagtacaagttccaaaatgctctgctggtgaggtacactaagaaggtgcctcaagtgtccactcctacactggtggaggtgagcagaaatctcggcaaggtcggcagcaaatgttgcaagcacccagaggccaagagaatgccttgtgctgaggactgtctgagcgtgtttctgaaccagctctgtgtgctgcacgagaagacaccagtcagcgacagagtgactaagtgctgcacagagtctctggtgaacggaaggccatgtttctccgctctggaggtcgacgagacttacgtgcctaaggagttcaacgccgagactttcacattccacgccgacatctgcactctctccgaaaaggaaaggcagatcaagaagcagacagctctggtggagctggtcaagcacaagccaaaggccacaaaggaacagctcaaggctgtcatggacgacttcgccgccttcgtcgagaagtgttgcaaagccgacgacaaggagacatgcttcgccgaggagggcaaaaaactggtcgctgccagccaagccgctctcggcctcggatctttccctctgcctgccggcaagaggcctcctgaggcccctgccgaggacagaagcctgggcagaagaagagcccctttcgccctgagcagcgacagcaacatgcctgaggactaccctgatcagttcgacgacgtgatggacttcatccaagccaccatcaagagactgaagagaagccctgacaagcagatggccgtgctgcctagaagagagagaaacagacaagccgccgccgccaaccctgagaacagcagaggcaagggcagaagaggacagagaggcaagaacagaggctgcgtgctgaccgccatccacctgaacgtgaccgacctgggcctgggctacgagaccaaggaggagctgatcttcagatactgcagcggcagctgcgacgccgccgagaccacctacgacaagatcctgaagaacctgagcagaaacagaagactggtgagcgacaaggtgggccaagcctgctgcagacctatcgccttcgacgacgacctgagcttcctggacgacaacctggtgtaccacatcctgagaaagcacagcgccaagagatgcggctgcatcggatcccatcaccatcaccatcactaataaggcgcgccgcggccgc

SEQ ID NO: 168 - protein, 110 aa, synthetic construct
ARLGARPCGLRELEVRVSELGLGYASDETVLFRYCAGACEAAARVYDLGLRRLRQRRRLRRERVRAQPCCRPTAYEDEVSFLDAHSRYHTVHELSARECACVGSHHHHHH

SEQ ID NO: 169 - DNA, 688 bp, synthetic construct
  source 1..688: mol_type = other DNA
acgcgttctagagtgtcgtgaaaactacccctaaaagccaaagccgccaccatgcagagatggaaggccgccgccctggctagcgtgctgtgcagcagcgtgctgagcatctggatgtgcagagagggcctgctgctgagccacagactgggccctgccctggtgcctctgcacagactgcctagaaccctggacgctagaatcgctagactggctcagtacagagccctgctgcaaggcgcccctgacgccatggagctaagagagttgacgccttgggccggaaggcctcctggtcctaggagacgcgctggacctagaagaagacgcgcaagagctagactgggcgctagaccttgcggcctcagagaacttgaagtaagagtgagcgagctgggcctgggctacgctagcgacgagactgtgctgttccgttattgcgccggcgcctgcgaagccgccgctagagtgtacgacctgggcctgagacgcctgcgtcaaagaagaagactgagaagagagagagtgagagctcagccttgctgcagacctaccgcctacgaggacgaggtgagcttcctggacgcccacagcagataccacaccgtgcacgagctgagcgctagagagtgcgcctgcgtgggatcccatcaccatcaccatcactaataaggcgcgccgcggccgc

SEQ ID NO: 170 - protein, 697 aa, synthetic construct
ARLGARPCGLRELEVRVSELGLGYASDETVLFRYCAGACEAAARVYDLGLRRLRQRRRLRRERVRAQPCCRPTAYEDEVSFLDAHSRYHTVHELSARECACVGSDAHKSEVAHRFKDLGEENFKALVLIAFAQYLQQCPFEDHVKLVNEVTEFAKTCVADESAENCDKSLHTLFGDKLCTVATLRETYGEMADCCAKQEPERNECFLQHKDDNPNLPRLVRPEVDVMCTAFHDNEETFLKKYLYEIARRHPYFYAPELLFFAKRYKAAFTECCQAADKAACLLPKLDELRDEGKASSAKQGLKCASLQKFGERAFKAWAVARLSQRFPKAEFAEVSKLVTDLTKVHTECCHGDLLECADDRADLAKYICENQDSISSKLKECCEKPLLEKSHCIAEVENDEMPADLPSLAADFVGSKDVCKNYAEAKDVFLGMFLYEYARRHPDYSVVLLLRLAKTYETTLEKCCAAADPHECYAKVFDEFKPLVEEPQNLIKQNCELFEQLGEYKFQNALLVRYTKKVPQVSTPTLVEVSRNLGKVGSKCCKHPEAKRMPCAEDCLSVFLNQLCVLHEKTPVSDRVTKCCTESLVNGRPCFSALEVDETYVPKEFNAETFTFHADICTLSEKERQIKKQTALVELVKHKPKATKEQLKAVMDDFAAFVEKCCKADDKETCFAEEGKKLVAASQAALGLGSHHHHHH

SEQ ID NO: 171 - DNA, 2441 bp, synthetic construct
  source 1..2441: mol_type = other DNA
acgcgttctagagtgtcgtgaaaactacccctaaaagccaaagccgccaccatgcagagatggaaggccgccgccctggctagcgtgctgtgcagcagcgtgctgagcatctggatgtgcagagagggcctgctgctgagccacagactgggccctgccctggtgcctctgcacagactgcctagaaccctggacgctagaatcgctagactggctcagtacagagccctgctgcaaggcgcccctgacgccatggagctaagagagttgacgccttgggccggaaggcctcctggtcctaggagacgcgctggacctagaagaagacgcgcaagagctagactgggcgctagaccttgcggcctcagagaacttgaagtaagagtgagcgagctgggcctgggctacgctagcgacgagactgtgctgttccgttattgcgccggcgcctgcgaagccgccgctagagtgtacgacctgggcctgagacgcctgcgtcaaagaagaagactgagaagagagagagtgagagctcagccttgctgcagacctaccgcctacgaggacgaggtgagcttcctggacgcccacagcagataccacaccgtgcacgagctgagcgctagagagtgcgcctgcgtgggatctgatgcccacaagagcgaggtcgcccatagattcaaggatctgggcgaggagaacttcaaggctctcgtgctcatcgctttcgcccagtatctgcagcagtgccctttcgaagaccatgtgaagctggtgaacgaggtgacagagttcgccaagacatgtgtggccgatgagagcgccgagaactgcgacaagtctctgcacacactgttcggagataagctgtgcacagtcgctactctgagggagacttacggcgaaatggccgactgttgtgccaagcaagagccagagaggaatgagtgcttcctccagcacaaggacgacaaccctaatctgcctagactcgtgaggccagaagtggatgtgatgtgcacagctttccacgacaacgaggagactttcctcaagaagtacctctacgagatcgctaggagacacccttacttctatgccccagagctgctcttcttcgccaagaggtataaagccgctttcacagagtgctgtcaagccgccgacaaagctgcttgtctgctgcctaagctggatgagctgagggatgagggcaaggcctctagcgccaaacaaggcctcaaatgcgcttccctccagaagttcggagagagggcctttaaggcttgggccgtcgctaggctcagccaaagattcccaaaggccgagttcgctgaggtgagcaagctggtcacagacctcactaaggtgcacactgagtgctgtcacggcgatctgctcgaatgtgccgacgacagagctgacctcgccaaatacatctgcgagaatcaagattccatcagctccaagctcaaggagtgctgtgagaagccactgctcgagaagagccattgcatcgccgaggtcgagaacgatgagatgccagccgatctgccttctctggctgccgatttcgtgggctccaaagacgtctgcaagaactacgccgaggctaaggacgtctttctgggcatgtttctgtacgagtatgctaggagacatccagattactccgtggtgctgctgctgagactggccaagacttacgagacaacactggaaaagtgctgcgccgctgctgacccacacgagtgctacgccaaggtgtttgacgagttcaagcctctcgtcgaggagccacagaatctgattaagcagaactgtgaactcttcgagcagctgggcgagtacaagttccaaaatgctctgctggtgaggtacactaagaaggtgcctcaagtgtccactcctacactggtggaggtgagcagaaatctcggcaaggtcggcagcaaatgttgcaagcacccagaggccaagagaatgccttgtgctgaggactgtctgagcgtgtttctgaaccagctctgtgtgctgcacgagaagacaccagtcagcgacagagtgactaagtgctgcacagagtctctggtgaacggaaggccatgtttctccgctctggaggtcgacgagacttacgtgcctaaggagttcaacgccgagactttcacattccacgccgacatctgcactctctccgaaaaggaaaggcagatcaagaagcagacagctctggtggagctggtcaagcacaagccaaaggccacaaaggaacagctcaaggctgtcatggacgacttcgccgccttcgtcgagaagtgttgcaaagccgacgacaaggagacatgcttcgccgaggagggcaaaaaactggtcgctgccagccaagccgctctcggcctcggatcccatcaccatcaccatcactgataagcggccgc

SEQ ID NO: 172 - protein, 773 aa, synthetic construct
DAHKSEVAHRFKDLGEENFKALVLIAFAQYLQQCPFEDHVKLVNEVTEFAKTCVADESAENCDKSLHTLFGDKLCTVATLRETYGEMADCCAKQEPERNECFLQHKDDNPNLPRLVRPEVDVMCTAFHDNEETFLKKYLYEIARRHPYFYAPELLFFAKRYKAAFTECCQAADKAACLLPKLDELRDEGKASSAKQGLKCASLQKFGERAFKAWAVARLSQRFPKAEFAEVSKLVTDLTKVHTECCHGDLLECADDRADLAKYICENQDSISSKLKECCEKPLLEKSHCIAEVENDEMPADLPSLAADFVGSKDVCKNYAEAKDVFLGMFLYEYARRHPDYSVVLLLRLAKTYETTLEKCCAAADPHECYAKVFDEFKPLVEEPQNLIKQNCELFEQLGEYKFQNALLVRYTKKVPQVSTPTLVEVSRNLGKVGSKCCKHPEAKRMPCAEDCLSVFLNQLCVLHEKTPVSDRVTKCCTESLVNGRPCFSALEVDETYVPKEFNAETFTFHADICTLSEKERQIKKQTALVELVKHKPKATKEQLKAVMDDFAAFVEKCCKADDKETCFAEEGKKLVAASQAALGLGSIWMCREGLLLSHRLGPALVPLHRLPRTLDARIARLAQYRALLQGAPDAMELRELTPWAGRPPGPRRRAGPRRRRARARLGARPCGLRELEVRVSELGLGYASDETVLFRYCAGACEAAARVYDLGLRRLRQRRRLRRERVRAQPCCRPTAYEDEVSFLDAHSRYHTVHELSARECACVGSHHHHHH

SEQ ID NO: 173 - DNA, 2428 bp, synthetic construct
  source 1..2428: mol_type = other DNA
acgcgtgccgccaccatgaagtgggtgactttcatctctctgctgttcctcttcagcagcgcctacagcagaggcgtgttcagaagggatgcccacaagagcgaggtcgcccatagattcaaggatctgggcgaggagaacttcaaggctctcgtgctcatcgctttcgcccagtatctgcagcagtgccctttcgaagaccatgtgaagctggtgaacgaggtgacagagttcgccaagacatgtgtggccgatgagagcgccgagaactgcgacaagtctctgcacacactgttcggagataagctgtgcacagtcgctactctgagggagacttacggcgaaatggccgactgttgtgccaagcaagagccagagaggaatgagtgcttcctccagcacaaggacgacaaccctaatctgcctagactcgtgaggccagaagtggatgtgatgtgcacagctttccacgacaacgaggagactttcctcaagaagtacctctacgagatcgctaggagacacccttacttctatgccccagagctgctcttcttcgccaagaggtataaagccgctttcacagagtgctgtcaagccgccgacaaagctgcttgtctgctgcctaagctggatgagctgagggatgagggcaaggcctctagcgccaaacaaggcctcaaatgcgcttccctccagaagttcggagagagggcctttaaggcttgggccgtcgctaggctcagccaaagattcccaaaggccgagttcgctgaggtgagcaagctggtcacagacctcactaaggtgcacactgagtgctgtcacggagatctgctcgaatgtgccgacgacagagctgacctcgccaaatacatctgcgagaatcaagattccatcagctccaagctcaaggagtgctgtgagaagccactgctcgagaagagccattgcatcgccgaggtcgagaacgatgagatgccagccgatctgccttctctggctgccgatttcgtgggctccaaagacgtctgcaagaactacgccgaggctaaggacgtctttctgggcatgtttctgtacgagtatgctaggagacatccagattactccgtggtgctgctgctgagactggccaagacttacgagacaacactggaaaagtgctgcgccgctgctgacccacacgagtgctacgccaaggtgtttgacgagttcaagcctctcgtcgaggagccacagaatctgattaagcagaactgtgaactcttcgagcagctgggcgagtacaagttccaaaatgctctgctggtgaggtacactaagaaggtgcctcaagtgtccactcctacactggtggaggtgagcagaaatctcggcaaggtcggcagcaaatgttgcaagcacccagaggccaagagaatgccttgtgctgaggactgtctgagcgtgtttctgaaccagctctgtgtgctgcacgagaagacaccagtcagcgacagagtgactaagtgctgcacagagtctctggtgaacggaaggccatgtttctccgctctggaggtcgacgagacttacgtgcctaaggagttcaacgccgagactttcacattccacgccgacatctgcactctctccgaaaaggaaaggcagatcaagaagcagacagctctggtggagctggtcaagcacaagccaaaggccacaaaggaacagctcaaggctgtcatggacgacttcgccgccttcgtcgagaagtgttgcaaagccgacgacaaggagacatgcttcgccgaggagggcaaaaaactggtcgctgccagccaagccgctctcggcctcggatctatctggatgtgcagagagggcctgctgctgagccacagactgggccctgccctggtgcctctgcacagactgcctagaaccctggacgctagaatcgctagactggctcagtacagagccctgctgcaaggcgcccctgacgccatggagctaagagagttgacgccttgggccggaaggcctcctggtcctaggagacgcgctggacctagaagaagacgcgcaagagctagactgggcgctagaccttgcggcctcagagaacttgaagtaagagtgagcgagctgggcctgggctacgctagcgacgagactgtgctgttccgttattgcgccggcgcctgcgaagccgccgctagagtgtacgacctgggcctgagacgcctgcgtcaaagaagaagactgagaagagagagagtgagagctcagccttgctgcagacctaccgcctacgaggacgaggtgagcttcctggacgcccacagcagataccacaccgtgcacgagctgagcgctagagagtgcgcctgcgtgggatcccatcaccatcaccatcactaataaggcgcgccgcggccgc

SEQ ID NO: 174 - protein, 121 aa, synthetic construct
AGGPGSRARAAGARGCRLRSQLVPVRALGLGHRSDELVRFRFCSGSCRRARSPHDLSLASLLGAGALRPPPGSRPVSQPCCRPTRYEAVSFMDVNSTWRTVDRLSATACGCLGGSHHHHHH

SEQ ID NO: 175 - DNA, 757 bp, synthetic construct
  source 1..757: mol_type = other DNA
acgcgttctagagtgtcgtgaaaactacccctaaaagccaaagccgccaccatggagctcggcctgggcggcctgtctaccctgtcccactgcccgtggcctcgacagcagccggcactctggcctacactcgctgccttggcactactaagctcggtcgccgaggctagcctgggtagcgcccctcgaagccccgcccctcgtgagggtcccccaccggtacttgcgtctcctgctggtcacctgcctgggggcagaaccgctagatggtgcagcggcagagctagacgaccaccccctcaaccgagcagacccgcccctccaccgcctgccccgccgagtgctttgcctcgtggtgggcgtgccgctagagccggcggccctggctcacgcgcacgggcagctggcgctagaggctgcagactgaggtctcagctggtgcctgtgagagccctaggcctgggccacagaagcgacgagctggtgagattcagattctgcagcggcagctgcagaagagctagatcccctcacgatttgagcctggcctcattgctcggcgccggcgccctgcgacctccaccgggcagcagacctgtgtctcagccttgctgcagacctacaagatacgaggccgtgagcttcatggacgtgaacagcacctggagaaccgtggacagactgagcgccaccgcctgcggctgcctgggcggatcccatcaccatcaccatcactaataaggcgcgccgcggccgc

SEQ ID NO: 176 - protein, 708 aa, synthetic construct
AGGPGSRARAAGARGCRLRSQLVPVRALGLGHRSDELVRFRFCSGSCRRARSPHDLSLASLLGAGALRPPPGSRPVSQPCCRPTRYEAVSFMDVNSTWRTVDRLSATACGCLGGSDAHKSEVAHRFKDLGEENFKALVLIAFAQYLQQCPFEDHVKLVNEVTEFAKTCVADESAENCDKSLHTLFGDKLCTVATLRETYGEMADCCAKQEPERNECFLQHKDDNPNLPRLVRPEVDVMCTAFHDNEETFLKKYLYEIARRHPYFYAPELLFFAKRYKAAFTECCQAADKAACLLPKLDELRDEGKASSAKQGLKCASLQKFGERAFKAWAVARLSQRFPKAEFAEVSKLVTDLTKVHTECCHGDLLECADDRADLAKYICENQDSISSKLKECCEKPLLEKSHCIAEVENDEMPADLPSLAADFVGSKDVCKNYAEAKDVFLGMFLYEYARRHPDYSVVLLLRLAKTYETTLEKCCAAADPHECYAKVFDEFKPLVEEPQNLIKQNCELFEQLGEYKFQNALLVRYTKKVPQVSTPTLVEVSRNLGKVGSKCCKHPEAKRMPCAEDCLSVFLNQLCVLHEKTPVSDRVTKCCTESLVNGRPCFSALEVDETYVPKEFNAETFTFHADICTLSEKERQIKKQTALVELVKHKPKATKEQLKAVMDDFAAFVEKCCKADDKETCFAEEGKKLVAASQAALGLGSHHHHHH

SEQ ID NO: 177 - DNA, 2510 bp, synthetic construct
  source 1..2510: mol_type = other DNA
acgcgttctagagtgtcgtgaaaactacccctaaaagccaaagccgccaccatggagctcggcctgggcggcctgtctaccctgtcccactgcccgtggcctcgacagcagccggcactctggcctacactcgctgccttggcactactaagctcggtcgccgaggctagcctgggtagcgcccctcgaagccccgcccctcgtgagggtcccccaccggtacttgcgtctcctgctggtcacctgcctgggggcagaaccgctagatggtgcagcggcagagctagacgaccaccccctcaaccgagcagacccgcccctccaccgcctgccccgccgagtgctttgcctcgtggtgggcgtgccgctagagccggcggccctggctcacgcgcacgggcagctggcgctagaggctgcagactgaggtctcagctggtgcctgtgagagccctaggcctgggccacagaagcgacgagctggtgagattcagattctgcagcggcagctgcagaagagctagatcccctcacgatttgagcctggcctcattgctcggcgccggcgccctgcgacctccaccgggcagcagacctgtgtctcagccttgctgcagacctacaagatacgaggccgtgagcttcatggacgtgaacagcacctggagaaccgtggacagactgagcgccaccgcctgcggctgcctgggcggatctgatgcccacaagagcgaggtcgcccatagattcaaggatctgggcgaggagaacttcaaggctctcgtgctcatcgctttcgcccagtatctgcagcagtgccctttcgaagaccatgtgaagctggtgaacgaggtgacagagttcgccaagacatgtgtggccgatgagagcgccgagaactgcgacaagtctctgcacacactgttcggagataagctgtgcacagtcgctactctgagggagacttacggcgaaatggccgactgttgtgccaagcaagagccagagaggaatgagtgcttcctccagcacaaggacgacaaccctaatctgcctagactcgtgaggccagaagtggatgtgatgtgcacagctttccacgacaacgaggagactttcctcaagaagtacctctacgagatcgctaggagacacccttacttctatgccccagagctgctcttcttcgccaagaggtataaagccgctttcacagagtgctgtcaagccgccgacaaagctgcttgtctgctgcctaagctggatgagctgagggatgagggcaaggcctctagcgccaaacaaggcctcaaatgcgcttccctccagaagttcggagagagggcctttaaggcttgggccgtcgctaggctcagccaaagattcccaaaggccgagttcgctgaggtgagcaagctggtcacagacctcactaaggtgcacactgagtgctgtcacggcgatctgctcgaatgtgccgacgacagagctgacctcgccaaatacatctgcgagaatcaagattccatcagctccaagctcaaggagtgctgtgagaagccactgctcgagaagagccattgcatcgccgaggtcgagaacgatgagatgccagccgatctgccttctctggctgccgatttcgtgggctccaaagacgtctgcaagaactacgccgaggctaaggacgtctttctgggcatgtttctgtacgagtatgctaggagacatccagattactccgtggtgctgctgctgagactggccaagacttacgagacaacactggaaaagtgctgcgccgctgctgacccacacgagtgctacgccaaggtgtttgacgagttcaagcctctcgtcgaggagccacagaatctgattaagcagaactgtgaactcttcgagcagctgggcgagtacaagttccaaaatgctctgctggtgaggtacactaagaaggtgcctcaagtgtccactcctacactggtggaggtgagcagaaatctcggcaaggtcggcagcaaatgttgcaagcacccagaggccaagagaatgccttgtgctgaggactgtctgagcgtgtttctgaaccagctctgtgtgctgcacgagaagacaccagtcagcgacagagtgactaagtgctgcacagagtctctggtgaacggaaggccatgtttctccgctctggaggtcgacgagacttacgtgcctaaggagttcaacgccgagactttcacattccacgccgacatctgcactctctccgaaaaggaaaggcagatcaagaagcagacagctctggtggagctggtcaagcacaagccaaaggccacaaaggaacagctcaaggctgtcatggacgacttcgccgccttcgtcgagaagtgttgcaaagccgacgacaaggagacatgcttcgccgaggagggcaaaaaactggtcgctgccagccaagccgctctcggcctcggatcccatcaccatcaccatcactgataagcggccgc

SEQ ID NO: 178 - protein, 776 aa, synthetic construct
DAHKSEVAHRFKDLGEENFKALVLIAFAQYLQQCPFEDHVKLVNEVTEFAKTCVADESAENCDKSLHTLFGDKLCTVATLRETYGEMADCCAKQEPERNECFLQHKDDNPNLPRLVRPEVDVMCTAFHDNEETFLKKYLYEIARRHPYFYAPELLFFAKRYKAAFTECCQAADKAACLLPKLDELRDEGKASSAKQGLKCASLQKFGERAFKAWAVARLSQRFPKAEFAEVSKLVTDLTKVHTECCHGDLLECADDRADLAKYICENQDSISSKLKECCEKPLLEKSHCIAEVENDEMPADLPSLAADFVGSKDVCKNYAEAKDVFLGMFLYEYARRHPDYSVVLLLRLAKTYETTLEKCCAAADPHECYAKVFDEFKPLVEEPQNLIKQNCELFEQLGEYKFQNALLVRYTKKVPQVSTPTLVEVSRNLGKVGSKCCKHPEAKRMPCAEDCLSVFLNQLCVLHEKTPVSDRVTKCCTESLVNGRPCFSALEVDETYVPKEFNAETFTFHADICTLSEKERQIKKQTALVELVKHKPKATKEQLKAVMDDFAAFVEKCCKADDKETCFAEEGKKLVAASQAALGLGSSLGSAPRSPAPREGPPPVLASPAGHLPGGRTARWCSGRARRPPPQPSRPAPPPPAPPSALPRGGRAARAGGPGSRARAAGARGCRLRSQLVPVRALGLGHRSDELVRFRFCSGSCRRARSPHDLSLASLLGAGALRPPPGSRPVSQPCCRPTRYEAVSFMDVNSTWRTVDRLSATACGCLGGSHHHHHH

SEQ ID NO: 179 - DNA, 2437 bp, synthetic construct
  source 1..2437: mol_type = other DNA
acgcgtgccgccaccatgaagtgggtgactttcatctctctgctgttcctcttcagcagcgcctacagcagaggcgtgttcagaagggatgcccacaagagcgaggtcgcccatagattcaaggatctgggcgaggagaacttcaaggctctcgtgctcatcgctttcgcccagtatctgcagcagtgccctttcgaagaccatgtgaagctggtgaacgaggtgacagagttcgccaagacatgtgtggccgatgagagcgccgagaactgcgacaagtctctgcacacactgttcggagataagctgtgcacagtcgctactctgagggagacttacggcgaaatggccgactgttgtgccaagcaagagccagagaggaatgagtgcttcctccagcacaaggacgacaaccctaatctgcctagactcgtgaggccagaagtggatgtgatgtgcacagctttccacgacaacgaggagactttcctcaagaagtacctctacgagatcgctaggagacacccttacttctatgccccagagctgctcttcttcgccaagaggtataaagccgctttcacagagtgctgtcaagccgccgacaaagctgcttgtctgctgcctaagctggatgagctgagggatgagggcaaggcctctagcgccaaacaaggcctcaaatgcgcttccctccagaagttcggagagagggcctttaaggcttgggccgtcgctaggctcagccaaagattcccaaaggccgagttcgctgaggtgagcaagctggtcacagacctcactaaggtgcacactgagtgctgtcacggagatctgctcgaatgtgccgacgacagagctgacctcgccaaatacatctgcgagaatcaagattccatcagctccaagctcaaggagtgctgtgagaagccactgctcgagaagagccattgcatcgccgaggtcgagaacgatgagatgccagccgatctgccttctctggctgccgatttcgtgggctccaaagacgtctgcaagaactacgccgaggctaaggacgtctttctgggcatgtttctgtacgagtatgctaggagacatccagattactccgtggtgctgctgctgagactggccaagacttacgagacaacactggaaaagtgctgcgccgctgctgacccacacgagtgctacgccaaggtgtttgacgagttcaagcctctcgtcgaggagccacagaatctgattaagcagaactgtgaactcttcgagcagctgggcgagtacaagttccaaaatgctctgctggtgaggtacactaagaaggtgcctcaagtgtccactcctacactggtggaggtgagcagaaatctcggcaaggtcggcagcaaatgttgcaagcacccagaggccaagagaatgccttgtgctgaggactgtctgagcgtgtttctgaaccagctctgtgtgctgcacgagaagacaccagtcagcgacagagtgactaagtgctgcacagagtctctggtgaacggaaggccatgtttctccgctctggaggtcgacgagacttacgtgcctaaggagttcaacgccgagactttcacattccacgccgacatctgcactctctccgaaaaggaaaggcagatcaagaagcagacagctctggtggagctggtcaagcacaagccaaaggccacaaaggaacagctcaaggctgtcatggacgacttcgccgccttcgtcgagaagtgttgcaaagccgacgacaaggagacatgcttcgccgaggagggcaaaaaactggtcgctgccagccaagccgctctcggcctcggatctagcctgggtagcgcccctcgaagccccgcccctcgtgagggtcccccaccggtacttgcgtctcctgctggtcacctgcctgggggcagaaccgctagatggtgcagcggcagagctagacgaccaccccctcaaccgagcagacccgcccctccaccgcctgccccgccgagtgctttgcctcgtggtgggcgtgccgctagagccggcggccctggctcacgcgcacgggcagctggcgctagaggctgcagactgaggtctcagctggtgcctgtgagagccctaggcctgggccacagaagcgacgagctggtgagattcagattctgcagcggcagctgcagaagagctagatcccctcacgatttgagcctggcctcattgctcggcgccggcgccctgcgacctccaccgggcagcagacctgtgtctcagccttgctgcagacctacaagatacgaggccgtgagcttcatggacgtgaacagcacctggagaaccgtggacagactgagcgccaccgcctgcggctgcctgggcggatcccatcaccatcaccatcactaataaggcgcgccgcggccgc

SEQ ID NO: 180 - protein, 104 aa, synthetic construct
ALSGPCQLWSLTLSVAELGLGYASEEKVIFRYCAGSCPRGARTQHGLALARLQGQGRAHGGPCCRPTRYTDVAFLDDRHRWQRLPQLSAAACGCGGGSHHHHHH

SEQ ID NO: 181 - DNA, 565 bp, synthetic construct
  source 1..565: mol_type = other DNA
acgcgttctagagtgtcgtgaaaactacccctaaaagccaaagccgccaccatggccgtgggcaagttcctcctgggcagtctcctcctgctgagtcttcaactgggccaaggctggggccctgacgctagaggcgtcccggtggccgatggcgaatttagcagcgagcaagtggccaaggccggcggcacgtggctgggcacccacagacctctcgctagactgagaagagccctgagcggcccttgtcagctgtggagcctgaccctgagcgtggccgagctgggcctgggctacgctagcgaggagaaggtgatcttcagatattgcgctggctcctgtcctaggggggctagaacccaacatggcctggccctagcccgcctgcaaggccaaggcagagcccacggcggcccttgctgcagacctacaagatacaccgacgtggccttcctggacgacagacacagatggcagagactgcctcagctgagcgccgccgcctgcggctgcggcggcggatcccatcaccatcaccatcactaataaggcgcgccgcggccgc

SEQ ID NO: 182 - protein, 691 aa, synthetic construct
ALSGPCQLWSLTLSVAELGLGYASEEKVIFRYCAGSCPRGARTQHGLALARLQGQGRAHGGPCCRPTRYTDVAFLDDRHRWQRLPQLSAAACGCGGGSDAHKSEVAHRFKDLGEENFKALVLIAFAQYLQQCPFEDHVKLVNEVTEFAKTCVADESAENCDKSLHTLFGDKLCTVATLRETYGEMADCCAKQEPERNECFLQHKDDNPNLPRLVRPEVDVMCTAFHDNEETFLKKYLYEIARRHPYFYAPELLFFAKRYKAAFTECCQAADKAACLLPKLDELRDEGKASSAKQGLKCASLQKFGERAFKAWAVARLSQRFPKAEFAEVSKLVTDLTKVHTECCHGDLLECADDRADLAKYICENQDSISSKLKECCEKPLLEKSHCIAEVENDEMPADLPSLAADFVGSKDVCKNYAEAKDVFLGMFLYEYARRHPDYSVVLLLRLAKTYETTLEKCCAAADPHECYAKVFDEFKPLVEEPQNLIKQNCELFEQLGEYKFQNALLVRYTKKVPQVSTPTLVEVSRNLGKVGSKCCKHPEAKRMPCAEDCLSVFLNQLCVLHEKTPVSDRVTKCCTESLVNGRPCFSALEVDETYVPKEFNAETFTFHADICTLSEKERQIKKQTALVELVKHKPKATKEQLKAVMDDFAAFVEKCCKADDKETCFAEEGKKLVAASQAALGLGSHHHHHH

SEQ ID NO: 183 - DNA, 2318 bp, synthetic construct
  source 1..2318: mol_type = other DNA
acgcgttctagagtgtcgtgaaaactacccctaaaagccaaagccgccaccatggccgtgggcaagttcctcctgggcagtctcctcctgctgagtcttcaactgggccaaggctggggccctgacgctagaggcgtcccggtggccgatggcgaatttagcagcgagcaagtggccaaggccggcggcacgtggctgggcacccacagacctctcgctagactgagaagagccctgagcggcccttgtcagctgtggagcctgaccctgagcgtggccgagctgggcctgggctacgctagcgaggagaaggtgatcttcagatattgcgctggctcctgtcctaggggggctagaacccaacatggcctggccctagcccgcctgcaaggccaaggcagagcccacggcggcccttgctgcagacctacaagatacaccgacgtggccttcctggacgacagacacagatggcagagactgcctcagctgagcgccgccgcctgcggctgcggcggcggatctgatgcccacaagagcgaggtcgcccatagattcaaggatctgggcgaggagaacttcaaggctctcgtgctcatcgctttcgcccagtatctgcagcagtgccctttcgaagaccatgtgaagctggtgaacgaggtgacagagttcgccaagacatgtgtggccgatgagagcgccgagaactgcgacaagtctctgcacacactgttcggagataagctgtgcacagtcgctactctgagggagacttacggcgaaatggccgactgttgtgccaagcaagagccagagaggaatgagtgcttcctccagcacaaggacgacaaccctaatctgcctagactcgtgaggccagaagtggatgtgatgtgcacagctttccacgacaacgaggagactttcctcaagaagtacctctacgagatcgctaggagacacccttacttctatgccccagagctgctcttcttcgccaagaggtataaagccgctttcacagagtgctgtcaagccgccgacaaagctgcttgtctgctgcctaagctggatgagctgagggatgagggcaaggcctctagcgccaaacaaggcctcaaatgcgcttccctccagaagttcggagagagggcctttaaggcttgggccgtcgctaggctcagccaaagattcccaaaggccgagttcgctgaggtgagcaagctggtcacagacctcactaaggtgcacactgagtgctgtcacggcgatctgctcgaatgtgccgacgacagagctgacctcgccaaatacatctgcgagaatcaagattccatcagctccaagctcaaggagtgctgtgagaagccactgctcgagaagagccattgcatcgccgaggtcgagaacgatgagatgccagccgatctgccttctctggctgccgatttcgtgggctccaaagacgtctgcaagaactacgccgaggctaaggacgtctttctgggcatgtttctgtacgagtatgctaggagacatccagattactccgtggtgctgctgctgagactggccaagacttacgagacaacactggaaaagtgctgcgccgctgctgacccacacgagtgctacgccaaggtgtttgacgagttcaagcctctcgtcgaggagccacagaatctgattaagcagaactgtgaactcttcgagcagctgggcgagtacaagttccaaaatgctctgctggtgaggtacactaagaaggtgcctcaagtgtccactcctacactggtggaggtgagcagaaatctcggcaaggtcggcagcaaatgttgcaagcacccagaggccaagagaatgccttgtgctgaggactgtctgagcgtgtttctgaaccagctctgtgtgctgcacgagaagacaccagtcagcgacagagtgactaagtgctgcacagagtctctggtgaacggaaggccatgtttctccgctctggaggtcgacgagacttacgtgcctaaggagttcaacgccgagactttcacattccacgccgacatctgcactctctccgaaaaggaaaggcagatcaagaagcagacagctctggtggagctggtcaagcacaagccaaaggccacaaaggaacagctcaaggctgtcatggacgacttcgccgccttcgtcgagaagtgttgcaaagccgacgacaaggagacatgcttcgccgaggagggcaaaaaactggtcgctgccagccaagccgctctcggcctcggatcccatcaccatcaccatcactgataagcggccgc

SEQ ID NO: 184 - protein, 730 aa, synthetic construct
DAHKSEVAHRFKDLGEENFKALVLIAFAQYLQQCPFEDHVKLVNEVTEFAKTCVADESAENCDKSLHTLFGDKLCTVATLRETYGEMADCCAKQEPERNECFLQHKDDNPNLPRLVRPEVDVMCTAFHDNEETFLKKYLYEIARRHPYFYAPELLFFAKRYKAAFTECCQAADKAACLLPKLDELRDEGKASSAKQGLKCASLQKFGERAFKAWAVARLSQRFPKAEFAEVSKLVTDLTKVHTECCHGDLLECADDRADLAKYICENQDSISSKLKECCEKPLLEKSHCIAEVENDEMPADLPSLAADFVGSKDVCKNYAEAKDVFLGMFLYEYARRHPDYSVVLLLRLAKTYETTLEKCCAAADPHECYAKVFDEFKPLVEEPQNLIKQNCELFEQLGEYKFQNALLVRYTKKVPQVSTPTLVEVSRNLGKVGSKCCKHPEAKRMPCAEDCLSVFLNQLCVLHEKTPVSDRVTKCCTESLVNGRPCFSALEVDETYVPKEFNAETFTFHADICTLSEKERQIKKQTALVELVKHKPKATKEQLKAVMDDFAAFVEKCCKADDKETCFAEEGKKLVAASQAALGLGSWGPDARGVPVADGEFSSEQVAKAGGTWLGTHRPLARLRRALSGPCQLWSLTLSVAELGLGYASEEKVIFRYCAGSCPRGARTQHGLALARLQGQGRAHGGPCCRPTRYTDVAFLDDRHRWQRLPQLSAAACGCGGGSHHHHHH

SEQ ID NO: 185 - DNA, 2299 bp, synthetic construct
  source 1..2299: mol_type = other DNA
acgcgtgccgccaccatgaagtgggtgactttcatctctctgctgttcctcttcagcagcgcctacagcagaggcgtgttcagaagggatgcccacaagagcgaggtcgcccatagattcaaggatctgggcgaggagaacttcaaggctctcgtgctcatcgctttcgcccagtatctgcagcagtgccctttcgaagaccatgtgaagctggtgaacgaggtgacagagttcgccaagacatgtgtggccgatgagagcgccgagaactgcgacaagtctctgcacacactgttcggagataagctgtgcacagtcgctactctgagggagacttacggcgaaatggccgactgttgtgccaagcaagagccagagaggaatgagtgcttcctccagcacaaggacgacaaccctaatctgcctagactcgtgaggccagaagtggatgtgatgtgcacagctttccacgacaacgaggagactttcctcaagaagtacctctacgagatcgctaggagacacccttacttctatgccccagagctgctcttcttcgccaagaggtataaagccgctttcacagagtgctgtcaagccgccgacaaagctgcttgtctgctgcctaagctggatgagctgagggatgagggcaaggcctctagcgccaaacaaggcctcaaatgcgcttccctccagaagttcggagagagggcctttaaggcttgggccgtcgctaggctcagccaaagattcccaaaggccgagttcgctgaggtgagcaagctggtcacagacctcactaaggtgcacactgagtgctgtcacggagatctgctcgaatgtgccgacgacagagctgacctcgccaaatacatctgcgagaatcaagattccatcagctccaagctcaaggagtgctgtgagaagccactgctcgagaagagccattgcatcgccgaggtcgagaacgatgagatgccagccgatctgccttctctggctgccgatttcgtgggctccaaagacgtctgcaagaactacgccgaggctaaggacgtctttctgggcatgtttctgtacgagtatgctaggagacatccagattactccgtggtgctgctgctgagactggccaagacttacgagacaacactggaaaagtgctgcgccgctgctgacccacacgagtgctacgccaaggtgtttgacgagttcaagcctctcgtcgaggagccacagaatctgattaagcagaactgtgaactcttcgagcagctgggcgagtacaagttccaaaatgctctgctggtgaggtacactaagaaggtgcctcaagtgtccactcctacactggtggaggtgagcagaaatctcggcaaggtcggcagcaaatgttgcaagcacccagaggccaagagaatgccttgtgctgaggactgtctgagcgtgtttctgaaccagctctgtgtgctgcacgagaagacaccagtcagcgacagagtgactaagtgctgcacagagtctctggtgaacggaaggccatgtttctccgctctggaggtcgacgagacttacgtgcctaaggagttcaacgccgagactttcacattccacgccgacatctgcactctctccgaaaaggaaaggcagatcaagaagcagacagctctggtggagctggtcaagcacaagccaaaggccacaaaggaacagctcaaggctgtcatggacgacttcgccgccttcgtcgagaagtgttgcaaagccgacgacaaggagacatgcttcgccgaggagggcaaaaaactggtcgctgccagccaagccgctctcggcctcggatcttggggccctgacgctagaggcgtcccggtggccgatggcgaatttagcagcgagcaagtggccaaggccggcggcacgtggctgggcacccacagacctctcgctagactgagaagagccctgagcggcccttgtcagctgtggagcctgaccctgagcgtggccgagctgggcctgggctacgctagcgaggagaaggtgatcttcagatattgcgctggctcctgtcctaggggggctagaacccaacatggcctggccctagcccgcctgcaaggccaaggcagagcccacggcggcccttgctgcagacctacaagatacaccgacgtggccttcctggacgacagacacagatggcagagactgcctcagctgagcgccgccgcctgcggctgcggcggcggatcccatcaccatcaccatcactaataaggcgcgccgcggccgc

SEQ ID NO: 186 - protein, 116 aa, synthetic construct
QVQLVESGGGLVQPGGSLRLSCAASGSIFDIYVMRWYRQAPGKGLEWVASIYDGGRNDYDNVVKGRFTISRDNSKNTLYLQMNSLRAEDTAVYFCNVLTYAGRPYWGQGTQVTVSS

SEQ ID NO: 187 - DNA, 348 bp, synthetic construct
  source 1..348: mol_type = other DNA
caagtgcagctggtcgagagcggaggaggactggtccagcccggcggctctctgagactgagctgtgccgccagcggcagcatcttcgacatctacgtgatgaggtggtacaggcaagcccccggcaagggactggagtgggtcgccagcatctacgatggcggaaggaatgactacgacaacgtggtgaagggaaggttcactatctctagggacaacagcaagaacactctctatctgcagatgaactctctgagggctgaggatacagccgtgtacttctgcaacgtgctgacttatgccggaaggccatactggggacaaggcactcaggtgacagtgagcagc

SEQ ID NO: 188 - DNA, 26 bp, synthetic construct
  source 1..26: mol_type = other DNA
ttgaattcacgcgtgccgccaccatg

SEQ ID NO: 189 - DNA, 29 bp, synthetic construct
  source 1..29: mol_type = other DNA
tttggatccgctgctcactgtcacctgag

SEQ ID NO: 190 - DNA, 47 bp, synthetic construct
  source 1..47: mol_type = other DNA
ttctgtctttgcggccgcttatcagaggccgagagcggcttggctgg

SEQ ID NO: 191 - protein, 240 aa, synthetic construct
HSDPARRGELSVCDSISEWVTAADKKTAVDMSGGTVTVLEKVPVSKGQLKQYFYETKCNPMGYTKEGCRGIDKRHWNSQCRTTQSYVRALTMDSKKRIGWRFIRIDTSCVCTLTIKRGRGSGGSQVQLVESGGGLVQPGGSLRLSCAASGSIFDIYVMRWYRQAPGKGLEWVASIYDGGRNDYDNVVKGRFTISRDNSKNTLYLQMNSLRAEDTAVYFCNVLTYAGRPYWGQGTQVTVSS

SEQ ID NO: 192 - protein, 827 aa, synthetic construct
HSDPARRGELSVCDSISEWVTAADKKTAVDMSGGTVTVLEKVPVSKGQLKQYFYETKCNPMGYTKEGCRGIDKRHWNSQCRTTQSYVRALTMDSKKRIGWRFIRIDTSCVCTLTIKRGRGSDAHKSEVAHRFKDLGEENFKALVLIAFAQYLQQCPFEDHVKLVNEVTEFAKTCVADESAENCDKSLHTLFGDKLCTVATLRETYGEMADCCAKQEPERNECFLQHKDDNPNLPRLVRPEVDVMCTAFHDNEETFLKKYLYEIARRHPYFYAPELLFFAKRYKAAFTECCQAADKAACLLPKLDELRDEGKASSAKQGLKCASLQKFGERAFKAWAVARLSQRFPKAEFAEVSKLVTDLTKVHTECCHGDLLECADDRADLAKYICENQDSISSKLKECCEKPLLEKSHCIAEVENDEMPADLPSLAADFVGSKDVCKNYAEAKDVFLGMFLYEYARRHPDYSVVLLLRLAKTYETTLEKCCAAADPHECYAKVFDEFKPLVEEPQNLIKQNCELFEQLGEYKFQNALLVRYTKKVPQVSTPTLVEVSRNLGKVGSKCCKHPEAKRMPCAEDCLSVFLNQLCVLHEKTPVSDRVTKCCTESLVNGRPCFSALEVDETYVPKEFNAETFTFHADICTLSEKERQIKKQTALVELVKHKPKATKEQLKAVMDDFAAFVEKCCKADDKETCFAEEGKKLVAASQAALGLGSGGSQVQLVESGGGLVQPGGSLRLSCAASGSIFDIYVMRWYRQAPGKGLEWVASIYDGGRNDYDNVVKGRFTISRDNSKNTLYLQMNSLRAEDTAVYFCNVLTYAGRPYWGQGTQVTVSS

SEQ ID NO: 193 - protein, 827 aa, synthetic construct
HSDPARRGELSVCDSISEWVTAADKKTAVDMSGGTVTVLEKVPVSKGQLKQYFYETKCNPMGYTKEGCRGIDKRHWNSQCRTTQSYVRALTMDSKKRIGWRFIRIDTSCVCTLTIKRGRGSGGSQVQLVESGGGLVQPGGSLRLSCAASGSIFDIYVMRWYRQAPGKGLEWVASIYDGGRNDYDNVVKGRFTISRDNSKNTLYLQMNSLRAEDTAVYFCNVLTYAGRPYWGQGTQVTVSSGSDAHKSEVAHRFKDLGEENFKALVLIAFAQYLQQCPFEDHVKLVNEVTEFAKTCVADESAENCDKSLHTLFGDKLCTVATLRETYGEMADCCAKQEPERNECFLQHKDDNPNLPRLVRPEVDVMCTAFHDNEETFLKKYLYEIARRHPYFYAPELLFFAKRYKAAFTECCQAADKAACLLPKLDELRDEGKASSAKQGLKCASLQKFGERAFKAWAVARLSQRFPKAEFAEVSKLVTDLTKVHTECCHGDLLECADDRADLAKYICENQDSISSKLKECCEKPLLEKSHCIAEVENDEMPADLPSLAADFVGSKDVCKNYAEAKDVFLGMFLYEYARRHPDYSVVLLLRLAKTYETTLEKCCAAADPHECYAKVFDEFKPLVEEPQNLIKQNCELFEQLGEYKFQNALLVRYTKKVPQVSTPTLVEVSRNLGKVGSKCCKHPEAKRMPCAEDCLSVFLNQLCVLHEKTPVSDRVTKCCTESLVNGRPCFSALEVDETYVPKEFNAETFTFHADICTLSEKERQIKKQTALVELVKHKPKATKEQLKAVMDDFAAFVEKCCKADDKETCFAEEGKKLVAASQAALGL

SEQ ID NO: 194 - DNA, 1757 bp, synthetic construct
  source 1..1757: mol_type = other DNA
gaattcacgcgtgccgccaccatgagcagctggattaggtggcacggaccagctatggctaggctctggggattctgttggctggtggtgggcttctggagagctgccttcgcttgccctacaagctgtaagtgcagcgcttctaggatctggtgcagcgacccaagccccggcattgtcgcctttcctaggctggagcctaacagcgtggacccagagaacattactgaaatcttcatcgccaaccagaagagactcgagatcatcaatgaggacgacgtggaagcctacgtcggactgagaaatctgacaatcgtcgatagcggactgaagtttgtggctcacaaggccttcctcaagaacagcaatctgcagcatatcaatttcacaagaaacaaactgacttccctctctaggaagcactttaggcatctggatctcagcgaactgattctggtcggcaacccattcacttgcagctgcgacatcatgtggatcaagacactccaagaggctaagtccagcccagatacacaagatttgtactgtctgaatgagtccagcaagaatatcccactcgccaatctgcagattccaaactgtggactcccttccgctaatctggctgccccaaatctgacagtggaggagggcaaatccatcacactgagctgtagcgtggctggcgatccagtccctaatatgtactgggacgtcggcaacctcgtcagcaagcacatgaacgagacatcccatactcaaggctctctgaggatcacaaacatcagcagcgatgactccggcaagcagatcagctgtgtggccgagaacctcgtcggcgaagaccaagatagcgtcaatctcactgtccacttcgcccctacaatcacttttctggagtcccctacttccgaccaccactggtgtatccctttcacagtgaagggaaatcctaagccagctctgcagtggttctataacggcgccattctgaacgagagcaagtacatctgcactaagatccacgtgactaatcacactgagtaccacggctgtctgcaactcgacaacccaactcacatgaacaacggcgactacactctcatcgccaaaaacgagtacggcaaggacgagaagcaaatctccgcccactttatgggctggcccggcatcgatgacggcgccaatccaaactacccagatgtcatctacgaggactatggcacagccgccaacgacatcggcgatactacaaataggtccaacgagatcccatccactgatgtcacagacaagactggaagggagcacatctctctggtcactgctctgcatctggtgctcggactcagcgctgtgctgggactgctgctgctgagatggcagtttccagcccactataggaggctgaggcatgctctgtggccatctctgcccgatctgcacagagtcctcggccagtatctgagggatacagccgctctgagcccacctaaggccacagtcagcgacacttgcgaagaggtcgaaccatctctgctggagattctgcctaaatcctccgagagaacaccactgccactctgcagcagccaagcccagatggactataggagactgcagcctagctgtctgggcacaatgcctctcagcgtctgccctcctatggctgagagcggcagctgttgcacaactcacatcgccaatcacagctacctccctctgtcctattggcagcagccataataagcggccgc

SEQ ID NO: 195 - protein, 8 aa, synthetic construct
GSHHHHHH

SEQ ID NO: 196 - protein, 5 aa, synthetic construct
GSGGS